European Patent Application EP 4 578 945 A1, published July 2, 2025. Title: CRISPR-CAS13 SYSTEM AND USE THEREOF. Applicant: GUANGZHOU REFORGENE MEDICINE CO., LTD. Application CN PCT/CN2023/115093, filed August 25, 2023. The sequence listing filed with the application follows.

SEQUENCE LISTING (280 sequences)

SEQ ID NO: 1 - protein, 893 aa, synthetic construct
MSKDKKTKAKRMGVKALLAHGEDKLTMTTFGKGNRSKIEFTEGYHGRALETPKHFGIRGFEVRRIDENVDLCGDLEEGKTIEALLVNPSEKVGEDYLKLKGTLEKRFFGREFPHDNIRIQLIYNILDIYKILGMNVADILYALGNMQDTELDIDMFGQSLNNEDNLKECLKRMRPYMGYFGDIFKISPKGENIADREHNKKVLRCISVLRNATAHDKQDEYPWFKSSDIYETKIFKADMWKIIKDQYREKIKKVNKDFLSKNAVNMAILFDLLNARDVEQKKQITDEFYRFTIRKDGKNLGMNLVKIREIIIDRYASGLRDKKHDPHRQKINVIADFLIFRALSQNQGIIDKTVSSLRLTKDEEEKDHVYQNAAELVWGMVSNCLTPYFNDPKNKYILKYKDAKTPGDFEDWITSKISEDDGEPFVKVLSFLCNFLEGKEINELLTAYIHKFECIQDFLNVISSLGENVQFQPRFALFNNASFAQNVAVQLRILASIGKMKPDLTEAKRPLYKAAIRMLCPPEKWEKYTSDEWLEKNMLLNSEDRKNDKKKKQVNPFRNFIAGNVIESRRFMYLVRYSKPKAVRAIMQNRSIVNYVLHRLPSEQVHRYASVFPENFADLEQEIDFLTKKLFEFSFEELLHEKDVILNNSRSHKPSLEIERLKAITGLYLSVAYIAIKNIVKANARYYIAFAVFERDKELVKAKDARIQTKIPETDFPDYFCLTQYYLDRDEEKKFPGDPRDKEAFFEHLRKTKRHFSKQWREWLNEKIADAKSSQATGLLLREARNDVEHLNVLRAIPDYIQDFRHGEKGETAMNSYFELYHYLMQRLMLKNTELDLSHWSGWIMRSGRPDRDLIQIAFVSLAYNLPRYRNLTKEHHFDDTVLQKIREKESLD

SEQ ID NO: 2 - protein, 966 aa, synthetic construct
IEKKKSFAKGMGVKSTLVSGSKVYMTTFAEGSDARLEKIVEGDSIRSVNEGEAFSAEMADKNAGYKIGNAKFSHPKGYAVVANNPLYTGPVQQDMLGLKETLEKRYFGESADGNDNICIQVIHNILDIEKILAEYITNAAYAVNNISGLDKDIIGFGKFSTVYTYDEFKDPEHHRAAFNNNDKLINAIKAQYDEFDNFLDNPRLGYFGQAFFSKEGRNYIINYGNECYDILALLSGLRHWVVHNNEEESRISRTWLYNLDKNLDNEYISTLNYLYDRITNELTNSFSKNSAANVNYIAETLGINPAEFAEQYFRFSIMKEQKNLGFNITKLREVMLDRKDMSEIRKNHKVFDSIRTKVYTMMDFVIYRYYIEEDAKVAAANKSLPDNEKSLSEKDIFVINLRGSFNDDQKDALYYDEANRIWRKLENIMHNIKEFRGNKTREYKKKDAPRLPRILPAGRDVSAFSKLMYALTMFLDGKEINDLLTTLINKFDNIQSFLKVMPLIGVNAKFVEEYAFFKDSAKIADELRLIKSFARMGEPIADARRAMYIDAIRILGTNLSYDELKALADTFSLDENGNKLKKGKHGMRNFIINNVISNKRFHYLIRYGDPAHLHEIAKNEAVVKFVLGRIADIQKKQGQNGKNQIDRYYETCIGKDKGKSVSEKVDALTKIITGMNYDQFDKKRSVIEDTGRENAEREKFKKIISLYLTVIYHILKNIVNINARYVIGFHCVERDAQLYKEKGYDINLKKLEEKGFSSVTKLCAGIDETAPDKRKDVEKEMAERAKESIDSLESANPKLYANYIKYSDEKKAEEFTRQINREKAKTALNAYLRNTKWNVIIREDLLRIDNKTCTLFRNKAVHLEVARYVHAYINDIAEVNSYFQLYHYIMQRIIMNERYEKSSGKVSEYFDAVNDEKKYNDRLLKLLCVPFGYCIPRFKNLSIEALFDRNEAAKFDKEKKKVSGNS

SEQ ID NO: 3 - RNA, 36 nt, synthetic construct
  source 1..36: mol_type = other RNA
ggaagataactctacaaacctgtagggttctgagac

SEQ ID NO: 4 - RNA, 30 nt, synthetic construct
  source 1..30: mol_type = other RNA
tgccgttcttctgcttgtcggccatgatat

SEQ ID NO: 5 - RNA, 26 nt, synthetic construct
  source 1..26: mol_type = other RNA
agggcagaaccgatgctgatgaagac

SEQ ID NO: 6 - RNA, 30 nt, synthetic construct
  source 1..30: mol_type = other RNA
gtggttggagaactggatgtagatgggctg

SEQ ID NO: 7 - RNA, 48 nt, synthetic construct
  source 1..48: mol_type = other RNA
ccacgaccctctttgtcttcactcgagtgaagacaaagagggtcgtgg

SEQ ID NO: 8 - RNA, 48 nt, synthetic construct
  source 1..48: mol_type = other RNA
cagcccatctacatccagttcctcgaggaactggatgtagatgggctg

SEQ ID NO: 9 - DNA, 2682 bp, synthetic construct
  source 1..2682: mol_type = other DNA
atgagcaaagacaaaaaaacaaaagcgaaacgaatgggagtcaaagccctgttggctcacggggaagataaactgacgatgaccacctttgggaaaggaaaccgttcgaagatcgagtttacggaagggtatcacggccgagcgcttgagacccccaaacactttggaatacgcggctttgaggtaaggaggatcgatgaaaacgtcgatctctgcggggatctcgaggaggggaaaacgatcgaggccttgctggtcaacccgtctgaaaaagtcggcgaggactacctcaagcttaaggggacactggaaaaacgtttcttcggccgtgaatttccgcatgacaacatccggatccagctcatctataatattctcgacatttataagattttggggatgaatgtcgctgatattctttacgcgctgggaaacatgcaggatacagagctggacattgatatgtttggacagtctttgaacaatgaagacaaccttaaagaatgtctgaaacgaatgcggccttatatgggctatttcggagatattttcaagatttccccaaaaggcgagaacatagccgatcgggaacataacaaaaaagttctgcgctgtatttctgttctgcgcaacgctaccgcccatgacaaacaagacgaatatccgtggttcaagagcagcgacatctacgaaacgaaaatttttaaggcggacatgtggaaaatcatcaaggaccaatatcgggaaaagatcaagaaagtcaataaggattttttatcgaaaaacgcggttaacatggccatcctatttgaccttctgaatgcccgtgatgtggaacagaaaaagcagatcacggatgaattctatcgtttcacgattcgaaaagacgggaagaatctggggatgaatctggttaagatccgcgagataattattgatcgttacgccagtggcctccgtgataaaaagcacgatcctcaccgccagaaaatcaatgtgatcgcggacttcctgattttccgcgctctttcgcaaaatcagggaatcatcgacaagaccgtttccagcctgcgcctcacgaaagacgaagaggaaaaagaccacgtgtaccagaatgccgcggaactggtctgggggatggtcagtaattgtttgaccccgtattttaacgaccctaaaaataaatacattcttaaatacaaagacgccaaaactcctggtgacttcgaggattggatcaccagtaaaatctcggaggatgacggggagccgttcgtgaaagtgctttcgttcctctgtaatttcctggaagggaaggaaatcaacgagctgctgaccgcttacattcataaattcgagtgtattcaggacttcttgaacgtgatttccagtcttggggaaaacgttcagtttcagcctcgtttcgcgctgttcaacaatgccagtttcgcccaaaatgttgcggtacagttgcgtatcctggcaagtatcgggaagatgaaacccgatttgaccgaggcgaaacgcccgctttacaaggcagcgattcggatgctttgtcctccagagaagtgggaaaaatacacctcggatgagtggcttgaaaaaaatatgctcctcaattccgaggaccgtaaaaatgataaaaagaagaaacaggtcaaccctttccggaatttcatcgcggggaatgtgatcgagtcacgtcggtttatgtatctggtccggtattcaaagccgaaagcggttcgtgcgattatgcaaaaccggagtatcgtgaactatgttcttcacaggcttccgtccgagcaggttcaccggtacgccagcgtgtttcctgaaaatttcgccgatctggaacaggaaattgacttcttgacaaagaaacttttcgaattctcattcgaggaactcctccatgaaaaggatgtgattttgaataattccagatctcacaaaccttccttagagatcgaacgccttaaagccattacagggctgtacctttcggttgcctacatcgccatcaaaaacatcgtgaaagccaacgcacggtattacatcgccttcgcggttttcgaacgtgacaaggaactggtgaaagccaaggacgcacgaatccagacgaagatccccgagacagattttccggactatttctgcctcacgcagtattaccttgaccgcgatgaggagaaaaaattcccgggtgacccgcgtgataaagaggcttttttcgaacatctccgcaagacgaaacggcatttctcaaaacagtggcgcgagtggctgaatgagaaaattgcggacgcaaagagctcccaggcaaccggccttttgttgagagaggcccgaaacgacgtggaacatttgaacgtcctgcgcgcgatcccggattacatccaggatttccgccatggggaaaaaggggaaacggcaatgaattcgtatttcgagctgtaccattacctcatgcagaggctgatgctcaaaaacacggaattggatttgtcccattggagcggctggatcatgcgttccggtcggccggatcgggatttgattcagatcgcgttcgtttcattggcttacaatctgccgcgctaccgtaatttgacgaaggaacaccatttcgatgatacggtattgcagaaaattcgtgagaaagagtccctagactaa

SEQ ID NO: 10 - DNA, 8182 bp, synthetic construct
  source 1..8182: mol_type = other DNA
tggcgaatgggacgcgccctgtagcggcgcattaagcgcggcgggtgtggtggttacgcgcagcgtgaccgctacacttgccagcgccctagcgcccgctcctttcgctttcttcccttcctttctcgccacgttcgccggctttccccgtcaagctctaaatcgggggctccctttagggttccgatttagtgctttacggcacctcgaccccaaaaaacttgattagggtgatggttcacgtagtgggccatcgccctgatagacggtttttcgccctttgacgttggagtccacgttctttaatagtggactcttgttccaaactggaacaacactcaaccctatctcggtctattcttttgatttataagggattttgccgatttcggcctattggttaaaaaatgagctgatttaacaaaaatttaacgcgaattttaacaaaatattaacgtttacaatttcaggtggcacttttcggggaaatgtgcgcggaacccctatttgtttatttttctaaatacattcaaatatgtatccgctcatgaattaattcttagaaaaactcatcgagcatcaaatgaaactgcaatttattcatatcaggattatcaataccatatttttgaaaaagccgtttctgtaatgaaggagaaaactcaccgaggcagttccataggatggcaagatcctggtatcggtctgcgattccgactcgtccaacatcaatacaacctattaatttcccctcgtcaaaaataaggttatcaagtgagaaatcaccatgagtgacgactgaatccggtgagaatggcaaaagtttatgcatttctttccagacttgttcaacaggccagccattacgctcgtcatcaaaatcactcgcatcaaccaaaccgttattcattcgtgattgcgcctgagcgagacgaaatacgcgatcgctgttaaaaggacaattacaaacaggaatcgaatgcaaccggcgcaggaacactgccagcgcatcaacaatattttcacctgaatcaggatattcttctaatacctggaatgctgttttcccggggatcgcagtggtgagtaaccatgcatcatcaggagtacggataaaatgcttgatggtcggaagaggcataaattccgtcagccagtttagtctgaccatctcatctgtaacatcattggcaacgctacctttgccatgtttcagaaacaactctggcgcatcgggcttcccatacaatcgatagattgtcgcacctgattgcccgacattatcgcgagcccatttatacccatataaatcagcatccatgttggaatttaatcgcggcctagagcaagacgtttcccgttgaatatggctcataacaccccttgtattactgtttatgtaagcagacagttttattgttcatgaccaaaatcccttaacgtgagttttcgttccactgagcgtcagaccccgtagaaaagatcaaaggatcttcttgagatcctttttttctgcgcgtaatctgctgcttgcaaacaaaaaaaccaccgctaccagcggtggtttgtttgccggatcaagagctaccaactctttttccgaaggtaactggcttcagcagagcgcagataccaaatactgtccttctagtgtagccgtagttaggccaccacttcaagaactctgtagcaccgcctacatacctcgctctgctaatcctgttaccagtggctgctgccagtggcgataagtcgtgtcttaccgggttggactcaagacgatagttaccggataaggcgcagcggtcgggctgaacggggggttcgtgcacacagcccagcttggagcgaacgacctacaccgaactgagatacctacagcgtgagctatgagaaagcgccacgcttcccgaagggagaaaggcggacaggtatccggtaagcggcagggtcggaacaggagagcgcacgagggagcttccagggggaaacgcctggtatctttatagtcctgtcgggtttcgccacctctgacttgagcgtcgatttttgtgatgctcgtcaggggggcggagcctatggaaaaacgccagcaacgcggcctttttacggttcctggccttttgctggccttttgctcacatgttctttcctgcgttatcccctgattctgtggataaccgtattaccgcctttgagtgagctgataccgctcgccgcagccgaacgaccgagcgcagcgagtcagtgagcgaggaagcggaagagcgcctgatgcggtattttctccttacgcatctgtgcggtatttcacaccgcatatatggtgcactctcagtacaatctgctctgatgccgcatagttaagccagtatacactccgctatcgctacgtgactgggtcatggctgcgccccgacacccgccaacacccgctgacgcgccctgacgggcttgtctgctcccggcatccgcttacagacaagctgtgaccgtctccgggagctgcatgtgtcagaggttttcaccgtcatcaccgaaacgcgcgaggcagctgcggtaaagctcatcagcgtggtcgtgaagcgattcacagatgtctgcctgttcatccgcgtccagctcgttgagtttctccagaagcgttaatgtctggcttctgataaagcgggccatgttaagggcggttttttcctgtttggtcactgatgcctccgtgtaagggggatttctgttcatgggggtaatgataccgatgaaacgagagaggatgctcacgatacgggttactgatgatgaacatgcccggttactggaacgttgtgagggtaaacaactggcggtatggatgcggcgggaccagagaaaaatcactcagggtcaatgccagcgcttcgttaatacagatgtaggtgttccacagggtagccagcagcatcctgcgatgcagatccggaacataatggtgcagggcgctgacttccgcgtttccagactttacgaaacacggaaaccgaagaccattcatgttgttgctcaggtcgcagacgttttgcagcagcagtcgcttcacgttcgctcgcgtatcggtgattcattctgctaaccagtaaggcaaccccgccagcctagccgggtcctcaacgacaggagcacgatcatgcgcacccgtggggccgccatgccggcgataatggcctgcttctcgccgaaacgtttggtggcgggaccagtgacgaaggcttgagcgagggcgtgcaagattccgaataccgcaagcgacaggccgatcatcgtcgcgctccagcgaaagcggtcctcgccgaaaatgacccagagcgctgccggcacctgtcctacgagttgcatgataaagaagacagtcataagtgcggcgacgatagtcatgccccgcgcccaccggaaggagctgactgggttgaaggctctcaagggcatcggtcgagatcccggtgcctaatgagtgagctaacttacattaattgcgttgcgctcactgcccgctttccagtcgggaaacctgtcgtgccagctgcattaatgaatcggccaacgcgcggggagaggcggtttgcgtattgggcgccagggtggtttttcttttcaccagtgagacgggcaacagctgattgcccttcaccgcctggccctgagagagttgcagcaagcggtccacgctggtttgccccagcaggcgaaaatcctgtttgatggtggttaacggcgggatataacatgagctgtcttcggtatcgtcgtatcccactaccgagatatccgcaccaacgcgcagcccggactcggtaatggcgcgcattgcgcccagcgccatctgatcgttggcaaccagcatcgcagtgggaacgatgccctcattcagcatttgcatggtttgttgaaaaccggacatggcactccagtcgccttcccgttccgctatcggctgaatttgattgcgagtgagatatttatgccagccagccagacgcagacgcgccgagacagaacttaatgggcccgctaacagcgcgatttgctggtgacccaatgcgaccagatgctccacgcccagtcgcgtaccgtcttcatgggagaaaataatactgttgatgggtgtctggtcagagacatcaagaaataacgccggaacattagtgcaggcagcttccacagcaatggcatcctggtcatccagcggatagttaatgatcagcccactgacgcgttgcgcgagaagattgtgcaccgccgctttacaggcttcgacgccgcttcgttctaccatcgacaccaccacgctggcacccagttgatcggcgcgagatttaatcgccgcgacaatttgcgacggcgcgtgcagggccagactggaggtggcaacgccaatcagcaacgactgtttgcccgccagttgttgtgccacgcggttgggaatgtaattcagctccgccatcgccgcttccactttttcccgcgttttcgcagaaacgtggctggcctggttcaccacgcgggaaacggtctgataagagacaccggcatactctgcgacatcgtataacgttactggtttcacattcaccaccctgaattgactctcttccgggcgctatcatgccataccgcgaaaggttttgcgccattcgatggtgtccgggatctcgacgctctcccttatgcgactcctgcattaggaagcagcccagtagtaggttgaggccgttgagcaccgccgccgcaaggaatggtgcatgcaaggagatggcgcccaacagtcccccggccacggggcctgccaccatacccacgccgaaacaagcgctcatgagcccgaagtggcgagcccgatcttccccatcggtgatgtcggcgatataggcgccagcaaccgcacctgtggcgccggtgatgccggccacgatgcgtccggcgtagaggatcgagatctcgatcccgcgaaattaatacgactcactataggggaattgtgagcggataacaattcccctctagaaataattttgtttaactttaagaaggagatataccatgggcagcagccatcatcatcatcatcacagcagcggcctggtgccgcgcggcagccatatggctagcatgactggtggacagcaaatgggtcgcggatccccggcagctaagaaaaagaaactggatggcagcgtcgacatgagcaaggacaagaaaaccaaggccaagagaatgggcgtgaaggccctgctggcccacggcgaggacaagctgaccatgaccaccttcggcaagggcaacagaagcaagatcgagttcaccgagggctaccacggcagagccctggagacacccaagcacttcggcatcagaggcttcgaggtgagaagaatcgacgagaacgtggacctgtgcggcgacctggaggagggcaagaccatcgaggccctgctggtgaaccccagcgagaaggtgggcgaggactacctgaagctgaagggcaccctggagaagagattcttcggcagagagttcccccacgacaacatcagaatccagctgatctacaacatcctggacatctacaagatcctgggcatgaacgtggccgacatcctgtacgccctgggcaacatgcaggacaccgagctggacatcgacatgttcggccagagcctgaacaacgaggacaacctgaaggagtgcctgaagagaatgaggccctacatgggctacttcggcgacatcttcaagatcagccccaagggcgagaacatcgccgacagagagcacaacaagaaggtgctgagatgcatcagcgtgctgagaaacgccaccgcccacgacaagcaggacgagtacccctggttcaagagcagcgacatctacgagacaaagatcttcaaggccgacatgtggaagatcatcaaggaccagtacagagagaagatcaagaaggtgaacaaggacttcctgagcaagaacgccgtgaacatggccatcctgttcgacctgctgaacgccagagacgtggagcagaagaagcagatcaccgacgagttctacagattcaccatcagaaaggacggcaagaacctgggcatgaacctggtgaagatcagagagatcatcatcgacagatacgccagcggcctgagagacaagaagcacgacccccacagacagaagatcaacgtgatcgccgacttcctgatcttcagagccctgagccagaaccagggcatcatcgacaagaccgtgagcagcctgagactgaccaaggacgaggaggagaaggaccacgtgtaccagaacgccgccgagctggtgtggggcatggtgagcaactgcctgaccccctacttcaacgaccccaagaacaagtacatcctgaagtacaaggacgccaagacccccggcgacttcgaggactggatcaccagcaagatcagcgaggacgacggcgagcccttcgtgaaggtgctgagcttcctgtgcaacttcctggagggcaaggagatcaacgagctgctgaccgcctacatccacaagttcgagtgcatccaggacttcctgaacgtgatcagcagcctgggcgagaacgtgcagttccagcccagattcgccctgttcaacaacgccagcttcgcccagaacgtggccgtgcagctgagaatcctggccagcatcggcaagatgaagcccgacctgaccgaggccaagaggcccctgtacaaggccgccatcagaatgctgtgcccccccgagaagtgggagaagtacaccagcgacgagtggctggagaagaacatgctgctgaacagcgaggacagaaagaacgacaagaagaagaagcaggtgaaccccttcagaaacttcatcgccggcaacgtgatcgagagcagaagattcatgtacctggtgagatacagcaagcccaaggccgtgagagccatcatgcagaacagaagcatcgtgaactacgtgctgcacagactgcccagcgagcaggtgcacagatacgccagcgtgttccccgagaacttcgccgacctggagcaggagatcgacttcctgaccaagaagctgttcgagttcagcttcgaggagctgctgcacgagaaggacgtgatcctgaacaacagcagaagccacaagcccagcctggagatcgagagactgaaggccatcaccggcctgtacctgagcgtggcctacatcgccatcaagaacatcgtgaaggccaacgccagatactacatcgccttcgccgtgttcgagagagacaaggagctggtgaaggccaaggacgccagaatccagaccaagatccccgagacagacttccccgactacttctgcctgacccagtactacctggacagagacgaggagaagaagttccccggcgaccccagagacaaggaggccttcttcgagcacctgagaaagaccaagagacacttcagcaagcagtggagagagtggctgaacgagaagatcgccgacgccaagagcagccaggccaccggcctgctgctgagagaggccagaaacgacgtggagcacctgaacgtgctgagagccatccccgactacatccaggacttcagacacggcgagaagggcgagacagccatgaacagctacttcgagctgtaccactacctgatgcagagactgatgctgaagaacaccgagctggacctgagccactggagcggctggatcatgagaagcggcagacccgacagagacttgatccagatcgccttcgtgagcctggcctacaacctgcccagatacagaaacctgaccaaggagcaccacttcgacgacaccgtgctgcagaagatcagagagaaggagagcctggacacaggcggcggccccggcggcggcgccgccgccggcagcggcagccctaagaaaaaacgaaaagttggcagcggaagcaaaaggccggcggccacgaaaaaggccggccaggcaaaaaagaaaaagtaactcgagcaccaccaccaccaccactgagatccggctgctaacaaagcccgaaaggaagctgagttggctgctgccaccgctgagcaataactagcataaccccttggggcctctaaacgggtcttgaggggttttttgctgaaaggaggaactatatccggat

SEQ ID NO: 11 - protein, 982 aa, synthetic construct
MGSSHHHHHHSSGLVPRGSHMASMTGGQQMGRGSPAAKKKKLDGSVDMSKDKKTKAKRMGVKALLAHGEDKLTMTTFGKGNRSKIEFTEGYHGRALETPKHFGIRGFEVRRIDENVDLCGDLEEGKTIEALLVNPSEKVGEDYLKLKGTLEKRFFGREFPHDNIRIQLIYNILDIYKILGMNVADILYALGNMQDTELDIDMFGQSLNNEDNLKECLKRMRPYMGYFGDIFKISPKGENIADREHNKKVLRCISVLRNATAHDKQDEYPWFKSSDIYETKIFKADMWKIIKDQYREKIKKVNKDFLSKNAVNMAILFDLLNARDVEQKKQITDEFYRFTIRKDGKNLGMNLVKIREIIIDRYASGLRDKKHDPHRQKINVIADFLIFRALSQNQGIIDKTVSSLRLTKDEEEKDHVYQNAAELVWGMVSNCLTPYFNDPKNKYILKYKDAKTPGDFEDWITSKISEDDGEPFVKVLSFLCNFLEGKEINELLTAYIHKFECIQDFLNVISSLGENVQFQPRFALFNNASFAQNVAVQLRILASIGKMKPDLTEAKRPLYKAAIRMLCPPEKWEKYTSDEWLEKNMLLNSEDRKNDKKKKQVNPFRNFIAGNVIESRRFMYLVRYSKPKAVRAIMQNRSIVNYVLHRLPSEQVHRYASVFPENFADLEQEIDFLTKKLFEFSFEELLHEKDVILNNSRSHKPSLEIERLKAITGLYLSVAYIAIKNIVKANARYYIAFAVFERDKELVKAKDARIQTKIPETDFPDYFCLTQYYLDRDEEKKFPGDPRDKEAFFEHLRKTKRHFSKQWREWLNEKIADAKSSQATGLLLREARNDVEHLNVLRAIPDYIQDFRHGEKGETAMNSYFELYHYLMQRLMLKNTELDLSHWSGWIMRSGRPDRDLIQIAFVSLAYNLPRYRNLTKEHHFDDTVLQKIREKESLDTGGGPGGGAAAGSGSPKKKRKVGSGSKRPAATKKAGQAKKKK

SEQ ID NO: 12 - DNA, 720 bp, synthetic construct
  source 1..720: mol_type = other DNA
atggtgagcaagggcgaggagctgttcaccggggtggtgcccatcctggtcgagctggacggcgacgtaaacggccacaagttcagcgtgtccggcgagggcgagggcgatgccacctacggcaagctgaccctgaagttcatctgcaccaccggcaagctgcccgtgccctggcccaccctcgtgaccaccctgacctacggcgtgcagtgcttcagccgctaccccgaccacatgaagcagcacgacttcttcaagtccgccatgcccgaaggctacgtccaggagcgcaccatcttcttcaaggacgacggcaactacaagacccgcgccgaggtgaagttcgagggcgacaccctggtgaaccgcatcgagctgaagggcatcgacttcaaggaggacggcaacatcctggggcacaagctggagtacaactacaacagccacaacgtctatatcatggccgacaagcagaagaacggcatcaaggtgaacttcaagatccgccacaacatcgaggacggcagcgtgcagctcgccgaccactaccagcagaacacccccatcggcgacggccccgtgctgctgcccgacaaccactacctgagcacccagtccgccctgagcaaagaccccaacgagaagcgcgatcacatggtcctgctggagttcgtgaccgccgccgggatcactctcggcatggacgagctgtacaagtaa

SEQ ID NO: 13 - DNA, 4828 bp, synthetic construct
  source 1..4828: mol_type = other DNA
cctgcaggcagctgcgcgctcgctcgctcactgaggccgcccgggcgtcgggcgacctttggtcgcccggcctcagtgagcgagcgagcgcgcagagagggagtggccaactccatcactaggggttcctgcggcctctagactcgaggcgttgacattgattattgactagttattaatagtaatcaattacggggtcattagttcatagcccatatatggagttccgcgttacataacttacggtaaatggcccgcctggctgaccgcccaacgacccccgcccattgacgtcaataatgacgtatgttcccatagtaacgccaatagggactttccattgacgtcaatgggtggagtatttacggtaaactgcccacttggcagtacatcaagtgtatcatatgccaagtacgccccctattgacgtcaatgacggtaaatggcccgcctggcattatgcccagtacatgaccttatgggactttcctacttggcagtacatctacgtattagtcatcgctattaccatggtgatgcggttttggcagtacatcaatgggcgtggatagcggtttgactcacggggatttccaagtctccaccccattgacgtcaatgggagtttgttttggcaccaaaatcaacgggactttccaaaatgtcgtaacaactccgccccattgacgcaaatgggcggtaggcgtgtacggtgggaggtctatataagcagagctctctggctaactaccggtgccaccatggtgagcaagggcgaggagctgttcaccggggtggtgcccatcctggtcgagctggacggcgacgtaaacggccacaagttcagcgtgtccggcgagggcgagggcgatgccacctacggcaagctgaccctgaagttcatctgcaccaccggcaagctgcccgtgccctggcccaccctcgtgaccaccctgacctacggcgtgcagtgcttcagccgctaccccgaccacatgaagcagcacgacttcttcaagtccgccatgcccgaaggctacgtccaggagcgcaccatcttcttcaaggacgacggcaactacaagacccgcgccgaggtgaagttcgagggcgacaccctggtgaaccgcatcgagctgaagggcatcgacttcaaggaggacggcaacatcctggggcacaagctggagtacaactacaacagccacaacgtctatatcatggccgacaagcagaagaacggcatcaaggtgaacttcaagatccgccacaacatcgaggacggcagcgtgcagctcgccgaccactaccagcagaacacccccatcggcgacggccccgtgctgctgcccgacaaccactacctgagcacccagtccgccctgagcaaagaccccaacgagaagcgcgatcacatggtcctgctggagttcgtgaccgccgccgggatcactctcggcatggacgagctgtacaagtaaagcggccgaattcctagagctcgctgatcagcctcgactgtgccttctagttgccagccatctgttgtttgcccctcccccgtgccttccttgaccctggaaggtgccactcccactgtcctttcctaataaaatgaggaaattgcatcgcattgtctgagtaggtgtcattctattctggggggtggggtggggcaggacagcaagggggaggattgggaagagaatagcaggcatgctggggaggtaccgagggcctatttcccatgattccttcatatttgcatatacgatacaaggctgttagagagataattggaattaatttgactgtaaacacaaagatattagtacaaaatacgtgacgtagaaagtaataatttcttgggtagtttgcagttttaaaattatgttttaaaatggactatcatatgcttaccgtaacttgaaagtatttcgatttcttggctttatatatcttgtggaaaggacgaaacaccggagaccacggcaggtctcagttttagtactctggaaacagaatctactaaaacaaggcaaaatgccgtgtttatctcgtcaacttgttggcgagatttttgcggccgcaggaacccctagtgatggagttggccactccctctctgcgcgctcgctcgctcactgaggccgggcgaccaaaggtcgcccgacgcccgggctttgcccgggcggcctcagtgagcgagcgagcgcgcagctgcctgcaggggcgcctgatgcggtattttctccttacgcatctgtgcggtatttcacaccgcatacgtcaaagcaaccatagtacgcgccctgtagcggcgcattaagcgcggcgggtgtggtggttacgcgcagcgtgaccgctacacttgccagcgccctagcgcccgctcctttcgctttcttcccttcctttctcgccacgttcgccggctttccccgtcaagctctaaatcgggggctccctttagggttccgatttagtgctttacggcacctcgaccccaaaaaacttgatttgggtgatggttcacgtagtgggccatcgccctgatagacggtttttcgccctttgacgttggagtccacgttctttaatagtggactcttgttccaaactggaacaacactcaaccctatctcgggctattcttttgatttataagggattttgccgatttcggcctattggttaaaaaatgagctgatttaacaaaaatttaacgcgaattttaacaaaatattaacgtttacaattttatggtgcactctcagtacaatctgctctgatgccgcatagttaagccagccccgacacccgccaacacccgctgacgcgccctgacgggcttgtctgctcccggcatccgcttacagacaagctgtgaccgtctccgggagctgcatgtgtcagaggttttcaccgtcatcaccgaaacgcgcgagacgaaagggcctcgtgatacgcctatttttataggttaatgtcatgataataatggtttcttagacgtcaggtggcacttttcggggaaatgtgcgcggaacccctatttgtttatttttctaaatacattcaaatatgtatccgctcatgagacaataaccctgataaatgcttcaataatattgaaaaaggaagagtatgagtattcaacatttccgtgtcgcccttattcccttttttgcggcattttgccttcctgtttttgctcacccagaaacgctggtgaaagtaaaagatgctgaagatcagttgggtgcacgagtgggttacatcgaactggatctcaacagcggtaagatccttgagagttttcgccccgaagaacgttttccaatgatgagcacttttaaagttctgctatgtggcgcggtattatcccgtattgacgccgggcaagagcaactcggtcgccgcatacactattctcagaatgacttggttgagtactcaccagtcacagaaaagcatcttacggatggcatgacagtaagagaattatgcagtgctgccataaccatgagtgataacactgcggccaacttacttctgacaacgatcggaggaccgaaggagctaaccgcttttttgcacaacatgggggatcatgtaactcgccttgatcgttgggaaccggagctgaatgaagccataccaaacgacgagcgtgacaccacgatgcctgtagcaatggcaacaacgttgcgcaaactattaactggcgaactacttactctagcttcccggcaacaattaatagactggatggaggcggataaagttgcaggaccacttctgcgctcggcccttccggctggctggtttattgctgataaatctggagccggtgagcgtggaagccgcggtatcattgcagcactggggccagatggtaagccctcccgtatcgtagttatctacacgacggggagtcaggcaactatggatgaacgaaatagacagatcgctgagataggtgcctcactgattaagcattggtaactgtcagaccaagtttactcatatatactttagattgatttaaaacttcatttttaatttaaaaggatctaggtgaagatcctttttgataatctcatgaccaaaatcccttaacgtgagttttcgttccactgagcgtcagaccccgtagaaaagatcaaaggatcttcttgagatcctttttttctgcgcgtaatctgctgcttgcaaacaaaaaaaccaccgctaccagcggtggtttgtttgccggatcaagagctaccaactctttttccgaaggtaactggcttcagcagagcgcagataccaaatactgtccttctagtgtagccgtagttaggccaccacttcaagaactctgtagcaccgcctacatacctcgctctgctaatcctgttaccagtggctgctgccagtggcgataagtcgtgtcttaccgggttggactcaagacgatagttaccggataaggcgcagcggtcgggctgaacggggggttcgtgcacacagcccagcttggagcgaacgacctacaccgaactgagatacctacagcgtgagctatgagaaagcgccacgcttcccgaagggagaaaggcggacaggtatccggtaagcggcagggtcggaacaggagagcgcacgagggagcttccagggggaaacgcctggtatctttatagtcctgtcgggtttcgccacctctgacttgagcgtcgatttttgtgatgctcgtcaggggggcggagcctatggaaaaacgccagcaacgcggcctttttacggttcctggccttttgctggccttttgctcacatgt

SEQ ID NO: 14 - DNA, 6803 bp, synthetic construct
  source 1..6803: mol_type = other DNA
cctgcaggcagctgcgcgctcgctcgctcactgaggccgcccgggcgtcgggcgacctttggtcgcccggcctcagtgagcgagcgagcgcgcagagagggagtggccaactccatcactaggggttcctgcggcctctagactcgaggcgttgacattgattattgactagttattaatagtaatcaattacggggtcattagttcatagcccatatatggagttccgcgttacataacttacggtaaatggcccgcctggctgaccgcccaacgacccccgcccattgacgtcaataatgacgtatgttcccatagtaacgccaatagggactttccattgacgtcaatgggtggagtatttacggtaaactgcccacttggcagtacatcaagtgtatcatatgccaagtacgccccctattgacgtcaatgacggtaaatggcccgcctggcattatgcccagtacatgaccttatgggactttcctacttggcagtacatctacgtattagtcatcgctattaccatggtgatgcggttttggcagtacatcaatgggcgtggatagcggtttgactcacggggatttccaagtctccaccccattgacgtcaatgggagtttgttttggcaccaaaatcaacgggactttccaaaatgtcgtaacaactccgccccattgacgcaaatgggcggtaggcgtgtacggtgggaggtctatataagcagagctctctggctaactaccggtgccaccatgccggcagctaagaaaaagaaactggatggcagcgtcgacatgagcaaggacaagaaaaccaaggccaagagaatgggcgtgaaggccctgctggcccacggcgaggacaagctgaccatgaccaccttcggcaagggcaacagaagcaagatcgagttcaccgagggctaccacggcagagccctggagacacccaagcacttcggcatcagaggcttcgaggtgagaagaatcgacgagaacgtggacctgtgcggcgacctggaggagggcaagaccatcgaggccctgctggtgaaccccagcgagaaggtgggcgaggactacctgaagctgaagggcaccctggagaagagattcttcggcagagagttcccccacgacaacatcagaatccagctgatctacaacatcctggacatctacaagatcctgggcatgaacgtggccgacatcctgtacgccctgggcaacatgcaggacaccgagctggacatcgacatgttcggccagagcctgaacaacgaggacaacctgaaggagtgcctgaagagaatgaggccctacatgggctacttcggcgacatcttcaagatcagccccaagggcgagaacatcgccgacagagagcacaacaagaaggtgctgagatgcatcagcgtgctgagaaacgccaccgcccacgacaagcaggacgagtacccctggttcaagagcagcgacatctacgagacaaagatcttcaaggccgacatgtggaagatcatcaaggaccagtacagagagaagatcaagaaggtgaacaaggacttcctgagcaagaacgccgtgaacatggccatcctgttcgacctgctgaacgccagagacgtggagcagaagaagcagatcaccgacgagttctacagattcaccatcagaaaggacggcaagaacctgggcatgaacctggtgaagatcagagagatcatcatcgacagatacgccagcggcctgagagacaagaagcacgacccccacagacagaagatcaacgtgatcgccgacttcctgatcttcagagccctgagccagaaccagggcatcatcgacaagaccgtgagcagcctgagactgaccaaggacgaggaggagaaggaccacgtgtaccagaacgccgccgagctggtgtggggcatggtgagcaactgcctgaccccctacttcaacgaccccaagaacaagtacatcctgaagtacaaggacgccaagacccccggcgacttcgaggactggatcaccagcaagatcagcgaggacgacggcgagcccttcgtgaaggtgctgagcttcctgtgcaacttcctggagggcaaggagatcaacgagctgctgaccgcctacatccacaagttcgagtgcatccaggacttcctgaacgtgatcagcagcctgggcgagaacgtgcagttccagcccagattcgccctgttcaacaacgccagcttcgcccagaacgtggccgtgcagctgagaatcctggccagcatcggcaagatgaagcccgacctgaccgaggccaagaggcccctgtacaaggccgccatcagaatgctgtgcccccccgagaagtgggagaagtacaccagcgacgagtggctggagaagaacatgctgctgaacagcgaggacagaaagaacgacaagaagaagaagcaggtgaaccccttcagaaacttcatcgccggcaacgtgatcgagagcagaagattcatgtacctggtgagatacagcaagcccaaggccgtgagagccatcatgcagaacagaagcatcgtgaactacgtgctgcacagactgcccagcgagcaggtgcacagatacgccagcgtgttccccgagaacttcgccgacctggagcaggagatcgacttcctgaccaagaagctgttcgagttcagcttcgaggagctgctgcacgagaaggacgtgatcctgaacaacagcagaagccacaagcccagcctggagatcgagagactgaaggccatcaccggcctgtacctgagcgtggcctacatcgccatcaagaacatcgtgaaggccaacgccagatactacatcgccttcgccgtgttcgagagagacaaggagctggtgaaggccaaggacgccagaatccagaccaagatccccgagacagacttccccgactacttctgcctgacccagtactacctggacagagacgaggagaagaagttccccggcgaccccagagacaaggaggccttcttcgagcacctgagaaagaccaagagacacttcagcaagcagtggagagagtggctgaacgagaagatcgccgacgccaagagcagccaggccaccggcctgctgctgagagaggccagaaacgacgtggagcacctgaacgtgctgagagccatccccgactacatccaggacttcagacacggcgagaagggcgagacagccatgaacagctacttcgagctgtaccactacctgatgcagagactgatgctgaagaacaccgagctggacctgagccactggagcggctggatcatgagaagcggcagacccgacagagacttgatccagatcgccttcgtgagcctggcctacaacctgcccagatacagaaacctgaccaaggagcaccacttcgacgacaccgtgctgcagaagatcagagagaaggagagcctggacacaggcggcggccccggcggcggcgccgccgccggcagcggcagccctaagaaaaaacgaaaagttggcagcggaagcaaaaggccggcggccacgaaaaaggccggccaggcaaaaaagaaaaagctcgagtacccatacgatgttccagattacgcttgagaattccccttgagcatctgacttctggctaataaaggaaatttattttcattgcaatagtgtgttggaattttttgtgtctctcaggtaccgagggcctatttcccatgattccttcatatttgcatatacgatacaaggctgttagagagataattggaattaatttgactgtaaacacaaagatattagtacaaaatacgtgacgtagaaagtaataatttcttgggtagtttgcagttttaaaattatgttttaaaatggactatcatatgcttaccgtaacttgaaagtatttcgatttcttggctttatatatcttgtggaaaggacgaaacaccggaagataactctacaaacctgtagggttctgagactgccgttcttctgcttgtcggccatgatatttttttgcggccgcaggaacccctagtgatggagttggccactccctctctgcgcgctcgctcgctcactgaggccgggcgaccaaaggtcgcccgacgcccgggctttgcccgggcggcctcagtgagcgagcgagcgcgcagctgcctgcaggggcgcctgatgcggtattttctccttacgcatctgtgcggtatttcacaccgcatacgtcaaagcaaccatagtacgcgccctgtagcggcgcattaagcgcggcgggtgtggtggttacgcgcagcgtgaccgctacacttgccagcgccttagcgcccgctcctttcgctttcttcccttcctttctcgccacgttcgccggctttccccgtcaagctctaaatcgggggctccctttagggttccgatttagtgctttacggcacctcgaccccaaaaaacttgatttgggtgatggttcacgtagtgggccatcgccctgatagacggtttttcgccctttgacgttggagtccacgttctttaatagtggactcttgttccaaactggaacaacactcaactctatctcgggctattcttttgatttataagggattttgccgatttcggtctattggttaaaaaatgagctgatttaacaaaaatttaacgcgaattttaacaaaatattaacgtttacaattttatggtgcactctcagtacaatctgctctgatgccgcatagttaagccagccccgacacccgccaacacccgctgacgcgccctgacgggcttgtctgctcccggcatccgcttacagacaagctgtgaccgtctccgggagctgcatgtgtcagaggttttcaccgtcatcaccgaaacgcgcgagacgaaagggcctcgtgatacgcctatttttataggttaatgtcatgataataatggtttcttagacgtcaggtggcacttttcggggaaatgtgcgcggaacccctatttgtttatttttctaaatacattcaaatatgtatccgctcatgagacaataaccctgataaatgcttcaataatattgaaaaaggaagagtatgagtattcaacatttccgtgtcgcccttattcccttttttgcggcattttgccttcctgtttttgctcacccagaaacgctggtgaaagtaaaagatgctgaagatcagttgggtgcacgagtgggttacatcgaactggatctcaacagcggtaagatccttgagagttttcgccccgaagaacgttttccaatgatgagcacttttaaagttctgctatgtggcgcggtattatcccgtattgacgccgggcaagagcaactcggtcgccgcatacactattctcagaatgacttggttgagtactcaccagtcacagaaaagcatcttacggatggcatgacagtaagagaattatgcagtgctgccataaccatgagtgataacactgcggccaacttacttctgacaacgatcggaggaccgaaggagctaaccgcttttttgcacaacatgggggatcatgtaactcgccttgatcgttgggaaccggagctgaatgaagccataccaaacgacgagcgtgacaccacgatgcctgtagcaatggcaacaacgttgcgcaaactattaactggcgaactacttactctagcttcccggcaacaattaatagactggatggaggcggataaagttgcaggaccacttctgcgctcggcccttccggctggctggtttattgctgataaatctggagccggtgagcgtggaagccgcggtatcattgcagcactggggccagatggtaagccctcccgtatcgtagttatctacacgacggggagtcaggcaactatggatgaacgaaatagacagatcgctgagataggtgcctcactgattaagcattggtaactgtcagaccaagtttactcatatatactttagattgatttaaaacttcatttttaatttaaaaggatctaggtgaagatcctttttgataatctcatgaccaaaatcccttaacgtgagttttcgttccactgagcgtcagaccccgtagaaaagatcaaaggatcttcttgagatcctttttttctgcgcgtaatctgctgcttgcaaacaaaaaaaccaccgctaccagcggtggtttgtttgccggatcaagagctaccaactctttttccgaaggtaactggcttcagcagagcgcagataccaaatactgttcttctagtgtagccgtagttaggccaccacttcaagaactctgtagcaccgcctacatacctcgctctgctaatcctgttaccagtggctgctgccagtggcgataagtcgtgtcttaccgggttggactcaagacgatagttaccggataaggcgcagcggtcgggctgaacggggggttcgtgcacacagcccagcttggagcgaacgacctacaccgaactgagatacctacagcgtgagctatgagaaagcgccacgcttcccgaagggagaaaggcggacaggtatccggtaagcggcagggtcggaacaggagagcgcacgagggagcttccagggggaaacgcctggtatctttatagtcctgtcgggtttcgccacctctgacttgagcgtcgatttttgtgatgctcgtcaggggggcggagcctatggaaaaacgccagcaacgcggcctttttacggttcctggccttttgctggccttttgctcacatgt

SEQ ID NO: 15 - DNA, 6793 bp, synthetic construct
  source 1..6793: mol_type = other DNA
cctgcaggcagctgcgcgctcgctcgctcactgaggccgcccgggcgtcgggcgacctttggtcgcccggcctcagtgagcgagcgagcgcgcagagagggagtggccaactccatcactaggggttcctgcggcctctagactcgaggcgttgacattgattattgactagttattaatagtaatcaattacggggtcattagttcatagcccatatatggagttccgcgttacataacttacggtaaatggcccgcctggctgaccgcccaacgacccccgcccattgacgtcaataatgacgtatgttcccatagtaacgccaatagggactttccattgacgtcaatgggtggagtatttacggtaaactgcccacttggcagtacatcaagtgtatcatatgccaagtacgccccctattgacgtcaatgacggtaaatggcccgcctggcattatgcccagtacatgaccttatgggactttcctacttggcagtacatctacgtattagtcatcgctattaccatggtgatgcggttttggcagtacatcaatgggcgtggatagcggtttgactcacggggatttccaagtctccaccccattgacgtcaatgggagtttgttttggcaccaaaatcaacgggactttccaaaatgtcgtaacaactccgccccattgacgcaaatgggcggtaggcgtgtacggtgggaggtctatataagcagagctctctggctaactaccggtgccaccatgccggcagctaagaaaaagaaactggatggcagcgtcgacatgagcaaggacaagaaaaccaaggccaagagaatgggcgtgaaggccctgctggcccacggcgaggacaagctgaccatgaccaccttcggcaagggcaacagaagcaagatcgagttcaccgagggctaccacggcagagccctggagacacccaagcacttcggcatcagaggcttcgaggtgagaagaatcgacgagaacgtggacctgtgcggcgacctggaggagggcaagaccatcgaggccctgctggtgaaccccagcgagaaggtgggcgaggactacctgaagctgaagggcaccctggagaagagattcttcggcagagagttcccccacgacaacatcagaatccagctgatctacaacatcctggacatctacaagatcctgggcatgaacgtggccgacatcctgtacgccctgggcaacatgcaggacaccgagctggacatcgacatgttcggccagagcctgaacaacgaggacaacctgaaggagtgcctgaagagaatgaggccctacatgggctacttcggcgacatcttcaagatcagccccaagggcgagaacatcgccgacagagagcacaacaagaaggtgctgagatgcatcagcgtgctgagaaacgccaccgcccacgacaagcaggacgagtacccctggttcaagagcagcgacatctacgagacaaagatcttcaaggccgacatgtggaagatcatcaaggaccagtacagagagaagatcaagaaggtgaacaaggacttcctgagcaagaacgccgtgaacatggccatcctgttcgacctgctgaacgccagagacgtggagcagaagaagcagatcaccgacgagttctacagattcaccatcagaaaggacggcaagaacctgggcatgaacctggtgaagatcagagagatcatcatcgacagatacgccagcggcctgagagacaagaagcacgacccccacagacagaagatcaacgtgatcgccgacttcctgatcttcagagccctgagccagaaccagggcatcatcgacaagaccgtgagcagcctgagactgaccaaggacgaggaggagaaggaccacgtgtaccagaacgccgccgagctggtgtggggcatggtgagcaactgcctgaccccctacttcaacgaccccaagaacaagtacatcctgaagtacaaggacgccaagacccccggcgacttcgaggactggatcaccagcaagatcagcgaggacgacggcgagcccttcgtgaaggtgctgagcttcctgtgcaacttcctggagggcaaggagatcaacgagctgctgaccgcctacatccacaagttcgagtgcatccaggacttcctgaacgtgatcagcagcctgggcgagaacgtgcagttccagcccagattcgccctgttcaacaacgccagcttcgcccagaacgtggccgtgcagctgagaatcctggccagcatcggcaagatgaagcccgacctgaccgaggccaagaggcccctgtacaaggccgccatcagaatgctgtgcccccccgagaagtgggagaagtacaccagcgacgagtggctggagaagaacatgctgctgaacagcgaggacagaaagaacgacaagaagaagaagcaggtgaaccccttcagaaacttcatcgccggcaacgtgatcgagagcagaagattcatgtacctggtgagatacagcaagcccaaggccgtgagagccatcatgcagaacagaagcatcgtgaactacgtgctgcacagactgcccagcgagcaggtgcacagatacgccagcgtgttccccgagaacttcgccgacctggagcaggagatcgacttcctgaccaagaagctgttcgagttcagcttcgaggagctgctgcacgagaaggacgtgatcctgaacaacagcagaagccacaagcccagcctggagatcgagagactgaaggccatcaccggcctgtacctgagcgtggcctacatcgccatcaagaacatcgtgaaggccaacgccagatactacatcgccttcgccgtgttcgagagagacaaggagctggtgaaggccaaggacgccagaatccagaccaagatccccgagacagacttccccgactacttctgcctgacccagtactacctggacagagacgaggagaagaagttccccggcgaccccagagacaaggaggccttcttcgagcacctgagaaagaccaagagacacttcagcaagcagtggagagagtggctgaacgagaagatcgccgacgccaagagcagccaggccaccggcctgctgctgagagaggccagaaacgacgtggagcacctgaacgtgctgagagccatccccgactacatccaggacttcagacacggcgagaagggcgagacagccatgaacagctacttcgagctgtaccactacctgatgcagagactgatgctgaagaacaccgagctggacctgagccactggagcggctggatcatgagaagcggcagacccgacagagacttgatccagatcgccttcgtgagcctggcctacaacctgcccagatacagaaacctgaccaaggagcaccacttcgacgacaccgtgctgcagaagatcagagagaaggagagcctggacacaggcggcggccccggcggcggcgccgccgccggcagcggcagccctaagaaaaaacgaaaagttggcagcggaagcaaaaggccggcggccacgaaaaaggccggccaggcaaaaaagaaaaagctcgagtacccatacgatgttccagattacgcttgagaattccccttgagcatctgacttctggctaataaaggaaatttattttcattgcaatagtgtgttggaattttttgtgtctctcaggtaccgagggcctatttcccatgattccttcatatttgcatatacgatacaaggctgttagagagataattggaattaatttgactgtaaacacaaagatattagtacaaaatacgtgacgtagaaagtaataatttcttgggtagtttgcagttttaaaattatgttttaaaatggactatcatatgcttaccgtaacttgaaagtatttcgatttcttggctttatatatcttgtggaaaggacgaaacaccggaagataactctacaaacctgtagggttctgagacggagaccacggcaggtctcattttttgcggccgcaggaacccctagtgatggagttggccactccctctctgcgcgctcgctcgctcactgaggccgggcgaccaaaggtcgcccgacgcccgggctttgcccgggcggcctcagtgagcgagcgagcgcgcagctgcctgcaggggcgcctgatgcggtattttctccttacgcatctgtgcggtatttcacaccgcatacgtcaaagcaaccatagtacgcgccctgtagcggcgcattaagcgcggcgggtgtggtggttacgcgcagcgtgaccgctacacttgccagcgccttagcgcccgctcctttcgctttcttcccttcctttctcgccacgttcgccggctttccccgtcaagctctaaatcgggggctccctttagggttccgatttagtgctttacggcacctcgaccccaaaaaacttgatttgggtgatggttcacgtagtgggccatcgccctgatagacggtttttcgccctttgacgttggagtccacgttctttaatagtggactcttgttccaaactggaacaacactcaactctatctcgggctattcttttgatttataagggattttgccgatttcggtctattggttaaaaaatgagctgatttaacaaaaatttaacgcgaattttaacaaaatattaacgtttacaattttatggtgcactctcagtacaatctgctctgatgccgcatagttaagccagccccgacacccgccaacacccgctgacgcgccctgacgggcttgtctgctcccggcatccgcttacagacaagctgtgaccgtctccgggagctgcatgtgtcagaggttttcaccgtcatcaccgaaacgcgcgagacgaaagggcctcgtgatacgcctatttttataggttaatgtcatgataataatggtttcttagacgtcaggtggcacttttcggggaaatgtgcgcggaacccctatttgtttatttttctaaatacattcaaatatgtatccgctcatgagacaataaccctgataaatgcttcaataatattgaaaaaggaagagtatgagtattcaacatttccgtgtcgcccttattcccttttttgcggcattttgccttcctgtttttgctcacccagaaacgctggtgaaagtaaaagatgctgaagatcagttgggtgcacgagtgggttacatcgaactggatctcaacagcggtaagatccttgagagttttcgccccgaagaacgttttccaatgatgagcacttttaaagttctgctatgtggcgcggtattatcccgtattgacgccgggcaagagcaactcggtcgccgcatacactattctcagaatgacttggttgagtactcaccagtcacagaaaagcatcttacggatggcatgacagtaagagaattatgcagtgctgccataaccatgagtgataacactgcggccaacttacttctgacaacgatcggaggaccgaaggagctaaccgcttttttgcacaacatgggggatcatgtaactcgccttgatcgttgggaaccggagctgaatgaagccataccaaacgacgagcgtgacaccacgatgcctgtagcaatggcaacaacgttgcgcaaactattaactggcgaactacttactctagcttcccggcaacaattaatagactggatggaggcggataaagttgcaggaccacttctgcgctcggcccttccggctggctggtttattgctgataaatctggagccggtgagcgtggaagccgcggtatcattgcagcactggggccagatggtaagccctcccgtatcgtagttatctacacgacggggagtcaggcaactatggatgaacgaaatagacagatcgctgagataggtgcctcactgattaagcattggtaactgtcagaccaagtttactcatatatactttagattgatttaaaacttcatttttaatttaaaaggatctaggtgaagatcctttttgataatctcatgaccaaaatcccttaacgtgagttttcgttccactgagcgtcagaccccgtagaaaagatcaaaggatcttcttgagatcctttttttctgcgcgtaatctgctgcttgcaaacaaaaaaaccaccgctaccagcggtggtttgtttgccggatcaagagctaccaactctttttccgaaggtaactggcttcagcagagcgcagataccaaatactgttcttctagtgtagccgtagttaggccaccacttcaagaactctgtagcaccgcctacatacctcgctctgctaatcctgttaccagtggctgctgccagtggcgataagtcgtgtcttaccgggttggactcaagacgatagttaccggataaggcgcagcggtcgggctgaacggggggttcgtgcacacagcccagcttggagcgaacgacctacaccgaactgagatacctacagcgtgagctatgagaaagcgccacgcttcccgaagggagaaaggcggacaggtatccggtaagcggcagggtcggaacaggagagcgcacgagggagcttccagggggaaacgcctggtatctttatagtcctgtcgggtttcgccacctctgacttgagcgtcgatttttgtgatgctcgtcaggggggcggagcctatggaaaaacgccagcaacgcggcctttttacggttcctggccttttgctggccttttgctcacatgt

SEQ ID NO: 16 - DNA, 9363 bp, synthetic construct
  source 1..9363: mol_type = other DNA
gtcgacggatcgggagatctcccgatcccctatggtgcactctcagtacaatctgctctgatgccgcatagttaagccagtatctgctccctgcttgtgtgttggaggtcgctgagtagtgcgcgagcaaaatttaagctacaacaaggcaaggcttgaccgacaattgcatgaagaatctgcttagggttaggcgttttgcgctgcttcgcgatgtacgggccagatatacgcgttgacattgattattgactagttattaatagtaatcaattacggggtcattagttcatagcccatatatggagttccgcgttacataacttacggtaaatggcccgcctggctgaccgcccaacgacccccgcccattgacgtcaataatgacgtatgttcccatagtaacgccaatagggactttccattgacgtcaatgggtggagtatttacggtaaactgcccacttggcagtacatcaagtgtatcatatgccaagtacgccccctattgacgtcaatgacggtaaatggcccgcctggcattatgcccagtacatgaccttatgggactttcctacttggcagtacatctacgtattagtcatcgctattaccatggtgatgcggttttggcagtacatcaatgggcgtggatagcggtttgactcacggggatttccaagtctccaccccattgacgtcaatgggagtttgttttggcaccaaaatcaacgggactttccaaaatgtcgtaacaactccgccccattgacgcaaatgggcggtaggcgtgtacggtgggaggtctatagaccagatctgagcctgggagctctctggctaactagggaacccactgcttaagcctcaataaagcttgccttgagtgcttcaagtagtgtgtgcccgtctgttgtgtgactctggtaactagagatccctcagacccttttagtcagtgtggaaaatctctagcagtggcgcccgaacagggacttgaaagcgaaagggaaaccagaggagctctctcgacgcaggactcggcttgctgaagcgcgcacggcaagaggcgaggggcggcgactggtgagtacgccaaaaattttgactagcggaggctagaaggagagagatgggtgcgagagcgtcagtattaagcgggggagaattagatcgcgatgggaaaaaattcggttaaggccagggggaaagaaaaaatataaataaacatatagtatgggcaagcagggagctagaacgattcgcagttaatcctggcctgttagaaacatcagaaggctgtagacaaatactgggacagctacaaccatcccttcagacaggatcagaagaacttagatcattatataatacagtagcaaccctctattgtgtgcatcaaaggatagagataaaagacaccaaggaagctttagacaagatagaggaagagcaaaacaaaagtaagaccaccgcacagcaagcggccggccgcgctgatcttcagacctggaggaggagatatgagggacaattggagaagtgaattatataaatataaagtagtaaaaattgaaccattaggagtagcacccaccaaggcaaagagaagagtggtgcagagagaaaaaagagcagtgggaataggagctttgttccttgggttcttgggagcagcaggaagcactatgggcgcagcgtcaatgacgctgacggtacaggccagacaattattgtctggtatagtgcagcagcagaacaatttgctgagggctattgaggcgcaacagcatctgttgcaactcacagtctggggcatcaagcagctccaggcaagaatcctggctgtggaaagatacctaaaggatcaacagctcctggggatttggggttgctctggaaaactcatttgcaccactgctgtgccttggaatgctagttggagtaataaatctctggaacagatttggaatcacacgacctggatggagtgggacagagaaattaacaattacacaagcttaatacactccttaattgaagaatcgcaaaaccagcaagaaaagaatgaacaagaattattggaattagataaatgggcaagtttgtggaattggtttaacataacaaattggctgtggtatataaaattattcataatgatagtaggaggcttggtaggtttaagaatagtttttgctgtactttctatagtgaatagagttaggcagggatattcaccattatcgtttcagacccacctcccaaccccgaggggacccgacaggcccgaaggaatagaagaagaaggtggagagagagacagagacagatccattcgattagtgaacggatcggcactgcgtgcgccaattctgcagacaaatggcagtattcatccacaattttaaaagaaaaggggggattggggggtacagtgcaggggaaagaatagtagacataatagcaacagacatacaaactaaagaattacaaaaacaaattacaaaaattcaaaattttcgggtttattacagggacagcagagatccagtttggttagtaccgggcccgctctagcgtcgaggagcttggcccattgcatacgttgtatccatatcataatatgtacatttatattggctcatgtccaacattaccgccatgttgacattgattattgactagttattaatagtaatcaattacggggtcattagttcatagcccatatatggagttccgcgttacataacttacggtaaatggcccgcctggctgaccgcccaacgacccccgcccattgacgtcaataatgacgtatgttcccatagtaacgccaatagggactttccattgacgtcaatgggtggagtatttacggtaaactgcccacttggcagtacatcaagtgtatcatatgccaagtacgccccctattgacgtcaatgacggtaaatggcccgcctggcattatgcccagtacatgaccttatgggactttcctacttggcagtacatctacgtattagtcatcgctattaccatggtgatgcggttttggcagtacatcaatgggcgtggatagcggtttgactcacggggatttccaagtctccaccccattgacgtcaatgggagtttgttttggcaccaaaatcaacgggactttccaaaatgtcgtaacaactccgccccattgacgcaaatgggcggtaggcgtgtacggtgggaggtctatataagcagagctcgtttagtgaaccgtcagatcgcctggagacgccatccacgctgttttgacctccatagaagacaccgggaccgatccagcctccgcggccccgaattcgccaccatggccagcgagttcaagaagaagctcttctggagggcagtggtggccgagttcctggccacgaccctctttgtcttcatcagcatcggttctgccctgggcttcaaatacccggtggggaacaaccagacggcggtccaggacaacgtgaaggtgtcgctggccttcgggctgagcatcgccacgctggcgcagagtgtgggccacatcagcggcgcccacctcaacccggctgtcacactggggctgctgctcagctgccagatcagcatcttccgtgccctcatgtacatcatcgcccagtgcgtgggggccatcgtcgccaccgccatcctctcaggcatcacctcctccctgactgggaactcgcttggccgcaatgacctggctgatggtgtgaactcgggccagggcctgggcatcgagatcatcgggaccctccagctggtgctatgcgtgctggctactaccgaccggaggcgccgtgaccttggtggctcagccccccttgccatcggcctctctgtagcccttggacacctcctggctattgactacactggctgtgggattaaccctgctcggtcctttggctccgcggtgatcacacacaacttcagcaaccactggattttctgggtggggccattcatcgggggagccctggctgtactcatctacgacttcatcctggccccacgcagcagtgacctcacagaccgcgtgaaggtgtggaccagcggccaggtggaggagtatgacctggatgccgacgacatcaactccagggtggagatgaagcccaaatacccatacgatgttccagattacgctggatccgctagcggcagtggagagggcagaggaagtctgctaacatgcggtgacgtcgaggagaatcctggcccagtgagcaagggcgaggagctgttcaccggggtggtgcccatcctggtcgagctggacggcgacgtaaacggccacaagttcagcgtgtccggcgagggcgagggcgatgccacctacggcaagctgaccctgaagttcatctgcaccaccggcaagctgcccgtgccctggcccaccctcgtgaccaccctgacctacggcgtgcagtgcttcagccgctaccccgaccacatgaagcagcacgacttcttcaagtccgccatgcccgaaggctacgtccaggagcgcaccatcttcttcaaggacgacggcaactacaagacccgcgccgaggtgaagttcgagggcgacaccctggtgaaccgcatcgagctgaagggcatcgacttcaaggaggacggcaacatcctggggcacaagctggagtacaactacaacagccacaacgtctatatcatggccgacaagcagaagaacggcatcaaggtgaacttcaagatccgccacaacatcgaggacggcagcgtgcagctcgccgaccactaccagcagaacacccccatcggcgacggccccgtgctgctgcccgacaaccactacctgagcacccagtccgccctgagcaaagaccccaacgagaagcgcgatcacatggtcctgctggagttcgtgaccgccgccgggatcactctcggcatggacgagctgtacaagtaaggatcctaggcggccgcgcatgccctgcaggtgatctatcgatcggccggcccctctccctccccccccccctaacgttactggccgaagccgcttggaataaggccggtgtgcgtttgtctatatgttattttccaccatattgccgtcttttggcaatgtgagggcccggaaacctggccctgtcttcttgacgagcattcctaggggtctttcccctctcgccaaaggaatgcaaggtctgttgaatgtcgtgaaggaagcagttcctctggaagcttcttgaagacaaacaacgtctgtagcgaccctttgcaggcagcggaaccccccacctggcgacaggtgcctctgcggccaaaagccacgtgtataagatacacctgcaaaggcggcacaaccccagtgccacgttgtgagttggatagttgtggaaagagtcaaatggctctcctcaagcgtattcaacaaggggctgaaggatgcccagaaggtaccccattgtatgggatctgatctggggcctcggtacacatgctttacatgtgtttagtcgaggttaaaaaaacgtctaggccccccgaaccacggggacgtggttttcctttgaaaaacacgatgataatatggccacaaccgggccggatatcacgcgtgatctgatcagcacgtgttgacaattaatcatcggcatagtatatcggcatagtataatacgacaaggtgaggaactaaaccatggccaagcctttgtctcaagaagaatccaccctcattgaaagagcaacggctacaatcaacagcatccccatctctgaagactacagcgtcgccagcgcagctctctctagcgacggccgcatcttcactggtgtcaatgtatatcattttactgggggaccttgtgcagaactcgtggtgctgggcactgctgctgctgcggcagctggcaacctgacttgtatcgtcgcgatcggaaatgagaacaggggcatcttgagcccctgcggacggtgccgacaggtgcttctcgatctgcatcctgggatcaaagccatagtgaaggacagtgatggacagccgacggcagttgggattcgtgaattgctgccctctggttatgtgtgggagggctaagcaatgcatacatgtgtttaaacctcgacttaattaagtcgagggtcgacggtatcgataagctcgcttcacgagatcatgtttaagggttccggttccactaggtacaattcgatatcaagcttatcgataatcaacctctggattacaaaatttgtgaaagattgactggtattcttaactatgttgctccttttacgctatgtggatacgctgctttaatgcctttgtatcatgctattgcttcccgtatggctttcattttctcctccttgtataaatcctggttgctgtctctttatgaggagttgtggcccgttgtcaggcaacgtggcgtggtgtgcactgtgtttgctgacgcaacccccactggttggggcattgccaccacctgtcagctcctttccgggactttcgctttccccctccctattgccacggcggaactcatcgccgcctgccttgcccgctgctggacaggggctcggctgttgggcactgacaattccgtggtgttgtcggggaaatcatcgtcctttccttggctgctcgcctgtgttgccacctggattctgcgcgggacgtccttctgctacgtcccttcggccctcaatccagcggaccttccttcccgcggcctgctgccggctctgcggcctcttccgcgtcttcgccttcgccctcagacgagtcggatctccctttgggccgcctccccgcatcgataccgtcgacctcgatcgagacctagaaaaacatggagcaatcacaagtagcaatacagcagctaccaatgctgattgtgcctggctagaagcacaagaggaggaggaggtgggttttccagtcacacctcaggtacctttaagaccaatgacttacaaggcagctgtagatcttagccactttttaaaagaaaaggggggactggaagggctaattcactcccaacgaagacaagatatccttgatctgtggatctaccacacacaaggctacttccctgattggcagaactacacaccagggccagggatcagatatccactgacctttggatggtgctacaagctagtaccagttgagcaagagaaggtagaagaagccaatgaaggagagaacacccgcttgttacaccctgtgagcctgcatgggatggatgacccggagagagaagtattagagtggaggtttgacagccgcctagcatttcatcacatggcccgagagctgcatccggactgtactgggtctctctggttagaccagatctgagcctgggagctctctggctaactagggaacccactgcttaagcctcaataaagcttgccttgagtgcttcaagtagtgtgtgcccgtctgttgtgtgactctggtaactagagatccctcagacccttttagtcagtgtggaaaatctctagcagcatgtgagcaaaaggccagcaaaaggccaggaaccgtaaaaaggccgcgttgctggcgtttttccataggctccgcccccctgacgagcatcacaaaaatcgacgctcaagtcagaggtggcgaaacccgacaggactataaagataccaggcgtttccccctggaagctccctcgtgcgctctcctgttccgaccctgccgcttaccggatacctgtccgcctttctcccttcgggaagcgtggcgctttctcatagctcacgctgtaggtatctcagttcggtgtaggtcgttcgctccaagctgggctgtgtgcacgaaccccccgttcagcccgaccgctgcgccttatccggtaactatcgtcttgagtccaacccggtaagacacgacttatcgccactggcagcagccactggtaacaggattagcagagcgaggtatgtaggcggtgctacagagttcttgaagtggtggcctaactacggctacactagaagaacagtatttggtatctgcgctctgctgaagccagttaccttcggaaaaagagttggtagctcttgatccggcaaacaaaccaccgctggtagcggtggtttttttgtttgcaagcagcagattacgcgcagaaaaaaaggatctcaagaagatcctttgatcttttctacggggtctgacgctcagtggaacgaaaactcacgttaagggattttggtcatgagattatcaaaaaggatcttcacctagatccttttaaattaaaaatgaagttttaaatcaatctaaagtatatatgagtaaacttggtctgacagttaccaatgcttaatcagtgaggcacctatctcagcgatctgtctatttcgttcatccatagttgcctgactccccgtcgtgtagataactacgatacgggagggcttaccatctggccccagtgctgcaatgataccgcgagacccacgctcaccggctccagatttatcagcaataaaccagccagccggaagggccgagcgcagaagtggtcctgcaactttatccgcctccatccagtctattaattgttgccgggaagctagagtaagtagttcgccagttaatagtttgcgcaacgttgttgccattgctacaggcatcgtggtgtcacgctcgtcgtttggtatggcttcattcagctccggttcccaacgatcaaggcgagttacatgatcccccatgttgtgcaaaaaagcggttagctccttcggtcctccgatcgttgtcagaagtaagttggccgcagtgttatcactcatggttatggcagcactgcataattctcttactgtcatgccatccgtaagatgcttttctgtgactggtgagtactcaaccaagtcattctgagaatagtgtatgcggcgaccgagttgctcttgcccggcgtcaatacgggataataccgcgccacatagcagaactttaaaagtgctcatcattggaaaacgttcttcggggcgaaaactctcaaggatcttaccgctgttgagatccagttcgatgtaacccactcgtgcacccaactgatcttcagcatcttttactttcaccagcgtttctgggtgagcaaaaacaggaaggcaaaatgccgcaaaaaagggaataagggcgacacggaaatgttgaatactcatactcttcctttttcaatattattgaagcatttatcagggttattgtctcatgagcggatacatatttgaatgtatttagaaaaataaacaaataggggttccgcgcacatttccccgaaaagtgccacctgac

SEQ ID NO: 17 - DNA, 7110 bp, synthetic construct
  source 1..7110: mol_type = other DNA
cctgcaggcagctgcgcgctcgctcgctcactgaggccgcccgggcgtcgggcgacctttggtcgcccggcctcagtgagcgagcgagcgcgcagagagggagtggccaactccatcactaggggttcctgcggcctctagactcgaggcgttgacattgattattgactagttattaatagtaatcaattacggggtcattagttcatagcccatatatggagttccgcgttacataacttacggtaaatggcccgcctggctgaccgcccaacgacccccgcccattgacgtcaataatgacgtatgttcccatagtaacgccaatagggactttccattgacgtcaatgggtggagtatttacggtaaactgcccacttggcagtacatcaagtgtatcatatgccaagtacgccccctattgacgtcaatgacggtaaatggcccgcctggcattatgcccagtacatgaccttatgggactttcctacttggcagtacatctacgtattagtcatcgctattaccatggtgatgcggttttggcagtacatcaatgggcgtggatagcggtttgactcacggggatttccaagtctccaccccattgacgtcaatgggagtttgttttggcaccaaaatcaacgggactttccaaaatgtcgtaacaactccgccccattgacgcaaatgggcggtaggcgtgtacggtgggaggtctatataagcagagctctctggctaactaccggtgccaccatgagccccaagaagaagagaaaggtggaggccagcatcgaaaaaaaaaagtccttcgccaagggcatgggcgtgaagtccacactcgtgtccggctccaaagtgtacatgacaaccttcgccgaaggcagcgacgccaggctggaaaagatcgtggagggcgacagcatcaggagcgtgaatgagggcgaggccttcagcgctgaaatggccgataaaaacgccggctataagatcggcaacgccaaattcagccatcctaagggctacgccgtggtggctaacaaccctctgtatacaggacccgtccagcaggatatgctcggcctgaaggaaactctggaaaagaggtacttcggcgagagcgctgatggcaatgacaatatttgtatccaggtgatccataacatcctggacattgaaaaaatcctcgccgaatacattaccaacgccgcctacgccgtcaacaatatctccggcctggataaggacattattggattcggcaagttctccacagtgtatacctacgacgaattcaaagaccccgagcaccatagggccgctttcaacaataacgataagctcatcaacgccatcaaggcccagtatgacgagttcgacaacttcctcgataaccccagactcggctatttcggccaggcctttttcagcaaggagggcagaaattacatcatcaattacggcaacgaatgctatgacattctggccctcctgagcggactgaggcactgggtggtccataacaacgaagaagagtccaggatctccaggacctggctctacaacctcgataagaacctcgacaacgaatacatctccaccctcaactacctctacgacaggatcaccaatgagctgaccaactccttctccaagaactccgccgccaacgtgaactatattgccgaaactctgggaatcaaccctgccgaattcgccgaacaatatttcagattcagcattatgaaagagcagaaaaacctcggattcaatatcaccaagctcagggaagtgatgctggacaggaaggatatgtccgagatcaggaaaaatcataaggtgttcgactccatcaggaccaaggtctacaccatgatggactttgtgatttataggtattacatcgaagaggatgccaaggtggctgccgccaataagtccctccccgataatgagaagtccctgagcgagaaggatatctttgtgattaacctgaggggctccttcaacgacgaccagaaggatgccctctactacgatgaagctaatagaatttggagaaagctcgaaaatatcatgcacaacatcaaggaatttaggggaaacaagacaagagagtataagaagaaggacgcccctagactgcccagaatcctgcccgctggccgtgatgtttccgccttcagcaaactcatgtatgccctgaccatgttcctggatggcaaggagatcaacgacctcctgaccaccctgattaataaattcgataacatccagagcttcctgaaggtgatgcctctcatcggagtcaacgctaagttcgtggaggaatacgcctttttcaaagactccgccaagatcgccgatgagctgaggctgatcaagtccttcgctagaatgggagaacctattgccgatgccaggagggccatgtatatcgacgccatccgtattttaggaaccaacctgtcctatgatgagctcaaggccctcgccgacaccttttccctggacgagaacggaaacaagctcaagaaaggcaagcacggcatgagaaatttcattattaataacgtgatcagcaataaaaggttccactacctgatcagatacggtgatcctgcccacctccatgagatcgccaaaaacgaggccgtggtgaagttcgtgctcggcaggatcgctgacatccagaaaaaacagggccagaacggcaagaaccagatcgacaggtactacgaaacttgtatcggaaaggataagggcaagagcgtgagcgaaaaggtggacgctctcacaaagatcatcaccggaatgaactacgaccaattcgacaagaaaaggagcgtcattgaggacaccggcagggaaaacgccgagagggagaagtttaaaaagatcatcagcctgtacctcaccgtgatctaccacatcctcaagaatattgtcaatatcaacgccaggtacgtcatcggattccattgcgtcgagcgtgatgctcaactgtacaaggagaaaggctacgacatcaatctcaagaaactggaagagaagggattcagctccgtcaccaagctctgcgctggcattgatgaaactgcccccgataagagaaaggacgtggaaaaggagatggctgaaagagccaaggagagcattgacagcctcgagagcgccaaccccaagctgtatgccaattacatcaaatacagcgacgagaagaaagccgaggagttcaccaggcagattaacagggagaaggccaaaaccgccctgaacgcctacctgaggaacaccaagtggaatgtgatcatcagggaggacctcctgagaattgacaacaagacatgtaccctgttcagaaacaaggccgtccacctggaagtggccaggtatgtccacgcctatatcaacgacattgccgaggtcaattcctacttccaactgtaccattacatcatgcagagaattatcatgaatgagaggtacgagaaaagcagcggaaaggtgtccgagtacttcgacgctgtgaatgacgagaagaagtacaacgataggctcctgaaactgctgtgtgtgcctttcggctactgtatccccaggtttaagaacctgagcatcgaggccctgttcgataggaacgaggccgccaagttcgacaaggagaaaaagaaggtgtccggcaattccggatccggacctaagaaaaagaggaaggtggcggccgcttacccatacgatgttccagattacgcttgaggtaccctagagctcgctgatcagcctcgactgtgccttctagttgccagccatctgttgtttgcccctcccccgtgccttccttgaccctggaaggtgccactcccactgtcctttcctaataaaatgaggaaattgcatcgcattgtctgagtaggtgtcattctattctggggggtggggtggggcaggacagcaagggggaggattgggaagagaatagcaggcatgctggggagagggcctatttcccatgattccttcatatttgcatatacgatacaaggctgttagagagataattggaattaatttgactgtaaacacaaagatattagtacaaaatacgtgacgtagaaagtaataatttcttgggtagtttgcagttttaaaattatgttttaaaatggactatcatatgcttaccgtaacttgaaagtatttcgatttcttggctttatatatcttgtggaaaggacgaaacaccgcaagtaaacccctaccaactggtcggggtttgaaacagggcagaaccgatgctgatgaagaccaagtaaacccctaccaactggtcggggtttgaaactttttttcccgggaatggccgcaggaacccctagtgatggagttggccactccctctctgcgcgctcgctcgctcactgaggccgggcgaccaaaggtcgcccgacgcccgggctttgcccgggcggcctcagtgagcgagcgagcgcgcagctgcctgcaggggcgcctgatgcggtattttctccttacgcatctgtgcggtatttcacaccgcatacgtcaaagcaaccatagtacgcgccctgtagcggcgcattaagcgcggcgggtgtggtggttacgcgcagcgtgaccgctacacttgccagcgccctagcgcccgctcctttcgctttcttcccttcctttctcgccacgttcgccggctttccccgtcaagctctaaatcgggggctccctttagggttccgatttagtgctttacggcacctcgaccccaaaaaacttgatttgggtgatggttcacgtagtgggccatcgccctgatagacggtttttcgccctttgacgttggagtccacgttctttaatagtggactcttgttccaaactggaacaacactcaaccctatctcgggctattcttttgatttataagggattttgccgatttcggcctattggttaaaaaatgagctgatttaacaaaaatttaacgcgaattttaacaaaatattaacgtttacaattttatggtgcactctcagtacaatctgctctgatgccgcatagttaagccagccccgacacccgccaacacccgctgacgcgccctgacgggcttgtctgctcccggcatccgcttacagacaagctgtgaccgtctccgggagctgcatgtgtcagaggttttcaccgtcatcaccgaaacgcgcgagacgaaagggcctcgtgatacgcctatttttataggttaatgtcatgataataatggtttcttagacgtcaggtggcacttttcggggaaatgtgcgcggaacccctatttgtttatttttctaaatacattcaaatatgtatccgctcatgagacaataaccctgataaatgcttcaataatattgaaaaaggaagagtatgagtattcaacatttccgtgtcgcccttattcccttttttgcggcattttgccttcctgtttttgctcacccagaaacgctggtgaaagtaaaagatgctgaagatcagttgggtgcacgagtgggttacatcgaactggatctcaacagcggtaagatccttgagagttttcgccccgaagaacgttttccaatgatgagcacttttaaagttctgctatgtggcgcggtattatcccgtattgacgccgggcaagagcaactcggtcgccgcatacactattctcagaatgacttggttgagtactcaccagtcacagaaaagcatcttacggatggcatgacagtaagagaattatgcagtgctgccataaccatgagtgataacactgcggccaacttacttctgacaacgatcggaggaccgaaggagctaaccgcttttttgcacaacatgggggatcatgtaactcgccttgatcgttgggaaccggagctgaatgaagccataccaaacgacgagcgtgacaccacgatgcctgtagcaatggcaacaacgttgcgcaaactattaactggcgaactacttactctagcttcccggcaacaattaatagactggatggaggcggataaagttgcaggaccacttctgcgctcggcccttccggctggctggtttattgctgataaatctggagccggtgagcgtggaagccgcggtatcattgcagcactggggccagatggtaagccctcccgtatcgtagttatctacacgacggggagtcaggcaactatggatgaacgaaatagacagatcgctgagataggtgcctcactgattaagcattggtaactgtcagaccaagtttactcatatatactttagattgatttaaaacttcatttttaatttaaaaggatctaggtgaagatcctttttgataatctcatgaccaaaatcccttaacgtgagttttcgttccactgagcgtcagaccccgtagaaaagatcaaaggatcttcttgagatcctttttttctgcgcgtaatctgctgcttgcaaacaaaaaaaccaccgctaccagcggtggtttgtttgccggatcaagagctaccaactctttttccgaaggtaactggcttcagcagagcgcagataccaaatactgtccttctagtgtagccgtagttaggccaccacttcaagaactctgtagcaccgcctacatacctcgctctgctaatcctgttaccagtggctgctgccagtggcgataagtcgtgtcttaccgggttggactcaagacgatagttaccggataaggcgcagcggtcgggctgaacggggggttcgtgcacacagcccagcttggagcgaacgacctacaccgaactgagatacctacagcgtgagctatgagaaagcgccacgcttcccgaagggagaaaggcggacaggtatccggtaagcggcagggtcggaacaggagagcgcacgagggagcttccagggggaaacgcctggtatctttatagtcctgtcgggtttcgccacctctgacttgagcgtcgatttttgtgatgctcgtcaggggggcggagcctatggaaaaacgccagcaacgcggcctttttacggttcctggccttttgctggccttttgctcacatgt

SEQ ID NO: 18 - DNA, 7114 bp, synthetic construct
  source 1..7114: mol_type = other DNA
cctgcaggcagctgcgcgctcgctcgctcactgaggccgcccgggcgtcgggcgacctttggtcgcccggcctcagtgagcgagcgagcgcgcagagagggagtggccaactccatcactaggggttcctgcggcctctagactcgaggcgttgacattgattattgactagttattaatagtaatcaattacggggtcattagttcatagcccatatatggagttccgcgttacataacttacggtaaatggcccgcctggctgaccgcccaacgacccccgcccattgacgtcaataatgacgtatgttcccatagtaacgccaatagggactttccattgacgtcaatgggtggagtatttacggtaaactgcccacttggcagtacatcaagtgtatcatatgccaagtacgccccctattgacgtcaatgacggtaaatggcccgcctggcattatgcccagtacatgaccttatgggactttcctacttggcagtacatctacgtattagtcatcgctattaccatggtgatgcggttttggcagtacatcaatgggcgtggatagcggtttgactcacggggatttccaagtctccaccccattgacgtcaatgggagtttgttttggcaccaaaatcaacgggactttccaaaatgtcgtaacaactccgccccattgacgcaaatgggcggtaggcgtgtacggtgggaggtctatataagcagagctctctggctaactaccggtgccaccatgagccccaagaagaagagaaaggtggaggccagcatcgaaaaaaaaaagtccttcgccaagggcatgggcgtgaagtccacactcgtgtccggctccaaagtgtacatgacaaccttcgccgaaggcagcgacgccaggctggaaaagatcgtggagggcgacagcatcaggagcgtgaatgagggcgaggccttcagcgctgaaatggccgataaaaacgccggctataagatcggcaacgccaaattcagccatcctaagggctacgccgtggtggctaacaaccctctgtatacaggacccgtccagcaggatatgctcggcctgaaggaaactctggaaaagaggtacttcggcgagagcgctgatggcaatgacaatatttgtatccaggtgatccataacatcctggacattgaaaaaatcctcgccgaatacattaccaacgccgcctacgccgtcaacaatatctccggcctggataaggacattattggattcggcaagttctccacagtgtatacctacgacgaattcaaagaccccgagcaccatagggccgctttcaacaataacgataagctcatcaacgccatcaaggcccagtatgacgagttcgacaacttcctcgataaccccagactcggctatttcggccaggcctttttcagcaaggagggcagaaattacatcatcaattacggcaacgaatgctatgacattctggccctcctgagcggactgaggcactgggtggtccataacaacgaagaagagtccaggatctccaggacctggctctacaacctcgataagaacctcgacaacgaatacatctccaccctcaactacctctacgacaggatcaccaatgagctgaccaactccttctccaagaactccgccgccaacgtgaactatattgccgaaactctgggaatcaaccctgccgaattcgccgaacaatatttcagattcagcattatgaaagagcagaaaaacctcggattcaatatcaccaagctcagggaagtgatgctggacaggaaggatatgtccgagatcaggaaaaatcataaggtgttcgactccatcaggaccaaggtctacaccatgatggactttgtgatttataggtattacatcgaagaggatgccaaggtggctgccgccaataagtccctccccgataatgagaagtccctgagcgagaaggatatctttgtgattaacctgaggggctccttcaacgacgaccagaaggatgccctctactacgatgaagctaatagaatttggagaaagctcgaaaatatcatgcacaacatcaaggaatttaggggaaacaagacaagagagtataagaagaaggacgcccctagactgcccagaatcctgcccgctggccgtgatgtttccgccttcagcaaactcatgtatgccctgaccatgttcctggatggcaaggagatcaacgacctcctgaccaccctgattaataaattcgataacatccagagcttcctgaaggtgatgcctctcatcggagtcaacgctaagttcgtggaggaatacgcctttttcaaagactccgccaagatcgccgatgagctgaggctgatcaagtccttcgctagaatgggagaacctattgccgatgccaggagggccatgtatatcgacgccatccgtattttaggaaccaacctgtcctatgatgagctcaaggccctcgccgacaccttttccctggacgagaacggaaacaagctcaagaaaggcaagcacggcatgagaaatttcattattaataacgtgatcagcaataaaaggttccactacctgatcagatacggtgatcctgcccacctccatgagatcgccaaaaacgaggccgtggtgaagttcgtgctcggcaggatcgctgacatccagaaaaaacagggccagaacggcaagaaccagatcgacaggtactacgaaacttgtatcggaaaggataagggcaagagcgtgagcgaaaaggtggacgctctcacaaagatcatcaccggaatgaactacgaccaattcgacaagaaaaggagcgtcattgaggacaccggcagggaaaacgccgagagggagaagtttaaaaagatcatcagcctgtacctcaccgtgatctaccacatcctcaagaatattgtcaatatcaacgccaggtacgtcatcggattccattgcgtcgagcgtgatgctcaactgtacaaggagaaaggctacgacatcaatctcaagaaactggaagagaagggattcagctccgtcaccaagctctgcgctggcattgatgaaactgcccccgataagagaaaggacgtggaaaaggagatggctgaaagagccaaggagagcattgacagcctcgagagcgccaaccccaagctgtatgccaattacatcaaatacagcgacgagaagaaagccgaggagttcaccaggcagattaacagggagaaggccaaaaccgccctgaacgcctacctgaggaacaccaagtggaatgtgatcatcagggaggacctcctgagaattgacaacaagacatgtaccctgttcagaaacaaggccgtccacctggaagtggccaggtatgtccacgcctatatcaacgacattgccgaggtcaattcctacttccaactgtaccattacatcatgcagagaattatcatgaatgagaggtacgagaaaagcagcggaaaggtgtccgagtacttcgacgctgtgaatgacgagaagaagtacaacgataggctcctgaaactgctgtgtgtgcctttcggctactgtatccccaggtttaagaacctgagcatcgaggccctgttcgataggaacgaggccgccaagttcgacaaggagaaaaagaaggtgtccggcaattccggatccggacctaagaaaaagaggaaggtggcggccgcttacccatacgatgttccagattacgcttgaggtaccctagagctcgctgatcagcctcgactgtgccttctagttgccagccatctgttgtttgcccctcccccgtgccttccttgaccctggaaggtgccactcccactgtcctttcctaataaaatgaggaaattgcatcgcattgtctgagtaggtgtcattctattctggggggtggggtggggcaggacagcaagggggaggattgggaagagaatagcaggcatgctggggagagggcctatttcccatgattccttcatatttgcatatacgatacaaggctgttagagagataattggaattaatttgactgtaaacacaaagatattagtacaaaatacgtgacgtagaaagtaataatttcttgggtagtttgcagttttaaaattatgttttaaaatggactatcatatgcttaccgtaacttgaaagtatttcgatttcttggctttatatatcttgtggaaaggacgaaacaccgcaagtaaacccctaccaactggtcggggtttgaaacgtggttggagaactggatgtagatgggctgcaagtaaacccctaccaactggtcggggtttgaaactttttttcccgggaatggccgcaggaacccctagtgatggagttggccactccctctctgcgcgctcgctcgctcactgaggccgggcgaccaaaggtcgcccgacgcccgggctttgcccgggcggcctcagtgagcgagcgagcgcgcagctgcctgcaggggcgcctgatgcggtattttctccttacgcatctgtgcggtatttcacaccgcatacgtcaaagcaaccatagtacgcgccctgtagcggcgcattaagcgcggcgggtgtggtggttacgcgcagcgtgaccgctacacttgccagcgccctagcgcccgctcctttcgctttcttcccttcctttctcgccacgttcgccggctttccccgtcaagctctaaatcgggggctccctttagggttccgatttagtgctttacggcacctcgaccccaaaaaacttgatttgggtgatggttcacgtagtgggccatcgccctgatagacggtttttcgccctttgacgttggagtccacgttctttaatagtggactcttgttccaaactggaacaacactcaaccctatctcgggctattcttttgatttataagggattttgccgatttcggcctattggttaaaaaatgagctgatttaacaaaaatttaacgcgaattttaacaaaatattaacgtttacaattttatggtgcactctcagtacaatctgctctgatgccgcatagttaagccagccccgacacccgccaacacccgctgacgcgccctgacgggcttgtctgctcccggcatccgcttacagacaagctgtgaccgtctccgggagctgcatgtgtcagaggttttcaccgtcatcaccgaaacgcgcgagacgaaagggcctcgtgatacgcctatttttataggttaatgtcatgataataatggtttcttagacgtcaggtggcacttttcggggaaatgtgcgcggaacccctatttgtttatttttctaaatacattcaaatatgtatccgctcatgagacaataaccctgataaatgcttcaataatattgaaaaaggaagagtatgagtattcaacatttccgtgtcgcccttattcccttttttgcggcattttgccttcctgtttttgctcacccagaaacgctggtgaaagtaaaagatgctgaagatcagttgggtgcacgagtgggttacatcgaactggatctcaacagcggtaagatccttgagagttttcgccccgaagaacgttttccaatgatgagcacttttaaagttctgctatgtggcgcggtattatcccgtattgacgccgggcaagagcaactcggtcgccgcatacactattctcagaatgacttggttgagtactcaccagtcacagaaaagcatcttacggatggcatgacagtaagagaattatgcagtgctgccataaccatgagtgataacactgcggccaacttacttctgacaacgatcggaggaccgaaggagctaaccgcttttttgcacaacatgggggatcatgtaactcgccttgatcgttgggaaccggagctgaatgaagccataccaaacgacgagcgtgacaccacgatgcctgtagcaatggcaacaacgttgcgcaaactattaactggcgaactacttactctagcttcccggcaacaattaatagactggatggaggcggataaagttgcaggaccacttctgcgctcggcccttccggctggctggtttattgctgataaatctggagccggtgagcgtggaagccgcggtatcattgcagcactggggccagatggtaagccctcccgtatcgtagttatctacacgacggggagtcaggcaactatggatgaacgaaatagacagatcgctgagataggtgcctcactgattaagcattggtaactgtcagaccaagtttactcatatatactttagattgatttaaaacttcatttttaatttaaaaggatctaggtgaagatcctttttgataatctcatgaccaaaatcccttaacgtgagttttcgttccactgagcgtcagaccccgtagaaaagatcaaaggatcttcttgagatcctttttttctgcgcgtaatctgctgcttgcaaacaaaaaaaccaccgctaccagcggtggtttgtttgccggatcaagagctaccaactctttttccgaaggtaactggcttcagcagagcgcagataccaaatactgtccttctagtgtagccgtagttaggccaccacttcaagaactctgtagcaccgcctacatacctcgctctgctaatcctgttaccagtggctgctgccagtggcgataagtcgtgtcttaccgggttggactcaagacgatagttaccggataaggcgcagcggtcgggctgaacggggggttcgtgcacacagcccagcttggagcgaacgacctacaccgaactgagatacctacagcgtgagctatgagaaagcgccacgcttcccgaagggagaaaggcggacaggtatccggtaagcggcagggtcggaacaggagagcgcacgagggagcttccagggggaaacgcctggtatctttatagtcctgtcgggtttcgccacctctgacttgagcgtcgatttttgtgatgctcgtcaggggggcggagcctatggaaaaacgccagcaacgcggcctttttacggttcctggccttttgctggccttttgctcacatgt

SEQ ID NO: 19 - DNA, 4780 bp, synthetic construct
  source 1..4780: mol_type = other DNA
cctgcaggcagctgcgcgctcgctcgctcactgaggccgcccgggcgtcgggcgacctttggtcgcccggcctcagtgagcgagcgagcgcgcagagagggagtggccaactccatcactaggggttcctgcggcctctagactcgaggcgttgacattgattattgactagttattaatagtaatcaattacggggtcattagttcatagcccatatatggagttccgcgttacataacttacggtaaatggcccgcctggctgaccgcccaacgacccccgcccattgacgtcaataatgacgtatgttcccatagtaacgccaatagggactttccattgacgtcaatgggtggagtatttacggtaaactgcccacttggcagtacatcaagtgtatcatatgccaagtacgccccctattgacgtcaatgacggtaaatggcccgcctggcattatgcccagtacatgaccttatgggactttcctacttggcagtacatctacgtattagtcatcgctattaccatggtgatgcggttttggcagtacatcaatgggcgtggatagcggtttgactcacggggatttccaagtctccaccccattgacgtcaatgggagtttgttttggcaccaaaatcaacgggactttccaaaatgtcgtaacaactccgccccattgacgcaaatgggcggtaggcgtgtacggtgggaggtctatataagcagagctctctggctaactaccggtgccaccatggtgagcaagggcgaggagctgttcaccggggtggtgcccatcctggtcgagctggacggcgacgtaaacggccacaagttcagcgtgtccggcgagggcgagggcgatgccacctacggcaagctgaccctgaagttcatctgcaccaccggcaagctgcccgtgccctggcccaccctcgtgaccaccctgacctacggcgtgcagtgcttcagccgctaccccgaccacatgaagcagcacgacttcttcaagtccgccatgcccgaaggctacgtccaggagcgcaccatcttcttcaaggacgacggcaactacaagacccgcgccgaggtgaagttcgagggcgacaccctggtgaaccgcatcgagctgaagggcatcgacttcaaggaggacggcaacatcctggggcacaagctggagtacaactacaacagccacaacgtctatatcatggccgacaagcagaagaacggcatcaaggtgaacttcaagatccgccacaacatcgaggacggcagcgtgcagctcgccgaccactaccagcagaacacccccatcggcgacggccccgtgctgctgcccgacaaccactacctgagcacccagtccgccctgagcaaagaccccaacgagaagcgcgatcacatggtcctgctggagttcgtgaccgccgccgggatcactctcggcatggacgagctgtacaagtaaagcggccgaattcctagagctcgctgatcagcctcgactgtgccttctagttgccagccatctgttgtttgcccctcccccgtgccttccttgaccctggaaggtgccactcccactgtcctttcctaataaaatgaggaaattgcatcgcattgtctgagtaggtgtcattctattctggggggtggggtggggcaggacagcaagggggaggattgggaagagaatagcaggcatgctggggaggtaccgagggcctatttcccatgattccttcatatttgcatatacgatacaaggctgttagagagataattggaattaatttgactgtaaacacaaagatattagtacaaaatacgtgacgtagaaagtaataatttcttgggtagtttgcagttttaaaattatgttttaaaatggactatcatatgcttaccgtaacttgaaagtatttcgatttcttggctttatatatcttgtggaaaggacgaaacaccgccacgaccctctttgtcttcactcgagtgaagacaaagagggtcgtggttttttggccgcaggaacccctagtgatggagttggccactccctctctgcgcgctcgctcgctcactgaggccgggcgaccaaaggtcgcccgacgcccgggctttgcccgggcggcctcagtgagcgagcgagcgcgcagctgcctgcaggggcgcctgatgcggtattttctccttacgcatctgtgcggtatttcacaccgcatacgtcaaagcaaccatagtacgcgccctgtagcggcgcattaagcgcggcgggtgtggtggttacgcgcagcgtgaccgctacacttgccagcgccctagcgcccgctcctttcgctttcttcccttcctttctcgccacgttcgccggctttccccgtcaagctctaaatcgggggctccctttagggttccgatttagtgctttacggcacctcgaccccaaaaaacttgatttgggtgatggttcacgtagtgggccatcgccctgatagacggtttttcgccctttgacgttggagtccacgttctttaatagtggactcttgttccaaactggaacaacactcaaccctatctcgggctattcttttgatttataagggattttgccgatttcggcctattggttaaaaaatgagctgatttaacaaaaatttaacgcgaattttaacaaaatattaacgtttacaattttatggtgcactctcagtacaatctgctctgatgccgcatagttaagccagccccgacacccgccaacacccgctgacgcgccctgacgggcttgtctgctcccggcatccgcttacagacaagctgtgaccgtctccgggagctgcatgtgtcagaggttttcaccgtcatcaccgaaacgcgcgagacgaaagggcctcgtgatacgcctatttttataggttaatgtcatgataataatggtttcttagacgtcaggtggcacttttcggggaaatgtgcgcggaacccctatttgtttatttttctaaatacattcaaatatgtatccgctcatgagacaataaccctgataaatgcttcaataatattgaaaaaggaagagtatgagtattcaacatttccgtgtcgcccttattcccttttttgcggcattttgccttcctgtttttgctcacccagaaacgctggtgaaagtaaaagatgctgaagatcagttgggtgcacgagtgggttacatcgaactggatctcaacagcggtaagatccttgagagttttcgccccgaagaacgttttccaatgatgagcacttttaaagttctgctatgtggcgcggtattatcccgtattgacgccgggcaagagcaactcggtcgccgcatacactattctcagaatgacttggttgagtactcaccagtcacagaaaagcatcttacggatggcatgacagtaagagaattatgcagtgctgccataaccatgagtgataacactgcggccaacttacttctgacaacgatcggaggaccgaaggagctaaccgcttttttgcacaacatgggggatcatgtaactcgccttgatcgttgggaaccggagctgaatgaagccataccaaacgacgagcgtgacaccacgatgcctgtagcaatggcaacaacgttgcgcaaactattaactggcgaactacttactctagcttcccggcaacaattaatagactggatggaggcggataaagttgcaggaccacttctgcgctcggcccttccggctggctggtttattgctgataaatctggagccggtgagcgtggaagccgcggtatcattgcagcactggggccagatggtaagccctcccgtatcgtagttatctacacgacggggagtcaggcaactatggatgaacgaaatagacagatcgctgagataggtgcctcactgattaagcattggtaactgtcagaccaagtttactcatatatactttagattgatttaaaacttcatttttaatttaaaaggatctaggtgaagatcctttttgataatctcatgaccaaaatcccttaacgtgagttttcgttccactgagcgtcagaccccgtagaaaagatcaaaggatcttcttgagatcctttttttctgcgcgtaatctgctgcttgcaaacaaaaaaaccaccgctaccagcggtggtttgtttgccggatcaagagctaccaactctttttccgaaggtaactggcttcagcagagcgcagataccaaatactgtccttctagtgtagccgtagttaggccaccacttcaagaactctgtagcaccgcctacatacctcgctctgctaatcctgttaccagtggctgctgccagtggcgataagtcgtgtcttaccgggttggactcaagacgatagttaccggataaggcgcagcggtcgggctgaacggggggttcgtgcacacagcccagcttggagcgaacgacctacaccgaactgagatacctacagcgtgagctatgagaaagcgccacgcttcccgaagggagaaaggcggacaggtatccggtaagcggcagggtcggaacaggagagcgcacgagggagcttccagggggaaacgcctggtatctttatagtcctgtcgggtttcgccacctctgacttgagcgtcgatttttgtgatgctcgtcaggggggcggagcctatggaaaaacgccagcaacgcggcctttttacggttcctggccttttgctggccttttgctcacatgt

SEQ ID NO: 20 - DNA, 4780 bp, synthetic construct
  source 1..4780: mol_type = other DNA
cctgcaggcagctgcgcgctcgctcgctcactgaggccgcccgggcgtcgggcgacctttggtcgcccggcctcagtgagcgagcgagcgcgcagagagggagtggccaactccatcactaggggttcctgcggcctctagactcgaggcgttgacattgattattgactagttattaatagtaatcaattacggggtcattagttcatagcccatatatggagttccgcgttacataacttacggtaaatggcccgcctggctgaccgcccaacgacccccgcccattgacgtcaataatgacgtatgttcccatagtaacgccaatagggactttccattgacgtcaatgggtggagtatttacggtaaactgcccacttggcagtacatcaagtgtatcatatgccaagtacgccccctattgacgtcaatgacggtaaatggcccgcctggcattatgcccagtacatgaccttatgggactttcctacttggcagtacatctacgtattagtcatcgctattaccatggtgatgcggttttggcagtacatcaatgggcgtggatagcggtttgactcacggggatttccaagtctccaccccattgacgtcaatgggagtttgttttggcaccaaaatcaacgggactttccaaaatgtcgtaacaactccgccccattgacgcaaatgggcggtaggcgtgtacggtgggaggtctatataagcagagctctctggctaactaccggtgccaccatggtgagcaagggcgaggagctgttcaccggggtggtgcccatcctggtcgagctggacggcgacgtaaacggccacaagttcagcgtgtccggcgagggcgagggcgatgccacctacggcaagctgaccctgaagttcatctgcaccaccggcaagctgcccgtgccctggcccaccctcgtgaccaccctgacctacggcgtgcagtgcttcagccgctaccccgaccacatgaagcagcacgacttcttcaagtccgccatgcccgaaggctacgtccaggagcgcaccatcttcttcaaggacgacggcaactacaagacccgcgccgaggtgaagttcgagggcgacaccctggtgaaccgcatcgagctgaagggcatcgacttcaaggaggacggcaacatcctggggcacaagctggagtacaactacaacagccacaacgtctatatcatggccgacaagcagaagaacggcatcaaggtgaacttcaagatccgccacaacatcgaggacggcagcgtgcagctcgccgaccactaccagcagaacacccccatcggcgacggccccgtgctgctgcccgacaaccactacctgagcacccagtccgccctgagcaaagaccccaacgagaagcgcgatcacatggtcctgctggagttcgtgaccgccgccgggatcactctcggcatggacgagctgtacaagtaaagcggccgaattcctagagctcgctgatcagcctcgactgtgccttctagttgccagccatctgttgtttgcccctcccccgtgccttccttgaccctggaaggtgccactcccactgtcctttcctaataaaatgaggaaattgcatcgcattgtctgagtaggtgtcattctattctggggggtggggtggggcaggacagcaagggggaggattgggaagagaatagcaggcatgctggggaggtaccgagggcctatttcccatgattccttcatatttgcatatacgatacaaggctgttagagagataattggaattaatttgactgtaaacacaaagatattagtacaaaatacgtgacgtagaaagtaataatttcttgggtagtttgcagttttaaaattatgttttaaaatggactatcatatgcttaccgtaacttgaaagtatttcgatttcttggctttatatatcttgtggaaaggacgaaacaccgcagcccatctacatccagttcctcgaggaactggatgtagatgggctgttttttggccgcaggaacccctagtgatggagttggccactccctctctgcgcgctcgctcgctcactgaggccgggcgaccaaaggtcgcccgacgcccgggctttgcccgggcggcctcagtgagcgagcgagcgcgcagctgcctgcaggggcgcctgatgcggtattttctccttacgcatctgtgcggtatttcacaccgcatacgtcaaagcaaccatagtacgcgccctgtagcggcgcattaagcgcggcgggtgtggtggttacgcgcagcgtgaccgctacacttgccagcgccctagcgcccgctcctttcgctttcttcccttcctttctcgccacgttcgccggctttccccgtcaagctctaaatcgggggctccctttagggttccgatttagtgctttacggcacctcgaccccaaaaaacttgatttgggtgatggttcacgtagtgggccatcgccctgatagacggtttttcgccctttgacgttggagtccacgttctttaatagtggactcttgttccaaactggaacaacactcaaccctatctcgggctattcttttgatttataagggattttgccgatttcggcctattggttaaaaaatgagctgatttaacaaaaatttaacgcgaattttaacaaaatattaacgtttacaattttatggtgcactctcagtacaatctgctctgatgccgcatagttaagccagccccgacacccgccaacacccgctgacgcgccctgacgggcttgtctgctcccggcatccgcttacagacaagctgtgaccgtctccgggagctgcatgtgtcagaggttttcaccgtcatcaccgaaacgcgcgagacgaaagggcctcgtgatacgcctatttttataggttaatgtcatgataataatggtttcttagacgtcaggtggcacttttcggggaaatgtgcgcggaacccctatttgtttatttttctaaatacattcaaatatgtatccgctcatgagacaataaccctgataaatgcttcaataatattgaaaaaggaagagtatgagtattcaacatttccgtgtcgcccttattcccttttttgcggcattttgccttcctgtttttgctcacccagaaacgctggtgaaagtaaaagatgctgaagatcagttgggtgcacgagtgggttacatcgaactggatctcaacagcggtaagatccttgagagttttcgccccgaagaacgttttccaatgatgagcacttttaaagttctgctatgtggcgcggtattatcccgtattgacgccgggcaagagcaactcggtcgccgcatacactattctcagaatgacttggttgagtactcaccagtcacagaaaagcatcttacggatggcatgacagtaagagaattatgcagtgctgccataaccatgagtgataacactgcggccaacttacttctgacaacgatcggaggaccgaaggagctaaccgcttttttgcacaacatgggggatcatgtaactcgccttgatcgttgggaaccggagctgaatgaagccataccaaacgacgagcgtgacaccacgatgcctgtagcaatggcaacaacgttgcgcaaactattaactggcgaactacttactctagcttcccggcaacaattaatagactggatggaggcggataaagttgcaggaccacttctgcgctcggcccttccggctggctggtttattgctgataaatctggagccggtgagcgtggaagccgcggtatcattgcagcactggggccagatggtaagccctcccgtatcgtagttatctacacgacggggagtcaggcaactatggatgaacgaaatagacagatcgctgagataggtgcctcactgattaagcattggtaactgtcagaccaagtttactcatatatactttagattgatttaaaacttcatttttaatttaaaaggatctaggtgaagatcctttttgataatctcatgaccaaaatcccttaacgtgagttttcgttccactgagcgtcagaccccgtagaaaagatcaaaggatcttcttgagatcctttttttctgcgcgtaatctgctgcttgcaaacaaaaaaaccaccgctaccagcggtggtttgtttgccggatcaagagctaccaactctttttccgaaggtaactggcttcagcagagcgcagataccaaatactgtccttctagtgtagccgtagttaggccaccacttcaagaactctgtagcaccgcctacatacctcgctctgctaatcctgttaccagtggctgctgccagtggcgataagtcgtgtcttaccgggttggactcaagacgatagttaccggataaggcgcagcggtcgggctgaacggggggttcgtgcacacagcccagcttggagcgaacgacctacaccgaactgagatacctacagcgtgagctatgagaaagcgccacgcttcccgaagggagaaaggcggacaggtatccggtaagcggcagggtcggaacaggagagcgcacgagggagcttccagggggaaacgcctggtatctttatagtcctgtcgggtttcgccacctctgacttgagcgtcgatttttgtgatgctcgtcaggggggcggagcctatggaaaaacgccagcaacgcggcctttttacggttcctggccttttgctggccttttgctcacatgt

SEQ ID NO: 21 - DNA, 7108 bp, synthetic construct
  source 1..7108: mol_type = other DNA
cctgcaggcagctgcgcgctcgctcgctcactgaggccgcccgggcgtcgggcgacctttggtcgcccggcctcagtgagcgagcgagcgcgcagagagggagtggccaactccatcactaggggttcctgcggcctctagactcgaggcgttgacattgattattgactagttattaatagtaatcaattacggggtcattagttcatagcccatatatggagttccgcgttacataacttacggtaaatggcccgcctggctgaccgcccaacgacccccgcccattgacgtcaataatgacgtatgttcccatagtaacgccaatagggactttccattgacgtcaatgggtggagtatttacggtaaactgcccacttggcagtacatcaagtgtatcatatgccaagtacgccccctattgacgtcaatgacggtaaatggcccgcctggcattatgcccagtacatgaccttatgggactttcctacttggcagtacatctacgtattagtcatcgctattaccatggtgatgcggttttggcagtacatcaatgggcgtggatagcggtttgactcacggggatttccaagtctccaccccattgacgtcaatgggagtttgttttggcaccaaaatcaacgggactttccaaaatgtcgtaacaactccgccccattgacgcaaatgggcggtaggcgtgtacggtgggaggtctatataagcagagctctctggctaactaccggtgccaccatgagccccaagaagaagagaaaggtggaggccagcatcgaaaaaaaaaagtccttcgccaagggcatgggcgtgaagtccacactcgtgtccggctccaaagtgtacatgacaaccttcgccgaaggcagcgacgccaggctggaaaagatcgtggagggcgacagcatcaggagcgtgaatgagggcgaggccttcagcgctgaaatggccgataaaaacgccggctataagatcggcaacgccaaattcagccatcctaagggctacgccgtggtggctaacaaccctctgtatacaggacccgtccagcaggatatgctcggcctgaaggaaactctggaaaagaggtacttcggcgagagcgctgatggcaatgacaatatttgtatccaggtgatccataacatcctggacattgaaaaaatcctcgccgaatacattaccaacgccgcctacgccgtcaacaatatctccggcctggataaggacattattggattcggcaagttctccacagtgtatacctacgacgaattcaaagaccccgagcaccatagggccgctttcaacaataacgataagctcatcaacgccatcaaggcccagtatgacgagttcgacaacttcctcgataaccccagactcggctatttcggccaggcctttttcagcaaggagggcagaaattacatcatcaattacggcaacgaatgctatgacattctggccctcctgagcggactgaggcactgggtggtccataacaacgaagaagagtccaggatctccaggacctggctctacaacctcgataagaacctcgacaacgaatacatctccaccctcaactacctctacgacaggatcaccaatgagctgaccaactccttctccaagaactccgccgccaacgtgaactatattgccgaaactctgggaatcaaccctgccgaattcgccgaacaatatttcagattcagcattatgaaagagcagaaaaacctcggattcaatatcaccaagctcagggaagtgatgctggacaggaaggatatgtccgagatcaggaaaaatcataaggtgttcgactccatcaggaccaaggtctacaccatgatggactttgtgatttataggtattacatcgaagaggatgccaaggtggctgccgccaataagtccctccccgataatgagaagtccctgagcgagaaggatatctttgtgattaacctgaggggctccttcaacgacgaccagaaggatgccctctactacgatgaagctaatagaatttggagaaagctcgaaaatatcatgcacaacatcaaggaatttaggggaaacaagacaagagagtataagaagaaggacgcccctagactgcccagaatcctgcccgctggccgtgatgtttccgccttcagcaaactcatgtatgccctgaccatgttcctggatggcaaggagatcaacgacctcctgaccaccctgattaataaattcgataacatccagagcttcctgaaggtgatgcctctcatcggagtcaacgctaagttcgtggaggaatacgcctttttcaaagactccgccaagatcgccgatgagctgaggctgatcaagtccttcgctagaatgggagaacctattgccgatgccaggagggccatgtatatcgacgccatccgtattttaggaaccaacctgtcctatgatgagctcaaggccctcgccgacaccttttccctggacgagaacggaaacaagctcaagaaaggcaagcacggcatgagaaatttcattattaataacgtgatcagcaataaaaggttccactacctgatcagatacggtgatcctgcccacctccatgagatcgccaaaaacgaggccgtggtgaagttcgtgctcggcaggatcgctgacatccagaaaaaacagggccagaacggcaagaaccagatcgacaggtactacgaaacttgtatcggaaaggataagggcaagagcgtgagcgaaaaggtggacgctctcacaaagatcatcaccggaatgaactacgaccaattcgacaagaaaaggagcgtcattgaggacaccggcagggaaaacgccgagagggagaagtttaaaaagatcatcagcctgtacctcaccgtgatctaccacatcctcaagaatattgtcaatatcaacgccaggtacgtcatcggattccattgcgtcgagcgtgatgctcaactgtacaaggagaaaggctacgacatcaatctcaagaaactggaagagaagggattcagctccgtcaccaagctctgcgctggcattgatgaaactgcccccgataagagaaaggacgtggaaaaggagatggctgaaagagccaaggagagcattgacagcctcgagagcgccaaccccaagctgtatgccaattacatcaaatacagcgacgagaagaaagccgaggagttcaccaggcagattaacagggagaaggccaaaaccgccctgaacgcctacctgaggaacaccaagtggaatgtgatcatcagggaggacctcctgagaattgacaacaagacatgtaccctgttcagaaacaaggccgtccacctggaagtggccaggtatgtccacgcctatatcaacgacattgccgaggtcaattcctacttccaactgtaccattacatcatgcagagaattatcatgaatgagaggtacgagaaaagcagcggaaaggtgtccgagtacttcgacgctgtgaatgacgagaagaagtacaacgataggctcctgaaactgctgtgtgtgcctttcggctactgtatccccaggtttaagaacctgagcatcgaggccctgttcgataggaacgaggccgccaagttcgacaaggagaaaaagaaggtgtccggcaattccggatccggacctaagaaaaagaggaaggtggcggccgcttacccatacgatgttccagattacgcttgaggtaccctagagctcgctgatcagcctcgactgtgccttctagttgccagccatctgttgtttgcccctcccccgtgccttccttgaccctggaaggtgccactcccactgtcctttcctaataaaatgaggaaattgcatcgcattgtctgagtaggtgtcattctattctggggggtggggtggggcaggacagcaagggggaggattgggaagagaatagcaggcatgctggggagagggcctatttcccatgattccttcatatttgcatatacgatacaaggctgttagagagataattggaattaatttgactgtaaacacaaagatattagtacaaaatacgtgacgtagaaagtaataatttcttgggtagtttgcagttttaaaattatgttttaaaatggactatcatatgcttaccgtaacttgaaagtatttcgatttcttggctttatatatcttgtggaaaggacgaaacaccgcaagtaaacccctaccaactggtcggggtttgaaacgatcaacattaaatgtgagcgagtcaagtaaacccctaccaactggtcggggtttgaaactttttttcccgggaatggccgcaggaacccctagtgatggagttggccactccctctctgcgcgctcgctcgctcactgaggccgggcgaccaaaggtcgcccgacgcccgggctttgcccgggcggcctcagtgagcgagcgagcgcgcagctgcctgcaggggcgcctgatgcggtattttctccttacgcatctgtgcggtatttcacaccgcatacgtcaaagcaaccatagtacgcgccctgtagcggcgcattaagcgcggcgggtgtggtggttacgcgcagcgtgaccgctacacttgccagcgccctagcgcccgctcctttcgctttcttcccttcctttctcgccacgttcgccggctttccccgtcaagctctaaatcgggggctccctttagggttccgatttagtgctttacggcacctcgaccccaaaaaacttgatttgggtgatggttcacgtagtgggccatcgccctgatagacggtttttcgccctttgacgttggagtccacgttctttaatagtggactcttgttccaaactggaacaacactcaaccctatctcgggctattcttttgatttataagggattttgccgatttcggcctattggttaaaaaatgagctgatttaacaaaaatttaacgcgaattttaacaaaatattaacgtttacaattttatggtgcactctcagtacaatctgctctgatgccgcatagttaagccagccccgacacccgccaacacccgctgacgcgccctgacgggcttgtctgctcccggcatccgcttacagacaagctgtgaccgtctccgggagctgcatgtgtcagaggttttcaccgtcatcaccgaaacgcgcgagacgaaagggcctcgtgatacgcctatttttataggttaatgtcatgataataatggtttcttagacgtcaggtggcacttttcggggaaatgtgcgcggaacccctatttgtttatttttctaaatacattcaaatatgtatccgctcatgagacaataaccctgataaatgcttcaataatattgaaaaaggaagagtatgagtattcaacatttccgtgtcgcccttattcccttttttgcggcattttgccttcctgtttttgctcacccagaaacgctggtgaaagtaaaagatgctgaagatcagttgggtgcacgagtgggttacatcgaactggatctcaacagcggtaagatccttgagagttttcgccccgaagaacgttttccaatgatgagcacttttaaagttctgctatgtggcgcggtattatcccgtattgacgccgggcaagagcaactcggtcgccgcatacactattctcagaatgacttggttgagtactcaccagtcacagaaaagcatcttacggatggcatgacagtaagagaattatgcagtgctgccataaccatgagtgataacactgcggccaacttacttctgacaacgatcggaggaccgaaggagctaaccgcttttttgcacaacatgggggatcatgtaactcgccttgatcgttgggaaccggagctgaatgaagccataccaaacgacgagcgtgacaccacgatgcctgtagcaatggcaacaacgttgcgcaaactattaactggcgaactacttactctagcttcccggcaacaattaatagactggatggaggcggataaagttgcaggaccacttctgcgctcggcccttccggctggctggtttattgctgataaatctggagccggtgagcgtggaagccgcggtatcattgcagcactggggccagatggtaagccctcccgtatcgtagttatctacacgacggggagtcaggcaactatggatgaacgaaatagacagatcgctgagataggtgcctcactgattaagcattggtaactgtcagaccaagtttactcatatatactttagattgatttaaaacttcatttttaatttaaaaggatctaggtgaagatcctttttgataatctcatgaccaaaatcccttaacgtgagttttcgttccactgagcgtcagaccccgtagaaaagatcaaaggatcttcttgagatcctttttttctgcgcgtaatctgctgcttgcaaacaaaaaaaccaccgctaccagcggtggtttgtttgccggatcaagagctaccaactctttttccgaaggtaactggcttcagcagagcgcagataccaaatactgtccttctagtgtagccgtagttaggccaccacttcaagaactctgtagcaccgcctacatacctcgctctgctaatcctgttaccagtggctgctgccagtggcgataagtcgtgtcttaccgggttggactcaagacgatagttaccggataaggcgcagcggtcgggctgaacggggggttcgtgcacacagcccagcttggagcgaacgacctacaccgaactgagatacctacagcgtgagctatgagaaagcgccacgcttcccgaagggagaaaggcggacaggtatccggtaagcggcagggtcggaacaggagagcgcacgagggagcttccagggggaaacgcctggtatctttatagtcctgtcgggtttcgccacctctgacttgagcgtcgatttttgtgatgctcgtcaggggggcggagcctatggaaaaacgccagcaacgcggcctttttacggttcctggccttttgctggccttttgctcacatgt

SEQ ID NO: 22 - DNA, 34 bp, synthetic construct
  source 1..34: mol_type = other DNA
agacgtggttggagaactggatgtagatgggctg

SEQ ID NO: 23 - DNA, 34 bp, synthetic construct
  source 1..34: mol_type = other DNA
aaaacagcccatctacatccagttctccaaccac

SEQ ID NO: 24 - DNA, 30 bp, synthetic construct
  source 1..30: mol_type = other DNA
agacagggcagaaccgatgctgatgaagac

SEQ ID NO: 25 - DNA, 30 bp, synthetic construct
  source 1..30: mol_type = other DNA
aaaagtcttcatcagcatcggttctgccct

SEQ ID NO: 26 - DNA, 22 bp, synthetic construct
  source 1..22: mol_type = other DNA
attgtcccagatatagccgttg

SEQ ID NO: 27 - DNA, 20 bp, synthetic construct
  source 1..20: mol_type = other DNA
gctgtcatttccgtttgctg

SEQ ID NO: 28 - DNA, 20 bp, synthetic construct
  source 1..20: mol_type = other DNA
gctcttctggagggcagtgg

SEQ ID NO: 29 - DNA, 21 bp, synthetic construct
  source 1..21: mol_type = other DNA
cagtgtgacagccgggttgag

SEQ ID NO: 30 - DNA, 20 bp, synthetic construct
  source 1..20: mol_type = other DNA
ccatggggaaggtgaaggtc

SEQ ID NO: 31 - DNA, 21 bp, synthetic construct
  source 1..21: mol_type = other DNA
gaaggggtcattgatggcaac

SEQ ID NO: 32 - protein, 928 aa, synthetic construct
MSKDKKTKAKRMGVKALLAHGEDKLTMTTFGKGNRSKIEFTEGYHGRALETPKHFGKRGFEVRKIDENVDLYGDLEEGKTIEALLINPSEKVGEDYLKLKGTLEKRFFGREFPHDNIRIQLIYNILDIYKILGMNVADILYALGNMQDTELDIDMFGQSLNNPEKAKDVVQRMKPYMGFFGGIFRTQKKEDRKKDSNLSEEEKEEKKKKQEELLQKDLQHNMDVARCISALRHATAHNKPATAHDKQDEYPWFKSSDIYETKIFKAGMWSVIEADYKKKIQDVNKQFFSKNKVNLAILFDLLDVRDVKQKKRISDEFYRFTIRKDGKNLGMNLVKIREIIIDRYASGLRDKKHDPHRQKINVIADFLIFRALSQNQGIIDKTVSSLRLTKDEEEKDHVYQNAAELVWGMVSNCLTPYFNDPKNKYILKYKDAKTPGDFEDWITSKISEDDGEPFVKVLSFLCNFLEGKEINELLTAYIHKFECIQDFLNVISSLGENVQFQPRFALFNNASFAQNVAVQLRILASIGKMKPDLTEAKRPLYKAAIRMLCPPEKWEKYTSDEWLEKNMLLNSEDRKNDKKKKQVNPFRNFIAGNVIESRRFMYLVRYSKPKAVRAIMQNRSIVNYVLHRLPSEQIKTYSRVFPEDFSDTEAEIDFLVNKLSEFSFETFISNQQTILNNSKRGFSPNRRETAEEIERLKAITGLYLSVAYIAIKNIVKANARYYIAFAVFERDKELVKAKDARIQTTIPNTKFTNYFCLTQYYLDRDEEKKFPGDPRDKEAFFEHLRKTKRHFSKQWREWLNEKIADAKSSQATGLLLREARNDVEHLNVLRAIPDYIQDFRHGEKGETAMNSYFELYHYLMQRLMLKNTELDLSHWSGWIMRSGRPDRDLIQIAFVSLAYNLPRYRNLTKEHHFDDTVLQKIREKESLD

SEQ ID NO: 33 - RNA, 36 nt, synthetic construct
  source 1..36: mol_type = other RNA
ggtcaacagtgtggggaattacccgcactctacaac

SEQ ID NO: 34 - protein, 891 aa, synthetic construct
MSKDKKTKAKRMGVKALLAHGEDKLTMTTFGKGNRSQIEFTEGYHGRALETPKRFGKRGFEVRKIDENVDLYGDLDEGKTIEALLVNPSENVGEDYLKLKSTLENYFFGREFPHDNIRIQLIYNILDIYKILGMNVADILYTLGNLQDAEGDIDLFGKSLNNEDNIKESLNRMRPYMGYFGEVFKKDNREHNKKVLRCISALRNATAHGKQDEYPWFKSSDIYEKTIFKADKWRIIEDQYREKIRKVNNEFFSKNKVNLAILFDLLHARDVEPKKQIADEFYRFTIRKDGKNLGMNLVKIREKIIDRFARDLRDKKHDPHRQKIHVIADFLIFRALSQNQEVIDKTVSRLRLTKDEEEKDRVYQNAAELVWGMVSNCLSPYFKDPKKYIIQYKSGGKIKIFDDWITSKISAKDGEPFVKVLSFLCNFLEGKEINELLTAYIHKFECIQDFLKVISSLGERAQFQPRFDLFNKPDFAQNVAVQLRILASIGKMKPDLTEAKRPLYKAAIQMLCPPEKWEKYTSDEWLEENMLLNSEDRQNKEKREKVNPFRNFIAGNVIESRRFMYLVRYSKPKAVRALMKNRSVVNYVLHRLPPEQIKTYSRVFPDDFNDTEAEIDFLVNKLSEFSFETFITSRQTILANSKRGFSPNRRETAEEIERLKAITGLYLSVAYIAIKNIVKANARYYIAFAVFERDKELVKAKDARIQTTIPNTTYTNYFCLTQYYLDRDEEKKFQGDPRDKEAFFEHLRKKKTHFSKQWREWLNEKIADAKSAQETGLLLTEARNDVEHLNVLRAIPDYIQDFRHGDKGETPMNSYFELYHYLLQRLMLKNRLLDLSSWRSWIERSGRPDRDLIQIAFVSLAYNLPRYRNLTKEHHFDDTVLQKIRERKSLD

SEQ ID NO: 35 - RNA, 34 nt, synthetic construct
  source 1..34: mol_type = other RNA
agtctcagaaccctacaggtttgtagagttatct

SEQ ID NO: 36 - DNA, 6898 bp, synthetic construct
  source 1..6898: mol_type = other DNA
cctgcaggcagctgcgcgctcgctcgctcactgaggccgcccgggcgtcgggcgacctttggtcgcccggcctcagtgagcgagcgagcgcgcagagagggagtggccaactccatcactaggggttcctgcggcctctagactcgaggcgttgacattgattattgactagttattaatagtaatcaattacggggtcattagttcatagcccatatatggagttccgcgttacataacttacggtaaatggcccgcctggctgaccgcccaacgacccccgcccattgacgtcaataatgacgtatgttcccatagtaacgccaatagggactttccattgacgtcaatgggtggagtatttacggtaaactgcccacttggcagtacatcaagtgtatcatatgccaagtacgccccctattgacgtcaatgacggtaaatggcccgcctggcattatgcccagtacatgaccttatgggactttcctacttggcagtacatctacgtattagtcatcgctattaccatggtgatgcggttttggcagtacatcaatgggcgtggatagcggtttgactcacggggatttccaagtctccaccccattgacgtcaatgggagtttgttttggcaccaaaatcaacgggactttccaaaatgtcgtaacaactccgccccattgacgcaaatgggcggtaggcgtgtacggtgggaggtctatataagcagagctctctggctaactaccggtgccaccatgccggcagctaagaaaaagaaactggatggcagcgtcgacatgagcaaggataagaaaaccaaagccaagaggatgggtgtgaaagccctgctggcccacggagaggacaagctgacaatgaccacattcggaaagggcaatagatccaaaatcgagttcacagagggataccacggcagggccctggaaacccccaagcactttggcaagaggggattcgaggtccggaagatcgatgagaatgttgacctgtacggggacctcgaggagggcaaaaccattgaagccctgctcattaatcctagcgagaaggtgggcgaggactacctcaagctgaaggggactctcgagaaacggttttttgggcgcgaatttccacatgacaatatcagaatccagctgatctacaacatcctggacatctacaaaatactgggcatgaacgtcgccgacatcctgtacgctctgggcaatatgcaggacacagagctggacattgatatgttcggccagtctctgaataatcctgagaaggccaaagatgtggtgcagaggatgaagccttacatgggcttttttggcggcatcttcagaacccagaagaaggaggaccggaagaaggacagcaatctcagcgaggaggagaaggaggagaagaagaagaagcaggaagagctgctgcagaaggacctgcagcacaacatggatgtcgccagatgtattagcgcactgagacatgccaccgcccacaataagccagccactgcccacgataagcaggacgaatacccctggttcaagagcagcgacatttatgagacaaagattttcaaagcaggcatgtggtcagtgatcgaggctgattataagaagaagatccaggatgttaataaacagttcttcagcaagaataaggtgaacctggccatcctctttgacctgctggacgtacgtgatgtgaagcaaaaaaagcggatcagcgatgagttctaccgttttaccatcaggaaggacgggaaaaacctgggcatgaatctcgtgaaaattagagagatcattatcgaccgctacgccagcgggctgcgcgataagaaacatgatccccacagacagaaaatcaacgtaattgcagacttcctgattttccgggccctgtcacagaaccaggggatcatagataagactgtgtctagtctgcggctgaccaaggacgaggaggagaaggaccatgtgtatcagaatgcagccgaactggtgtgggggatggtgtccaactgcctgaccccatacttcaatgatcccaagaataaatacatcctgaaatacaaagacgccaagactcccggggatttcgaggattggatcaccagcaaaatcagtgaggacgatggggagccttttgtgaaggtgctgagctttctgtgtaatttcttagagggaaaggaaattaacgagctgcttaccgcctacatccataaattcgaatgtatccaggattttctgaacgtgatatcttcactgggcgagaacgtccagtttcagcccagatttgccctgtttaataatgctagcttcgctcagaacgttgccgtccagctgaggattttggccagcatcggcaagatgaagcctgatctgaccgaggccaaaaggcccctgtacaaagcagccatcagaatgctgtgcccccccgagaagtgggagaagtacaccagtgatgaatggctggagaagaacatgctgctgaatagcgaggacagaaagaacgacaagaaaaagaaacaggtgaaccctttcaggaattttattgcagggaacgttatcgagtctcgccgctttatgtatctggtgaggtacagcaagccaaaggccgtgcgggccatcatgcagaacaggtcaatcgtgaactacgtgctccaccggctgccttcagagcagatcaaaacttactcccgtgtgttccccgaggacttctccgacaccgaggccgaaatcgactttctcgtgaataaactgagtgaattttcatttgaaaccttcatctccaaccagcagacaattctgaacaactccaagagaggctttagccccaatagacgggaaacggccgaggagattgaacggctgaaggccattaccggcctgtacctctcagtggcctatatcgccatcaaaaacatcgtgaaggccaacgctaggtactatattgcattcgccgtgttcgaaagagataaggagctggtgaaagccaaggacgcccgcatacagaccactatccctaacacaaaatttactaactatttttgtctgactcagtactatctggaccgcgacgaagagaagaagtttcctggcgacccccgcgacaaggaggccttctttgaacatctgaggaaaactaagcggcactttagtaaacagtggagagagtggctgaacgagaagatcgccgacgccaagagcagccaggccaccgggctgctgctgcgggaggcaagaaatgatgtggaacacctgaatgtgctgagagctatccccgactacatccaggactttcgccacggagagaagggcgagacagccatgaatagctacttcgagctgtatcactacctgatgcagaggctgatgcttaagaacaccgagctggacctgagccactggagcggctggatcatgaggtccggtcgacctgacagggatctgatacagattgctttcgtgtccctggcatacaatctgccacggtacagaaatctgaccaaagagcatcacttcgatgacaccgtgcttcagaagatcagggagaaagagagcctggatacaggcggcggccccggcggcggcgccgccgccggcagcggcagccctaagaaaaaacgaaaagttggcagcggaagcaaaaggccggcggccacgaaaaaggccggccaggcaaaaaagaaaaagctcgagtacccatacgatgttccagattacgcttgagaattccccttgagcatctgacttctggctaataaaggaaatttattttcattgcaatagtgtgttggaattttttgtgtctctcaggtaccgagggcctatttcccatgattccttcatatttgcatatacgatacaaggctgttagagagataattggaattaatttgactgtaaacacaaagatattagtacaaaatacgtgacgtagaaagtaataatttcttgggtagtttgcagttttaaaattatgttttaaaatggactatcatatgcttaccgtaacttgaaagtatttcgatttcttggctttatatatcttgtggaaaggacgaaacaccggtcaacagtgtggggaattacccgcactctacaacggagaccacggcaggtctcattttttgcggccgcaggaacccctagtgatggagttggccactccctctctgcgcgctcgctcgctcactgaggccgggcgaccaaaggtcgcccgacgcccgggctttgcccgggcggcctcagtgagcgagcgagcgcgcagctgcctgcaggggcgcctgatgcggtattttctccttacgcatctgtgcggtatttcacaccgcatacgtcaaagcaaccatagtacgcgccctgtagcggcgcattaagcgcggcgggtgtggtggttacgcgcagcgtgaccgctacacttgccagcgccttagcgcccgctcctttcgctttcttcccttcctttctcgccacgttcgccggctttccccgtcaagctctaaatcgggggctccctttagggttccgatttagtgctttacggcacctcgaccccaaaaaacttgatttgggtgatggttcacgtagtgggccatcgccctgatagacggtttttcgccctttgacgttggagtccacgttctttaatagtggactcttgttccaaactggaacaacactcaactctatctcgggctattcttttgatttataagggattttgccgatttcggtctattggttaaaaaatgagctgatttaacaaaaatttaacgcgaattttaacaaaatattaacgtttacaattttatggtgcactctcagtacaatctgctctgatgccgcatagttaagccagccccgacacccgccaacacccgctgacgcgccctgacgggcttgtctgctcccggcatccgcttacagacaagctgtgaccgtctccgggagctgcatgtgtcagaggttttcaccgtcatcaccgaaacgcgcgagacgaaagggcctcgtgatacgcctatttttataggttaatgtcatgataataatggtttcttagacgtcaggtggcacttttcggggaaatgtgcgcggaacccctatttgtttatttttctaaatacattcaaatatgtatccgctcatgagacaataaccctgataaatgcttcaataatattgaaaaaggaagagtatgagtattcaacatttccgtgtcgcccttattcccttttttgcggcattttgccttcctgtttttgctcacccagaaacgctggtgaaagtaaaagatgctgaagatcagttgggtgcacgagtgggttacatcgaactggatctcaacagcggtaagatccttgagagttttcgccccgaagaacgttttccaatgatgagcacttttaaagttctgctatgtggcgcggtattatcccgtattgacgccgggcaagagcaactcggtcgccgcatacactattctcagaatgacttggttgagtactcaccagtcacagaaaagcatcttacggatggcatgacagtaagagaattatgcagtgctgccataaccatgagtgataacactgcggccaacttacttctgacaacgatcggaggaccgaaggagctaaccgcttttttgcacaacatgggggatcatgtaactcgccttgatcgttgggaaccggagctgaatgaagccataccaaacgacgagcgtgacaccacgatgcctgtagcaatggcaacaacgttgcgcaaactattaactggcgaactacttactctagcttcccggcaacaattaatagactggatggaggcggataaagttgcaggaccacttctgcgctcggcccttccggctggctggtttattgctgataaatctggagccggtgagcgtggaagccgcggtatcattgcagcactggggccagatggtaagccctcccgtatcgtagttatctacacgacggggagtcaggcaactatggatgaacgaaatagacagatcgctgagataggtgcctcactgattaagcattggtaactgtcagaccaagtttactcatatatactttagattgatttaaaacttcatttttaatttaaaaggatctaggtgaagatcctttttgataatctcatgaccaaaatcccttaacgtgagttttcgttccactgagcgtcagaccccgtagaaaagatcaaaggatcttcttgagatcctttttttctgcgcgtaatctgctgcttgcaaacaaaaaaaccaccgctaccagcggtggtttgtttgccggatcaagagctaccaactctttttccgaaggtaactggcttcagcagagcgcagataccaaatactgttcttctagtgtagccgtagttaggccaccacttcaagaactctgtagcaccgcctacatacctcgctctgctaatcctgttaccagtggctgctgccagtggcgataagtcgtgtcttaccgggttggactcaagacgatagttaccggataaggcgcagcggtcgggctgaacggggggttcgtgcacacagcccagcttggagcgaacgacctacaccgaactgagatacctacagcgtgagctatgagaaagcgccacgcttcccgaagggagaaaggcggacaggtatccggtaagcggcagggtcggaacaggagagcgcacgagggagcttccagggggaaacgcctggtatctttatagtcctgtcgggtttcgccacctctgacttgagcgtcgatttttgtgatgctcgtcaggggggcggagcctatggaaaaacgccagcaacgcggcctttttacggttcctggccttttgctggccttttgctcacatgt

SEQ ID NO: 37 - DNA, 6786 bp, synthetic construct
  source 1..6786: mol_type = other DNA
cctgcaggcagctgcgcgctcgctcgctcactgaggccgcccgggcgtcgggcgacctttggtcgcccggcctcagtgagcgagcgagcgcgcagagagggagtggccaactccatcactaggggttcctgcggcctctagactcgaggcgttgacattgattattgactagttattaatagtaatcaattacggggtcattagttcatagcccatatatggagttccgcgttacataacttacggtaaatggcccgcctggctgaccgcccaacgacccccgcccattgacgtcaataatgacgtatgttcccatagtaacgccaatagggactttccattgacgtcaatgggtggagtatttacggtaaactgcccacttggcagtacatcaagtgtatcatatgccaagtacgccccctattgacgtcaatgacggtaaatggcccgcctggcattatgcccagtacatgaccttatgggactttcctacttggcagtacatctacgtattagtcatcgctattaccatggtgatgcggttttggcagtacatcaatgggcgtggatagcggtttgactcacggggatttccaagtctccaccccattgacgtcaatgggagtttgttttggcaccaaaatcaacgggactttccaaaatgtcgtaacaactccgccccattgacgcaaatgggcggtaggcgtgtacggtgggaggtctatataagcagagctctctggctaactaccggtgccaccatgccggcagctaagaaaaagaaactggatggcagcgtcgacatgtccaaggacaagaaaaccaaggccaagcggatgggcgtgaaagcactgctggcccatggcgaggataagctcaccatgaccacttttggtaagggaaataggtcccagatcgagtttacagaaggctatcacggccgagccctggagacacccaaaagattcggcaagagggggtttgaggtgagaaagatcgatgaaaacgtcgacctgtatggtgacctggacgagggcaagactattgaggccctgctggtgaacccctccgagaacgttggagaggactatctgaaactgaaaagcacactggagaactattttttcggtcgcgagttccctcatgacaatatccgcatccagctgatctacaacatcttggatatctataagatcctggggatgaacgtggctgacatcctctacaccctgggcaatctgcaggacgctgaaggagatatcgatctgttcgggaagtccctcaacaacgaggacaacattaaagaaagtctgaatagaatgaggccctacatgggctactttggggaggtgtttaaaaaggacaatagagaacataacaagaaagtgctccggtgcatctccgctctgcgcaacgccacagcccacggcaaacaggatgaatatccttggttcaagagcagcgatatctatgaaaagactatcttcaaagccgacaagtggcggatcatcgaggaccagtacagagaaaagattaggaaggtgaacaacgagtttttcagcaaaaacaaagtcaatctggctatcctcttcgatcttctgcacgccagagatgtggaacctaagaaacagattgccgatgaattttacaggttcaccatcagaaaggatggcaaaaatctggggatgaacctggtgaagatcagggagaaaatcatcgatcggtttgcccgcgatctgcgagacaagaaacacgacccacacagacagaaaattcacgtgatcgccgatttcctgattttcagggccctgagtcagaatcaggaagtgatcgacaaaacagtcagccggctgaggctgaccaaggatgaagaggagaaagatagagtgtaccagaacgccgccgagctcgtgtggggaatggtgtccaactgtctgagcccatatttcaaagaccctaagaaatacatcatccagtataagtccggcggaaaaatcaaaatcttcgacgactggatcacctctaagatttccgccaaagatggcgagccatttgtgaaggtgctgtcctttctctgcaatttcctggagggcaaggagatcaacgagctgctgaccgcctacatccacaagttcgagtgcatccaggattttctgaaagtcatttccagcctgggcgagagggcccagtttcagcctcggttcgatctgttcaataagcctgactttgcacagaacgtggccgtgcagctgcgcatcctcgccagtattgggaaaatgaagcccgatctgactgaggccaaaaggcctctctacaaagctgccatccagatgctctgccctcctgagaaatgggagaaatacacaagcgacgagtggctggaggagaacatgctgctgaactccgaggataggcagaataaggagaagcgagagaaggtcaatccctttcggaatttcatcgccggcaatgtgattgagagccgccgatttatgtacctcgtgaggtactccaagcccaaggcagttcgggctctgatgaaaaatagatcagtggtgaactacgtgctgcacaggctgcctccagagcagatcaagacctactccagggtgttccctgatgacttcaatgatactgaagctgagatcgatttcctggtgaacaagctcagcgaattttccttcgagacattcatcaccagcagacagaccattctggcaaattccaagagggggttttctcctaaccggcgggagacagccgaggagatcgaaaggctgaaagccatcacaggcctgtacctcagcgtggcctacattgctatcaaaaatatcgtgaaagcaaatgcccgatactacatagccttcgccgtgttcgagcgggacaaggagctcgtgaaagccaaggacgccaggatacagactaccatccccaatacaacctacactaattacttctgcctgactcagtactacctggaccgtgacgaggagaaaaagtttcagggcgaccctcgggataaggaggctttctttgaacatctccgtaagaagaaaacacactttagcaagcagtggcgggagtggctgaatgagaagatcgctgatgccaagtccgcccaggaaaccggcctgctgctgaccgaggccaggaatgacgtggaacacctgaatgtgctgcgggccattcccgattatatccaggacttcaggcacggagataagggggaaactcctatgaacagctacttcgagctgtatcattacctgctgcagaggctcatgctgaaaaatcggctgctcgacctgtctagctggcgctcctggatcgagaggtctggccgacctgatcgcgacctgattcagatcgcatttgtgagcctggcttataatctgcctagatatcggaatctgaccaaggagcaccactttgatgataccgtgctgcagaagattagagaaaggaagagcctggacacaggcggcggccccggcggcggcgccgccgccggcagcggcagccctaagaaaaaacgaaaagttggcagcggaagcaaaaggccggcggccacgaaaaaggccggccaggcaaaaaagaaaaagctcgagtacccatacgatgttccagattacgcttgagaattccccttgagcatctgacttctggctaataaaggaaatttattttcattgcaatagtgtgttggaattttttgtgtctctcaggtaccgagggcctatttcccatgattccttcatatttgcatatacgatacaaggctgttagagagataattggaattaatttgactgtaaacacaaagatattagtacaaaatacgtgacgtagaaagtaataatttcttgggtagtttgcagttttaaaattatgttttaaaatggactatcatatgcttaccgtaacttgaaagtatttcgatttcttggctttatatatcttgtggaaaggacgaaacaccgagtctcagaaccctacaggtttgtagagttatctggagaccacggcaggtctcattttttgcggccgcaggaacccctagtgatggagttggccactccctctctgcgcgctcgctcgctcactgaggccgggcgaccaaaggtcgcccgacgcccgggctttgcccgggcggcctcagtgagcgagcgagcgcgcagctgcctgcaggggcgcctgatgcggtattttctccttacgcatctgtgcggtatttcacaccgcatacgtcaaagcaaccatagtacgcgccctgtagcggcgcattaagcgcggcgggtgtggtggttacgcgcagcgtgaccgctacacttgccagcgccttagcgcccgctcctttcgctttcttcccttcctttctcgccacgttcgccggctttccccgtcaagctctaaatcgggggctccctttagggttccgatttagtgctttacggcacctcgaccccaaaaaacttgatttgggtgatggttcacgtagtgggccatcgccctgatagacggtttttcgccctttgacgttggagtccacgttctttaatagtggactcttgttccaaactggaacaacactcaactctatctcgggctattcttttgatttataagggattttgccgatttcggtctattggttaaaaaatgagctgatttaacaaaaatttaacgcgaattttaacaaaatattaacgtttacaattttatggtgcactctcagtacaatctgctctgatgccgcatagttaagccagccccgacacccgccaacacccgctgacgcgccctgacgggcttgtctgctcccggcatccgcttacagacaagctgtgaccgtctccgggagctgcatgtgtcagaggttttcaccgtcatcaccgaaacgcgcgagacgaaagggcctcgtgatacgcctatttttataggttaatgtcatgataataatggtttcttagacgtcaggtggcacttttcggggaaatgtgcgcggaacccctatttgtttatttttctaaatacattcaaatatgtatccgctcatgagacaataaccctgataaatgcttcaataatattgaaaaaggaagagtatgagtattcaacatttccgtgtcgcccttattcccttttttgcggcattttgccttcctgtttttgctcacccagaaacgctggtgaaagtaaaagatgctgaagatcagttgggtgcacgagtgggttacatcgaactggatctcaacagcggtaagatccttgagagttttcgccccgaagaacgttttccaatgatgagcacttttaaagttctgctatgtggcgcggtattatcccgtattgacgccgggcaagagcaactcggtcgccgcatacactattctcagaatgacttggttgagtactcaccagtcacagaaaagcatcttacggatggcatgacagtaagagaattatgcagtgctgccataaccatgagtgataacactgcggccaacttacttctgacaacgatcggaggaccgaaggagctaaccgcttttttgcacaacatgggggatcatgtaactcgccttgatcgttgggaaccggagctgaatgaagccataccaaacgacgagcgtgacaccacgatgcctgtagcaatggcaacaacgttgcgcaaactattaactggcgaactacttactctagcttcccggcaacaattaatagactggatggaggcggataaagttgcaggaccacttctgcgctcggcccttccggctggctggtttattgctgataaatctggagccggtgagcgtggaagccgcggtatcattgcagcactggggccagatggtaagccctcccgtatcgtagttatctacacgacggggagtcaggcaactatggatgaacgaaatagacagatcgctgagataggtgcctcactgattaagcattggtaactgtcagaccaagtttactcatatatactttagattgatttaaaacttcatttttaatttaaaaggatctaggtgaagatcctttttgataatctcatgaccaaaatcccttaacgtgagttttcgttccactgagcgtcagaccccgtagaaaagatcaaaggatcttcttgagatcctttttttctgcgcgtaatctgctgcttgcaaacaaaaaaaccaccgctaccagcggtggtttgtttgccggatcaagagctaccaactctttttccgaaggtaactggcttcagcagagcgcagataccaaatactgttcttctagtgtagccgtagttaggccaccacttcaagaactctgtagcaccgcctacatacctcgctctgctaatcctgttaccagtggctgctgccagtggcgataagtcgtgtcttaccgggttggactcaagacgatagttaccggataaggcgcagcggtcgggctgaacggggggttcgtgcacacagcccagcttggagcgaacgacctacaccgaactgagatacctacagcgtgagctatgagaaagcgccacgcttcccgaagggagaaaggcggacaggtatccggtaagcggcagggtcggaacaggagagcgcacgagggagcttccagggggaaacgcctggtatctttatagtcctgtcgggtttcgccacctctgacttgagcgtcgatttttgtgatgctcgtcaggggggcggagcctatggaaaaacgccagcaacgcggcctttttacggttcctggccttttgctggccttttgctcacatgt

SEQ ID NO: 38 - DNA, 34 bp, synthetic construct
  source 1..34: mol_type = other DNA
caacgtggttggagaactggatgtagatgggctg

SEQ ID NO: 39 - DNA, 34 bp, synthetic construct
  source 1..34: mol_type = other DNA
atctgtggttggagaactggatgtagatgggctg

SEQ ID NO: 40 - RNA, 21 nt, synthetic construct
  source 1..21: mol_type = other RNA
gcccatctacatccagttctc

SEQ ID NO: 41 - RNA, 21 nt, synthetic construct
  source 1..21: mol_type = other RNA
cagcccatctacatccagttc

SEQ ID NO: 42 - RNA, 30 nt, synthetic construct
  source 1..30: mol_type = other RNA
catgaaaaacttgagagttgctgggtctga

SEQ ID NO: 43 - RNA, 30 nt, synthetic construct
  source 1..30: mol_type = other RNA
gaattaagttagttagttgctcttctaaat

SEQ ID NO: 44 - RNA, 30 nt, synthetic construct
  source 1..30: mol_type = other RNA
cgatgttgaattaatgtccatggactacct

SEQ ID NO: 45 - RNA, 30 nt, synthetic construct
  source 1..30: mol_type = other RNA
gatagagaaatttctgtgggttcttgaata

SEQ ID NO: 46 - RNA, 30 nt, synthetic construct
  source 1..30: mol_type = other RNA
ctggagaaggtctttgatgctattatcttg

SEQ ID NO: 47 - RNA, 30 nt, synthetic construct
  source 1..30: mol_type = other RNA
cactatggagtatatcttctctaggcccaa

SEQ ID NO: 48 - RNA, 30 nt, synthetic construct
  source 1..30: mol_type = other RNA
ccacactcatcatgccaccaccagcctcct

SEQ ID NO: 49 - RNA, 30 nt, synthetic construct
  source 1..30: mol_type = other RNA
gaccatctaaaattgattcccacatcacaa

SEQ ID NO: 50 - DNA, 21 bp, synthetic construct
  source 1..21: mol_type = other DNA
ccagaacacccagaagtaact

SEQ ID NO: 51 - DNA, 24 bp, synthetic construct
  source 1..24: mol_type = other DNA
tctgtgggttcttgaatactagtc

SEQ ID NO: 52 - DNA, 9915 bp, synthetic construct
  source 1..9915: mol_type = other DNA
gtcgacggatcgggagatctcccgatcccctatggtgcactctcagtacaatctgctctgatgccgcatagttaagccagtatctgctccctgcttgtgtgttggaggtcgctgagtagtgcgcgagcaaaatttaagctacaacaaggcaaggcttgaccgacaattgcatgaagaatctgcttagggttaggcgttttgcgctgcttcgcgatgtacgggccagatatacgcgttgacattgattattgactagttattaatagtaatcaattacggggtcattagttcatagcccatatatggagttccgcgttacataacttacggtaaatggcccgcctggctgaccgcccaacgacccccgcccattgacgtcaataatgacgtatgttcccatagtaacgccaatagggactttccattgacgtcaatgggtggagtatttacggtaaactgcccacttggcagtacatcaagtgtatcatatgccaagtacgccccctattgacgtcaatgacggtaaatggcccgcctggcattatgcccagtacatgaccttatgggactttcctacttggcagtacatctacgtattagtcatcgctattaccatggtgatgcggttttggcagtacatcaatgggcgtggatagcggtttgactcacggggatttccaagtctccaccccattgacgtcaatgggagtttgttttggcaccaaaatcaacgggactttccaaaatgtcgtaacaactccgccccattgacgcaaatgggcggtaggcgtgtacggtgggaggtctatagaccagatctgagcctgggagctctctggctaactagggaacccactgcttaagcctcaataaagcttgccttgagtgcttcaagtagtgtgtgcccgtctgttgtgtgactctggtaactagagatccctcagacccttttagtcagtgtggaaaatctctagcagtggcgcccgaacagggacttgaaagcgaaagggaaaccagaggagctctctcgacgcaggactcggcttgctgaagcgcgcacggcaagaggcgaggggcggcgactggtgagtacgccaaaaattttgactagcggaggctagaaggagagagatgggtgcgagagcgtcagtattaagcgggggagaattagatcgcgatgggaaaaaattcggttaaggccagggggaaagaaaaaatataaataaacatatagtatgggcaagcagggagctagaacgattcgcagttaatcctggcctgttagaaacatcagaaggctgtagacaaatactgggacagctacaaccatcccttcagacaggatcagaagaacttagatcattatataatacagtagcaaccctctattgtgtgcatcaaaggatagagataaaagacaccaaggaagctttagacaagatagaggaagagcaaaacaaaagtaagaccaccgcacagcaagcggccggccgcgctgatcttcagacctggaggaggagatatgagggacaattggagaagtgaattatataaatataaagtagtaaaaattgaaccattaggagtagcacccaccaaggcaaagagaagagtggtgcagagagaaaaaagagcagtgggaataggagctttgttccttgggttcttgggagcagcaggaagcactatgggcgcagcgtcaatgacgctgacggtacaggccagacaattattgtctggtatagtgcagcagcagaacaatttgctgagggctattgaggcgcaacagcatctgttgcaactcacagtctggggcatcaagcagctccaggcaagaatcctggctgtggaaagatacctaaaggatcaacagctcctggggatttggggttgctctggaaaactcatttgcaccactgctgtgccttggaatgctagttggagtaataaatctctggaacagatttggaatcacacgacctggatggagtgggacagagaaattaacaattacacaagcttaatacactccttaattgaagaatcgcaaaaccagcaagaaaagaatgaacaagaattattggaattagataaatgggcaagtttgtggaattggtttaacataacaaattggctgtggtatataaaattattcataatgatagtaggaggcttggtaggtttaagaatagtttttgctgtactttctatagtgaatagagttaggcagggatattcaccattatcgtttcagacccacctcccaaccccgaggggacccgacaggcccgaaggaatagaagaagaaggtggagagagagacagagacagatccattcgattagtgaacggatcggcactgcgtgcgccaattctgcagacaaatggcagtattcatccacaattttaaaagaaaaggggggattggggggtacagtgcaggggaaagaatagtagacataatagcaacagacatacaaactaaagaattacaaaaacaaattacaaaaattcaaaattttcgggtttattacagggacagcagagatccagtttggttagtaccgggcccgctctagcgtcgaggagcttggcccattgcatacgttgtatccatatcataatatgtacatttatattggctcatgtccaacattaccgccatgttgacattgattattgactagttattaatagtaatcaattacggggtcattagttcatagcccatatatggagttccgcgttacataacttacggtaaatggcccgcctggctgaccgcccaacgacccccgcccattgacgtcaataatgacgtatgttcccatagtaacgccaatagggactttccattgacgtcaatgggtggagtatttacggtaaactgcccacttggcagtacatcaagtgtatcatatgccaagtacgccccctattgacgtcaatgacggtaaatggcccgcctggcattatgcccagtacatgaccttatgggactttcctacttggcagtacatctacgtattagtcatcgctattaccatggtgatgcggttttggcagtacatcaatgggcgtggatagcggtttgactcacggggatttccaagtctccaccccattgacgtcaatgggagtttgttttggcaccaaaatcaacgggactttccaaaatgtcgtaacaactccgccccattgacgcaaatgggcggtaggcgtgtacggtgggaggtctatataagcagagctcgtttagtgaaccgtcagatcgcctggagacgccatccacgctgttttgacctccatagaagacaccgggaccgatccagcctccgcggccccgaattcgccaccatggccatgttcacaattaagctccttctttttattgttcctctagttatttcctccagaattgatcaagacaattcatcatttgattctctatctccagagccaaaatcaagatttgctatgttagacgatgtaaaaattttagccaatggcctccttcagttgggacatggtcttaaagactttgtccataagacgaagggccaaattaatgacatatttcaaaaactcaacatatttgatcagtctttttatgatctatcgctgcaaaccagtgaaatcaaagaagaagaaaaggaactgagaagaactacatataaactacaagtcaaaaatgaagaggtaaagaatatgtcacttgaactcaactcaaaacttgaaagcctcctagaagaaaaaattctacttcaacaaaaagtgaaatatttagaagagcaactaactaacttaattcaaaatcaacctgaaactccagaacacccagaagtaacttcacttaaaacttttgtagaaaaacaagataatagcatcaaagaccttctccagaccgtggaagaccaatataaacaattaaaccaacagcatagtcaaataaaagaaatagaaaatcagctcagaaggactagtattcaagaacccacagaaatttctctatcttccaagccaagagcaccaagaactactccctttcttcagttgaatgaaataagaaatgtaaaacatgatggcattcctgctgaatgtaccaccatttataacagaggtgaacatacaagtggcatgtatgccatcagacccagcaactctcaagtttttcatgtctactgtgatgttatatcaggtagtccatggacattaattcaacatcgaatagatggatcacaaaacttcaatgaaacgtgggagaactacaaatatggttttgggaggcttgatggagaattttggttgggcctagagaagatatactccatagtgaagcaatctaattatgttttacgaattgagttggaagactggaaagacaacaaacattatattgaatattctttttacttgggaaatcacgaaaccaactatacgctacatctagttgcgattactggcaatgtccccaatgcaatcccggaaaacaaagatttggtgttttctacttgggatcacaaagcaaaaggacacttcaactgtccagagggttattcaggaggctggtggtggcatgatgagtgtggagaaaacaacctaaatggtaaatataacaaaccaagagcaaaatctaagccagagaggagaagaggattatcttggaagtctcaaaatggaaggttatactctataaaatcaaccaaaatgttgatccatccaacagattcagaaagctttgaaggatccgctagcggcagtggagagggcagaggaagtctgctaacatgcggtgacgtcgaggagaatcctggcccagtgagcaagggcgaggagctgttcaccggggtggtgcccatcctggtcgagctggacggcgacgtaaacggccacaagttcagcgtgtccggcgagggcgagggcgatgccacctacggcaagctgaccctgaagttcatctgcaccaccggcaagctgcccgtgccctggcccaccctcgtgaccaccctgacctacggcgtgcagtgcttcagccgctaccccgaccacatgaagcagcacgacttcttcaagtccgccatgcccgaaggctacgtccaggagcgcaccatcttcttcaaggacgacggcaactacaagacccgcgccgaggtgaagttcgagggcgacaccctggtgaaccgcatcgagctgaagggcatcgacttcaaggaggacggcaacatcctggggcacaagctggagtacaactacaacagccacaacgtctatatcatggccgacaagcagaagaacggcatcaaggtgaacttcaagatccgccacaacatcgaggacggcagcgtgcagctcgccgaccactaccagcagaacacccccatcggcgacggccccgtgctgctgcccgacaaccactacctgagcacccagtccgccctgagcaaagaccccaacgagaagcgcgatcacatggtcctgctggagttcgtgaccgccgccgggatcactctcggcatggacgagctgtacaagtaaggatcctaggcggccgcgcatgccctgcaggtgatctatcgatcggccggcccctctccctccccccccccctaacgttactggccgaagccgcttggaataaggccggtgtgcgtttgtctatatgttattttccaccatattgccgtcttttggcaatgtgagggcccggaaacctggccctgtcttcttgacgagcattcctaggggtctttcccctctcgccaaaggaatgcaaggtctgttgaatgtcgtgaaggaagcagttcctctggaagcttcttgaagacaaacaacgtctgtagcgaccctttgcaggcagcggaaccccccacctggcgacaggtgcctctgcggccaaaagccacgtgtataagatacacctgcaaaggcggcacaaccccagtgccacgttgtgagttggatagttgtggaaagagtcaaatggctctcctcaagcgtattcaacaaggggctgaaggatgcccagaaggtaccccattgtatgggatctgatctggggcctcggtacacatgctttacatgtgtttagtcgaggttaaaaaaacgtctaggccccccgaaccacggggacgtggttttcctttgaaaaacacgatgataatatggccacaaccgggccggatatcacgcgtgatctgatcagcacgtgttgacaattaatcatcggcatagtatatcggcatagtataatacgacaaggtgaggaactaaaccatggccaagcctttgtctcaagaagaatccaccctcattgaaagagcaacggctacaatcaacagcatccccatctctgaagactacagcgtcgccagcgcagctctctctagcgacggccgcatcttcactggtgtcaatgtatatcattttactgggggaccttgtgcagaactcgtggtgctgggcactgctgctgctgcggcagctggcaacctgacttgtatcgtcgcgatcggaaatgagaacaggggcatcttgagcccctgcggacggtgccgacaggtgcttctcgatctgcatcctgggatcaaagccatagtgaaggacagtgatggacagccgacggcagttgggattcgtgaattgctgccctctggttatgtgtgggagggctaagcaatgcatacatgtgtttaaacctcgacttaattaagtcgagggtcgacggtatcgataagctcgcttcacgagatcatgtttaagggttccggttccactaggtacaattcgatatcaagcttatcgataatcaacctctggattacaaaatttgtgaaagattgactggtattcttaactatgttgctccttttacgctatgtggatacgctgctttaatgcctttgtatcatgctattgcttcccgtatggctttcattttctcctccttgtataaatcctggttgctgtctctttatgaggagttgtggcccgttgtcaggcaacgtggcgtggtgtgcactgtgtttgctgacgcaacccccactggttggggcattgccaccacctgtcagctcctttccgggactttcgctttccccctccctattgccacggcggaactcatcgccgcctgccttgcccgctgctggacaggggctcggctgttgggcactgacaattccgtggtgttgtcggggaaatcatcgtcctttccttggctgctcgcctgtgttgccacctggattctgcgcgggacgtccttctgctacgtcccttcggccctcaatccagcggaccttccttcccgcggcctgctgccggctctgcggcctcttccgcgtcttcgccttcgccctcagacgagtcggatctccctttgggccgcctccccgcatcgataccgtcgacctcgatcgagacctagaaaaacatggagcaatcacaagtagcaatacagcagctaccaatgctgattgtgcctggctagaagcacaagaggaggaggaggtgggttttccagtcacacctcaggtacctttaagaccaatgacttacaaggcagctgtagatcttagccactttttaaaagaaaaggggggactggaagggctaattcactcccaacgaagacaagatatccttgatctgtggatctaccacacacaaggctacttccctgattggcagaactacacaccagggccagggatcagatatccactgacctttggatggtgctacaagctagtaccagttgagcaagagaaggtagaagaagccaatgaaggagagaacacccgcttgttacaccctgtgagcctgcatgggatggatgacccggagagagaagtattagagtggaggtttgacagccgcctagcatttcatcacatggcccgagagctgcatccggactgtactgggtctctctggttagaccagatctgagcctgggagctctctggctaactagggaacccactgcttaagcctcaataaagcttgccttgagtgcttcaagtagtgtgtgcccgtctgttgtgtgactctggtaactagagatccctcagacccttttagtcagtgtggaaaatctctagcagcatgtgagcaaaaggccagcaaaaggccaggaaccgtaaaaaggccgcgttgctggcgtttttccataggctccgcccccctgacgagcatcacaaaaatcgacgctcaagtcagaggtggcgaaacccgacaggactataaagataccaggcgtttccccctggaagctccctcgtgcgctctcctgttccgaccctgccgcttaccggatacctgtccgcctttctcccttcgggaagcgtggcgctttctcatagctcacgctgtaggtatctcagttcggtgtaggtcgttcgctccaagctgggctgtgtgcacgaaccccccgttcagcccgaccgctgcgccttatccggtaactatcgtcttgagtccaacccggtaagacacgacttatcgccactggcagcagccactggtaacaggattagcagagcgaggtatgtaggcggtgctacagagttcttgaagtggtggcctaactacggctacactagaagaacagtatttggtatctgcgctctgctgaagccagttaccttcggaaaaagagttggtagctcttgatccggcaaacaaaccaccgctggtagcggtggtttttttgtttgcaagcagcagattacgcgcagaaaaaaaggatctcaagaagatcctttgatcttttctacggggtctgacgctcagtggaacgaaaactcacgttaagggattttggtcatgagattatcaaaaaggatcttcacctagatccttttaaattaaaaatgaagttttaaatcaatctaaagtatatatgagtaaacttggtctgacagttaccaatgcttaatcagtgaggcacctatctcagcgatctgtctatttcgttcatccatagttgcctgactccccgtcgtgtagataactacgatacgggagggcttaccatctggccccagtgctgcaatgataccgcgagacccacgctcaccggctccagatttatcagcaataaaccagccagccggaagggccgagcgcagaagtggtcctgcaactttatccgcctccatccagtctattaattgttgccgggaagctagagtaagtagttcgccagttaatagtttgcgcaacgttgttgccattgctacaggcatcgtggtgtcacgctcgtcgtttggtatggcttcattcagctccggttcccaacgatcaaggcgagttacatgatcccccatgttgtgcaaaaaagcggttagctccttcggtcctccgatcgttgtcagaagtaagttggccgcagtgttatcactcatggttatggcagcactgcataattctcttactgtcatgccatccgtaagatgcttttctgtgactggtgagtactcaaccaagtcattctgagaatagtgtatgcggcgaccgagttgctcttgcccggcgtcaatacgggataataccgcgccacatagcagaactttaaaagtgctcatcattggaaaacgttcttcggggcgaaaactctcaaggatcttaccgctgttgagatccagttcgatgtaacccactcgtgcacccaactgatcttcagcatcttttactttcaccagcgtttctgggtgagcaaaaacaggaaggcaaaatgccgcaaaaaagggaataagggcgacacggaaatgttgaatactcatactcttcctttttcaatattattgaagcatttatcagggttattgtctcatgagcggatacatatttgaatgtatttagaaaaataaacaaataggggttccgcgcacatttccccgaaaagtgccacctgac

SEQ ID NO: 53 - protein, 11 aa, synthetic construct
SPKKKRKVEAS

SEQ ID NO: 54 - protein, 11 aa, synthetic construct
GPKKKRKVAAA

SEQ ID NO: 55 - protein, 7 aa, synthetic construct
PKKKRKV

SEQ ID NO: 56 - protein, 16 aa, synthetic construct
KRPAATKKAGQAKKKK

SEQ ID NO: 57 - protein, 9 aa, synthetic construct
PAAKRVKLD

SEQ ID NO: 58 - protein, 11 aa, synthetic construct
RQRRNELKRSP

SEQ ID NO: 59 - protein, 38 aa, synthetic construct
NQSSNFGPMKGGNFGGRSSGPYGGGGQYFAKPRNQGGY

SEQ ID NO: 60 - protein, 42 aa, synthetic construct
RMRIZFKNKGKDTAELRRRRVEVSVELRKAKKDEQILKRRNV

SEQ ID NO: 61 - protein, 8 aa, synthetic construct
VSRKRPRP

SEQ ID NO: 62 - protein, 8 aa, synthetic construct
PPKKARED

SEQ ID NO: 63 - protein, 8 aa, synthetic construct
POPKKKPL

SEQ ID NO: 64 - protein, 12 aa, synthetic construct
SALIKKKKKMAP

SEQ ID NO: 65 - protein, 5 aa, synthetic construct
DRLRR

SEQ ID NO: 66 - protein, 7 aa, synthetic construct
PKQKKRK

SEQ ID NO: 67 - protein, 10 aa, synthetic construct
RKLKKKIKKL

SEQ ID NO: 68 - protein, 10 aa, synthetic construct
REKKKFLKRR

SEQ ID NO: 69 - protein, 20 aa, synthetic construct
KRKGDEVDGVDEVAKKKSKK

SEQ ID NO: 70 - protein, 17 aa, synthetic construct
RKCLQAGMNLEARKTKK

SEQ ID NO: 71 - protein, 9 aa, synthetic construct
PAAKKKKLD

SEQ ID NO: 72 - DNA, 6802 bp, synthetic construct
  source 1..6802: mol_type = other DNA
cctgcaggcagctgcgcgctcgctcgctcactgaggccgcccgggcgtcgggcgacctttggtcgcccggcctcagtgagcgagcgagcgcgcagagagggagtggccaactccatcactaggggttcctgcggcctctagactcgaggcgttgacattgattattgactagttattaatagtaatcaattacggggtcattagttcatagcccatatatggagttccgcgttacataacttacggtaaatggcccgcctggctgaccgcccaacgacccccgcccattgacgtcaataatgacgtatgttcccatagtaacgccaatagggactttccattgacgtcaatgggtggagtatttacggtaaactgcccacttggcagtacatcaagtgtatcatatgccaagtacgccccctattgacgtcaatgacggtaaatggcccgcctggcattatgcccagtacatgaccttatgggactttcctacttggcagtacatctacgtattagtcatcgctattaccatggtgatgcggttttggcagtacatcaatgggcgtggatagcggtttgactcacggggatttccaagtctccaccccattgacgtcaatgggagtttgttttggcaccaaaatcaacgggactttccaaaatgtcgtaacaactccgccccattgacgcaaatgggcggtaggcgtgtacggtgggaggtctatataagcagagctctctggctaactaccggtgccaccatgccggcagctaagaaaaagaaactggatggcagcgtcgacatgagcaaggacaagaaaaccaaggccaagagaatgggcgtgaaggccctgctggcccacggcgaggacaagctgaccatgaccaccttcggcaagggcaacagaagcaagatcgagttcaccgagggctaccacggcagagccctggagacacccaagcacttcggcatcagaggcttcgaggtgagaagaatcgacgagaacgtggacctgtgcggcgacctggaggagggcaagaccatcgaggccctgctggtgaaccccagcgagaaggtgggcgaggactacctgaagctgaagggcaccctggagaagagattcttcggcagagagttcccccacgacaacatcagaatccagctgatctacaacatcctggacatctacaagatcctgggcatgaacgtggccgacatcctgtacgccctgggcaacatgcaggacaccgagctggacatcgacatgttcggccagagcctgaacaacgaggacaacctgaaggagtgcctgaagagaatgaggccctacatgggctacttcggcgacatcttcaagatcagccccaagggcgagaacatcgccgacagagagcacaacaagaaggtgctgagatgcatcagcgtgctgagaaacgccaccgcccacgacaagcaggacgagtacccctggttcaagagcagcgacatctacgagacaaagatcttcaaggccgacatgtggaagatcatcaaggaccagtacagagagaagatcaagaaggtgaacaaggacttcctgagcaagaacgccgtgaacatggccatcctgttcgacctgctgaacgccagagacgtggagcagaagaagcagatcaccgacgagttctacagattcaccatcagaaaggacggcaagaacctgggcatgaacctggtgaagatcagagagatcatcatcgacagatacgccagcggcctgagagacaagaagcacgacccccacagacagaagatcaacgtgatcgccgacttcctgatcttcagagccctgagccagaaccagggcatcatcgacaagaccgtgagcagcctgagactgaccaaggacgaggaggagaaggaccacgtgtaccagaacgccgccgagctggtgtggggcatggtgagcaactgcctgaccccctacttcaacgaccccaagaacaagtacatcctgaagtacaaggacgccaagacccccggcgacttcgaggactggatcaccagcaagatcagcgaggacgacggcgagcccttcgtgaaggtgctgagcttcctgtgcaacttcctggagggcaaggagatcaacgagctgctgaccgcctacatccacaagttcgagtgcatccaggacttcctgaacgtgatcagcagcctgggcgagaacgtgcagttccagcccagattcgccctgttcaacaacgccagcttcgcccagaacgtggccgtgcagctgagaatcctggccagcatcggcaagatgaagcccgacctgaccgaggccaagaggcccctgtacaaggccgccatcagaatgctgtgcccccccgagaagtgggagaagtacaccagcgacgagtggctggagaagaacatgctgctgaacagcgaggacagaaagaacgacaagaagaagaagcaggtgaaccccttcagaaacttcatcgccggcaacgtgatcgagagcagaagattcatgtacctggtgagatacagcaagcccaaggccgtgagagccatcatgcagaacagaagcatcgtgaactacgtgctgcacagactgcccagcgagcaggtgcacagatacgccagcgtgttccccgagaacttcgccgacctggagcaggagatcgacttcctgaccaagaagctgttcgagttcagcttcgaggagctgctgcacgagaaggacgtgatcctgaacaacagcagaagccacaagcccagcctggagatcgagagactgaaggccatcaccggcctgtacctgagcgtggcctacatcgccatcaagaacatcgtgaaggccaacgccagatactacatcgccttcgccgtgttcgagagagacaaggagctggtgaaggccaaggacgccagaatccagaccaagatccccgagacagacttccccgactacttctgcctgacccagtactacctggacagagacgaggagaagaagttccccggcgaccccagagacaaggaggccttcttcgagcacctgagaaagaccaagagacacttcagcaagcagtggagagagtggctgaacgagaagatcgccgacgccaagagcagccaggccaccggcctgctgctgagagaggccagaaacgacgtggagcacctgaacgtgctgagagccatccccgactacatccaggacttcagacacggcgagaagggcgagacagccatgaacagctacttcgagctgtaccactacctgatgcagagactgatgctgaagaacaccgagctggacctgagccactggagcggctggatcatgagaagcggcagacccgacagagacttgatccagatcgccttcgtgagcctggcctacaacctgcccagatacagaaacctgaccaaggagcaccacttcgacgacaccgtgctgcagaagatcagagagaaggagagcctggacacaggcggcggccccggcggcggcgccgccgccggcagcggcagccctaagaaaaaacgaaaagttggcagcggaagcaaaaggccggcggccacgaaaaaggccggccaggcaaaaaagaaaaagctcgagtacccatacgatgttccagattacgcttgagaattccccttgagcatctgacttctggctaataaaggaaatttattttcattgcaatagtgtgttggaattttttgtgtctctcaggtaccgagggcctatttcccatgattccttcatatttgcatatacgatacaaggctgttagagagataattggaattaatttgactgtaaacacaaagatattagtacaaaatacgtgacgtagaaagtaataatttcttgggtagtttgcagttttaaaattatgttttaaaatggactatcatatgcttaccgtaacttgaaagtatttcgatttcttggctttatatatcttgtggaaaggacgaaacaccggaagataactctacaaacctgtagggttctgagactgggtgcagcctgggaccacttggcatggttttttgcggccgcaggaacccctagtgatggagttggccactccctctctgcgcgctcgctcgctcactgaggccgggcgaccaaaggtcgcccgacgcccgggctttgcccgggcggcctcagtgagcgagcgagcgcgcagctgcctgcaggggcgcctgatgcggtattttctccttacgcatctgtgcggtatttcacaccgcatacgtcaaagcaaccatagtacgcgccctgtagcggcgcattaagcgcggcgggtgtggtggttacgcgcagcgtgaccgctacacttgccagcgccttagcgcccgctcctttcgctttcttcccttcctttctcgccacgttcgccggctttccccgtcaagctctaaatcgggggctccctttagggttccgatttagtgctttacggcacctcgaccccaaaaaacttgatttgggtgatggttcacgtagtgggccatcgccctgatagacggtttttcgccctttgacgttggagtccacgttctttaatagtggactcttgttccaaactggaacaacactcaactctatctcgggctattcttttgatttataagggattttgccgatttcggtctattggttaaaaaatgagctgatttaacaaaaatttaacgcgaattttaacaaaatattaacgtttacaattttatggtgcactctcagtacaatctgctctgatgccgcatagttaagccagccccgacacccgccaacacccgctgacgcgccctgacgggcttgtctgctcccggcatccgcttacagacaagctgtgaccgtctccgggagctgcatgtgtcagaggttttcaccgtcatcaccgaaacgcgcgagacgaaagggcctcgtgatacgcctatttttataggttaatgtcatgataataatggtttcttagacgtcaggtggcacttttcggggaaatgtgcgcggaacccctatttgtttatttttctaaatacattcaaatatgtatccgctcatgagacaataaccctgataaatgcttcaataatattgaaaaaggaagagtatgagtattcaacatttccgtgtcgcccttattcccttttttgcggcattttgccttcctgtttttgctcacccagaaacgctggtgaaagtaaaagatgctgaagatcagttgggtgcacgagtgggttacatcgaactggatctcaacagcggtaagatccttgagagttttcgccccgaagaacgttttccaatgatgagcacttttaaagttctgctatgtggcgcggtattatcccgtattgacgccgggcaagagcaactcggtcgccgcatacactattctcagaatgacttggttgagtactcaccagtcacagaaaagcatcttacggatggcatgacagtaagagaattatgcagtgctgccataaccatgagtgataacactgcggccaacttacttctgacaacgatcggaggaccgaaggagctaaccgcttttttgcacaacatgggggatcatgtaactcgccttgatcgttgggaaccggagctgaatgaagccataccaaacgacgagcgtgacaccacgatgcctgtagcaatggcaacaacgttgcgcaaactattaactggcgaactacttactctagcttcccggcaacaattaatagactggatggaggcggataaagttgcaggaccacttctgcgctcggcccttccggctggctggtttattgctgataaatctggagccggtgagcgtggaagccgcggtatcattgcagcactggggccagatggtaagccctcccgtatcgtagttatctacacgacggggagtcaggcaactatggatgaacgaaatagacagatcgctgagataggtgcctcactgattaagcattggtaactgtcagaccaagtttactcatatatactttagattgatttaaaacttcatttttaatttaaaaggatctaggtgaagatcctttttgataatctcatgaccaaaatcccttaacgtgagttttcgttccactgagcgtcagaccccgtagaaaagatcaaaggatcttcttgagatcctttttttctgcgcgtaatctgctgcttgcaaacaaaaaaaccaccgctaccagcggtggtttgtttgccggatcaagagctaccaactctttttccgaaggtaactggcttcagcagagcgcagataccaaatactgttcttctagtgtagccgtagttaggccaccacttcaagaactctgtagcaccgcctacatacctcgctctgctaatcctgttaccagtggctgctgccagtggcgataagtcgtgtcttaccgggttggactcaagacgatagttaccggataaggcgcagcggtcgggctgaacggggggttcgtgcacacagcccagcttggagcgaacgacctacaccgaactgagatacctacagcgtgagctatgagaaagcgccacgcttcccgaagggagaaaggcggacaggtatccggtaagcggcagggtcggaacaggagagcgcacgagggagcttccagggggaaacgcctggtatctttatagtcctgtcgggtttcgccacctctgacttgagcgtcgatttttgtgatgctcgtcaggggggcggagcctatggaaaaacgccagcaacgcggcctttttacggttcctggccttttgctggccttttgctcacatgt

SEQ ID NO: 73 - DNA, 29 bp, synthetic construct
  source 1..29: mol_type = other DNA
tgggtgcagcctgggaccacttggcatgg

SEQ ID NO: 74 - DNA, 18 bp, synthetic construct
  source 1..18: mol_type = other DNA
agaaacgccaccgcccac

SEQ ID NO: 75 - DNA, 18 bp, synthetic construct
  source 1..18: mol_type = other DNA
gcaaacgccaccgccgcc

SEQ ID NO: 76 - DNA, 18 bp, synthetic construct
  source 1..18: mol_type = other DNA
agaaagaccaagagacac

SEQ ID NO: 77 - DNA, 18 bp, synthetic construct
  source 1..18: mol_type = other DNA
gcaaagaccaagagagcc

SEQ ID NO: 78 - DNA, 18 bp, synthetic construct
  source 1..18: mol_type = other DNA
agaaacgacgtggagcac

SEQ ID NO: 79 - DNA, 18 bp, synthetic construct
  source 1..18: mol_type = other DNA
gcaaacgacgtggaggcc

SEQ ID NO: 80 - DNA, 36 bp, synthetic construct
  source 1..36: mol_type = other DNA
ccgcacagtccctacaggtttgtagagtcatcttcc

SEQ ID NO: 81 - DNA, 36 bp, synthetic construct
  source 1..36: mol_type = other DNA
ggaagatgactctacaaacctgtagggactgtgcgg

SEQ ID NO: 82 - DNA, 36 bp, synthetic construct
  source 1..36: mol_type = other DNA
ggtgtacagggtgcctggatttgacagggttacagc

SEQ ID NO: 83 - DNA, 36 bp, synthetic construct
  source 1..36: mol_type = other DNA
gctgtaaccctgtcaaatccaggcaccctgtacacc

SEQ ID NO: 84 - DNA, 36 bp, synthetic construct
  source 1..36: mol_type = other DNA
ggtgtacagggtgcctagatttgacagggttacagc

SEQ ID NO: 85 - DNA, 36 bp, synthetic construct
  source 1..36: mol_type = other DNA
gctgtaaccctgtcaaatctaggcaccctgtacacc

SEQ ID NO: 86 - DNA, 34 bp, synthetic construct
  source 1..34: mol_type = other DNA
ggaagaactctacaaacctgtagggttctgagac

SEQ ID NO: 87 - DNA, 36 bp, synthetic construct
  source 1..36: mol_type = other DNA
ggaagataactctacaaacctgtagagttctgagac

SEQ ID NO: 88 - DNA, 20 bp, synthetic construct
  source 1..20: mol_type = other DNA
acctccaccatgccaagtgg

SEQ ID NO: 89 - DNA, 20 bp, synthetic construct
  source 1..20: mol_type = other DNA
cagggtctcgattggatggc

SEQ ID NO: 90 - DNA, 30 bp, synthetic construct
  source 1..30: mol_type = other DNA
tgccgttcttctgcttgtcggccatgatat

SEQ ID NO: 91 - DNA, 7023 bp, synthetic construct
  source 1..7023: mol_type = other DNA
cctgcaggcagctgcgcgctcgctcgctcactgaggccgcccgggcgtcgggcgacctttggtcgcccggcctcagtgagcgagcgagcgcgcagagagggagtggccaactccatcactaggggttcctgcggcctctagactcgaggcgttgacattgattattgactagttattaatagtaatcaattacggggtcattagttcatagcccatatatggagttccgcgttacataacttacggtaaatggcccgcctggctgaccgcccaacgacccccgcccattgacgtcaataatgacgtatgttcccatagtaacgccaatagggactttccattgacgtcaatgggtggagtatttacggtaaactgcccacttggcagtacatcaagtgtatcatatgccaagtacgccccctattgacgtcaatgacggtaaatggcccgcctggcattatgcccagtacatgaccttatgggactttcctacttggcagtacatctacgtattagtcatcgctattaccatggtgatgcggttttggcagtacatcaatgggcgtggatagcggtttgactcacggggatttccaagtctccaccccattgacgtcaatgggagtttgttttggcaccaaaatcaacgggactttccaaaatgtcgtaacaactccgccccattgacgcaaatgggcggtaggcgtgtacggtgggaggtctatataagcagagctctctggctaactaccggtgccaccatgccggcagctaagaaaaagaaactggatggcagcgtcgacatcgagaagaaaaaatcctttgctaagggcatgggcgttaagagcactctggtgtcaggctctaaagtgtacatgaccacattcgccgagggctctgatgctcgcctggaaaaaattgtggaaggagactcaatcagatccgtgaacgagggggaggccttcagcgccgagatggccgacaagaatgccggatataagattggaaacgctaagttcagccatcccaagggatacgccgtggtcgccaacaatcctctgtacactggacctgtgcagcaggacatgttaggtctgaaggagactctggagaagaggtacttcggcgagtccgcagatggcaacgacaacatttgcattcaggtgatccataacatcctggacattgagaagatcctggccgagtatatcaccaacgcagcctacgctgtgaataatatatctggtctggataaggatatcattgggttcgggaaattttctaccgtgtacacctacgatgagtttaaagaccccgagcaccacagagccgccttcaacaacaacgacaagctgatcaatgccattaaggcacagtacgatgagttcgacaattttctggacaacccccggctgggctacttcggccaggcttttttttctaaggaaggccgcaattacatcatcaactacggcaacgagtgctatgacattctggcccttctgagcggcctgaggcattgggtggtgcataacaacgaagaggaatcccgcatctcaagaacatggctgtacaatctcgacaaaaacctggacaatgagtacatttccactctgaactatctgtacgacaggatcacgaatgagctgaccaattccttttccaagaatagcgccgccaatgtgaactacatcgccgaaaccctggggatcaatcccgccgagttcgccgagcagtattttcgattcagcatcatgaaagagcagaaaaatctgggctttaatatcaccaaactgagagaagtgatgctggacaggaaggatatgtctgagatcaggaagaaccacaaggtgttcgacagtatcagaaccaaggtgtatacaatgatggatttcgtgatctataggtactacattgaggaggacgccaaggtggccgccgccaacaaatccctgcctgataacgagaagtccctgtctgagaaggatatcttcgtcatcaacctgaggggcagcttcaatgatgaccagaaggacgctctttactacgacgaagccaaccggatctggcggaagctggaaaacatcatgcacaacatcaaggagttccgcgggaacaaaacacgggagtacaagaaaaaagacgctcccagactgcccagaatcctgcctgcaggcagggatgtgagcgcattctccaagctgatgtacgccctgacaatgttcctggatggcaaggaaatcaacgacctgctgaccactctgatcaacaagtttgataacattcagagctttctgaaagtgatgcccctgatcggagtgaatgcaaaattcgtcgaagaatacgctttcttcaaggattctgctaaaatcgccgacgagctgaggctgattaagtcctttgcaaggatgggggagccaatcgccgacgccagaagagccatgtatattgatgctatcagaatcctgggcaccaatctgtcctatgacgaactgaaggccctggctgacacattttctctggatgagaatggtaacaagctgaagaaggggaagcacggcatgcgaaactttattattaacaatgttatctctaataagaggttccattatctgattcgctacggcgaccccgcccatttgcacgagatcgccaagaatgaagcggtggtgaagttcgtcctgggacggatcgccgacatccagaaaaagcagggccagaatggcaaaaaccagatcgacagatattatgagacttgcatcggcaaggataagggtaaaagtgtctccgagaaagtggatgccctgactaagatcattacggggatgaattacgaccagtttgacaaaaagaggagcgtgatcgaggacaccggcagagagaatgccgagcgggagaagtttaagaagatcatcagcctgtatctgaccgtgatttaccatatcctgaagaatatcgtgaatatcaatgccagatacgtgatcggcttccactgcgtggaaagagacgcccagctctacaaagagaaaggctacgacatcaatctgaagaagctggaggaaaagggctttagcagcgtgacaaaactgtgtgcaggaatcgacgagactgcccctgacaagaggaaggacgtggagaaagagatggccgaacgcgccaaggagtctatcgactccctggagtccgccaaccccaagctgtacgccaactacatcaagtatagcgacgagaagaaggcagaagagttcacccggcagatcaatagagagaaggccaaaaccgcactgaatgcctatctgaggaatacaaagtggaacgtgattattagagaagatctgctgaggattgacaataagacctgtaccctattcaggaacaaggccgtgcatctggaggtggccaggtacgtgcatgcctatattaatgatatagctgaagtcaactcctatttccagctgtatcattacatcatgcagcgtattattatgaacgaaagatatgaaaagagctccggcaaagtgtctgagtacttcgatgccgtgaacgacgaaaaaaagtacaatgatcgcctgctgaagctgctgtgtgtgcccttcgggtactgtatccccagatttaagaatctgtccattgaagccctgttcgatagaaacgaagccgccaaattcgacaaggagaagaagaaggtgagcggcaatagtacaggcggcggccccggcggcggcgccgccgccggcagcggcagccctaagaaaaaacgaaaagttggcagcggaagcaaaaggccggcggccacgaaaaaggccggccaggcaaaaaagaaaaagctcgagtacccatacgatgttccagattacgcttgagaattccccttgagcatctgacttctggctaataaaggaaatttattttcattgcaatagtgtgttggaattttttgtgtctctcaggtaccgagggcctatttcccatgattccttcatatttgcatatacgatacaaggctgttagagagataattggaattaatttgactgtaaacacaaagatattagtacaaaatacgtgacgtagaaagtaataatttcttgggtagtttgcagttttaaaattatgttttaaaatggactatcatatgcttaccgtaacttgaaagtatttcgatttcttggctttatatatcttgtggaaaggacgaaacaccgcaagtaaacccctaccaactggtcggggtttgaaacgtggttggagaactggatgtagatgggctgttttttgcggccgcaggaacccctagtgatggagttggccactccctctctgcgcgctcgctcgctcactgaggccgggcgaccaaaggtcgcccgacgcccgggctttgcccgggcggcctcagtgagcgagcgagcgcgcagctgcctgcaggggcgcctgatgcggtattttctccttacgcatctgtgcggtatttcacaccgcatacgtcaaagcaaccatagtacgcgccctgtagcggcgcattaagcgcggcgggtgtggtggttacgcgcagcgtgaccgctacacttgccagcgccttagcgcccgctcctttcgctttcttcccttcctttctcgccacgttcgccggctttccccgtcaagctctaaatcgggggctccctttagggttccgatttagtgctttacggcacctcgaccccaaaaaacttgatttgggtgatggttcacgtagtgggccatcgccctgatagacggtttttcgccctttgacgttggagtccacgttctttaatagtggactcttgttccaaactggaacaacactcaactctatctcgggctattcttttgatttataagggattttgccgatttcggtctattggttaaaaaatgagctgatttaacaaaaatttaacgcgaattttaacaaaatattaacgtttacaattttatggtgcactctcagtacaatctgctctgatgccgcatagttaagccagccccgacacccgccaacacccgctgacgcgccctgacgggcttgtctgctcccggcatccgcttacagacaagctgtgaccgtctccgggagctgcatgtgtcagaggttttcaccgtcatcaccgaaacgcgcgagacgaaagggcctcgtgatacgcctatttttataggttaatgtcatgataataatggtttcttagacgtcaggtggcacttttcggggaaatgtgcgcggaacccctatttgtttatttttctaaatacattcaaatatgtatccgctcatgagacaataaccctgataaatgcttcaataatattgaaaaaggaagagtatgagtattcaacatttccgtgtcgcccttattcccttttttgcggcattttgccttcctgtttttgctcacccagaaacgctggtgaaagtaaaagatgctgaagatcagttgggtgcacgagtgggttacatcgaactggatctcaacagcggtaagatccttgagagttttcgccccgaagaacgttttccaatgatgagcacttttaaagttctgctatgtggcgcggtattatcccgtattgacgccgggcaagagcaactcggtcgccgcatacactattctcagaatgacttggttgagtactcaccagtcacagaaaagcatcttacggatggcatgacagtaagagaattatgcagtgctgccataaccatgagtgataacactgcggccaacttacttctgacaacgatcggaggaccgaaggagctaaccgcttttttgcacaacatgggggatcatgtaactcgccttgatcgttgggaaccggagctgaatgaagccataccaaacgacgagcgtgacaccacgatgcctgtagcaatggcaacaacgttgcgcaaactattaactggcgaactacttactctagcttcccggcaacaattaatagactggatggaggcggataaagttgcaggaccacttctgcgctcggcccttccggctggctggtttattgctgataaatctggagccggtgagcgtggaagccgcggtatcattgcagcactggggccagatggtaagccctcccgtatcgtagttatctacacgacggggagtcaggcaactatggatgaacgaaatagacagatcgctgagataggtgcctcactgattaagcattggtaactgtcagaccaagtttactcatatatactttagattgatttaaaacttcatttttaatttaaaaggatctaggtgaagatcctttttgataatctcatgaccaaaatcccttaacgtgagttttcgttccactgagcgtcagaccccgtagaaaagatcaaaggatcttcttgagatcctttttttctgcgcgtaatctgctgcttgcaaacaaaaaaaccaccgctaccagcggtggtttgtttgccggatcaagagctaccaactctttttccgaaggtaactggcttcagcagagcgcagataccaaatactgttcttctagtgtagccgtagttaggccaccacttcaagaactctgtagcaccgcctacatacctcgctctgctaatcctgttaccagtggctgctgccagtggcgataagtcgtgtcttaccgggttggactcaagacgatagttaccggataaggcgcagcggtcgggctgaacggggggttcgtgcacacagcccagcttggagcgaacgacctacaccgaactgagatacctacagcgtgagctatgagaaagcgccacgcttcccgaagggagaaaggcggacaggtatccggtaagcggcagggtcggaacaggagagcgcacgagggagcttccagggggaaacgcctggtatctttatagtcctgtcgggtttcgccacctctgacttgagcgtcgatttttgtgatgctcgtcaggggggcggagcctatggaaaaacgccagcaacgcggcctttttacggttcctggccttttgctggccttttgctcacatgt

SEQ ID NO: 92 - DNA, 7394 bp, synthetic construct
  source 1..7394: mol_type = other DNA
cctgcaggcagctgcgcgctcgctcgctcactgaggccgcccgggcgtcgggcgacctttggtcgcccggcctcagtgagcgagcgagcgcgcagagagggagtggccaactccatcactaggggttcctgcggcctctagactcgaggcgttgacattgattattgactagttattaatagtaatcaattacggggtcattagttcatagcccatatatggagttccgcgttacataacttacggtaaatggcccgcctggctgaccgcccaacgacccccgcccattgacgtcaataatgacgtatgttcccatagtaacgccaatagggactttccattgacgtcaatgggtggagtatttacggtaaactgcccacttggcagtacatcaagtgtatcatatgccaagtacgccccctattgacgtcaatgacggtaaatggcccgcctggcattatgcccagtacatgaccttatgggactttcctacttggcagtacatctacgtattagtcatcgctattaccatggtgatgcggttttggcagtacatcaatgggcgtggatagcggtttgactcacggggatttccaagtctccaccccattgacgtcaatgggagtttgttttggcaccaaaatcaacgggactttccaaaatgtcgtaacaactccgccccattgacgcaaatgggcggtaggcgtgtacggtgggaggtctatataagcagagctctctggctaactaccggtgccaccatgccggcagctaagaaaaagaaactggatggcagcgtcgacatgaacatccccgctctggtggaaaaccagaagaagtactttggcacctacagcgtgatggccatgctgaacgctcagaccgtgctggaccacatccagaaggtggccgatattgagggcgagcagaacgagaacaacgagaatctgtggtttcaccccgtgatgagccacctgtacaacgccaagaacggctacgacaagcagcccgagaaaaccatgttcatcatcgagcggctgcagagctacttcccattcctgaagatcatggccgagaaccagagagagtacagcaacggcaagtacaagcagaaccgcgtggaagtgaacagcaacgacatcttcgaggtgctgaagcgcgccttcggcgtgctgaagatgtacagggacctgaccaaccactacaagacctacgaggaaaagctgaacgacggctgcgagttcctgaccagcacagagcaacctctgagcggcatgatcaacaactactacacagtggccctgcggaacatgaacgagagatacggctacaagacagaggacctggccttcatccaggacaagcggttcaagttcgtgaaggacgcctacggcaagaaaaagtcccaagtgaataccggattcttcctgagcctgcaggactacaacggcgacacacagaagaagctgcacctgagcggagtgggaatcgccctgctgatctgcctgttcctggacaagcagtacatcaacatctttctgagcaggctgcccatcttctccagctacaatgcccagagcgaggaacggcggatcatcatcagatccttcggcatcaacagcatcaagctgcccaaggaccggatccacagcgagaagtccaacaagagcgtggccatggatatgctcaacgaagtgaagcggtgccccgacgagctgttcacaacactgtctgccgagaagcagtcccggttcagaatcatcagcgacgaccacaatgaagtgctgatgaagcggagcagcgacagattcgtgcctctgctgctgcagtatatcgattacggcaagctgttcgaccacatcaggttccacgtgaacatgggcaagctgagatacctgctgaaggccgacaagacctgcatcgacggccagaccagagtcagagtgatcgagcagcccctgaacggcttcggcagactggaagaggccgagacaatgcggaagcaagagaacggcaccttcggcaacagcggcatccggatcagagacttcgagaacatgaagcgggacgacgccaatcctgccaactatccctacatcgtggacacctacacacactacatcctggaaaacaacaaggtcgagatgtttatcaacgacaaagaggacagcgccccactgctgcccgtgatcgaggatgatagatacgtggtcaagacaatccccagctgccggatgagcaccctggaaattccagccatggccttccacatgtttctgttcggcagcaagaaaaccgagaagctgatcgtggacgtgcacaaccggtacaagagactgttccaggccatgcagaaagaagaagtgaccgccgagaatatcgccagcttcggaatcgccgagagcgacctgcctcagaagatcctggatctgatcagcggcaatgcccacggcaaggatgtggacgccttcatcagactgaccgtggacgacatgctgaccgacaccgagcggagaatcaagagattcaaggacgaccggaagtccattcggagcgccgacaacaagatgggaaagagaggcttcaagcagatctccacaggcaagctggccgacttcctggccaaggacatcgtgctgtttcagcccagcgtgaacgatggcgagaacaagatcaccggcctgaactaccggatcatgcagagcgccattgccgtgtacgatagcggcgacgattacgaggccaagcagcagttcaagctgatgttcgagaaggcccggctgatcggcaagggcacaacagagcctcatccatttctgtacaaggtgttcgcccgcagcatccccgccaatgccgtcgagttctacgagcgctacctgatcgagcggaagttctacctgaccggcctgtccaacgagatcaagaaaggcaacagagtggatgtgcccttcatccggcgggaccagaacaagtggaaaacacccgccatgaagaccctgggcagaatctacagcgaggatctgcccgtggaactgcccagacagatgttcgacaatgagatcaagtcccacctgaagtccctgccacagatggaaggcatcgacttcaacaatgccaacgtgacctatctgatcgccgagtacatgaagagagtgctggacgacgacttccagaccttctaccagtggaaccgcaactaccggtacatggacatgcttaagggcgagtacgacagaaagggctccctgcagcactgcttcaccagcgtggaagagagagaaggcctctggaaagagcgggcctccagaacagagcggtacagaaagcaggccagcaacaagatccgcagcaaccggcagatgagaaacgccagcagcgaagagatcgagacaatcctggataagcggctgagcaacagccggaacgagtaccagaaaagcgagaaagtgatccggcgctacagagtgcaggatgccctgctgtttctgctggccaaaaagaccctgaccgaactggccgatttcgacggcgagaggttcaaactgaaagaaatcatgcccgacgccgagaagggaatcctgagcgagatcatgcccatgagcttcaccttcgagaaaggcggcaagaagtacaccatcaccagcgagggcatgaagctgaagaactacggcgacttctttgtgctggctagcgacaagaggatcggcaacctgctggaactcgtgggcagcgacatcgtgtccaaagaggatatcatggaagagttcaacaaatacgaccagtgcaggcccgagatcagctccatcgtgttcaacctggaaaagtgggccttcgacacataccccgagctgtctgccagagtggaccgggaagagaaggtggacttcaagagcatcctgaaaatcctgctgaacaacaagaacatcaacaaagagcagagcgacatcctgcggaagatccggaacgccttcgatcacaacaattaccccgacaaaggcgtggtggaaatcaaggccctgcctgagatcgccatgagcatcaagaaggcctttggggagtacgccatcatgaagacaggcggcggccccggcggcggcgccgccgccggcagcggcagccctaagaaaaaacgaaaagttggcagcggaagcaaaaggccggcggccacgaaaaaggccggccaggcaaaaaagaaaaagctcgagtacccatacgatgttccagattacgcttgagaattccccttgagcatctgacttctggctaataaaggaaatttattttcattgcaatagtgtgttggaattttttgtgtctctcaggtaccgagggcctatttcccatgattccttcatatttgcatatacgatacaaggctgttagagagataattggaattaatttgactgtaaacacaaagatattagtacaaaatacgtgacgtagaaagtaataatttcttgggtagtttgcagttttaaaattatgttttaaaatggactatcatatgcttaccgtaacttgaaagtatttcgatttcttggctttatatatcttgtggaaaggacgaaacaccgtggttggagaactggatgtagatgggctggttgtggaaggtccagttttgaggggctattacaacttttttgcggccgcaggaacccctagtgatggagttggccactccctctctgcgcgctcgctcgctcactgaggccgggcgaccaaaggtcgcccgacgcccgggctttgcccgggcggcctcagtgagcgagcgagcgcgcagctgcctgcaggggcgcctgatgcggtattttctccttacgcatctgtgcggtatttcacaccgcatacgtcaaagcaaccatagtacgcgccctgtagcggcgcattaagcgcggcgggtgtggtggttacgcgcagcgtgaccgctacacttgccagcgccttagcgcccgctcctttcgctttcttcccttcctttctcgccacgttcgccggctttccccgtcaagctctaaatcgggggctccctttagggttccgatttagtgctttacggcacctcgaccccaaaaaacttgatttgggtgatggttcacgtagtgggccatcgccctgatagacggtttttcgccctttgacgttggagtccacgttctttaatagtggactcttgttccaaactggaacaacactcaactctatctcgggctattcttttgatttataagggattttgccgatttcggtctattggttaaaaaatgagctgatttaacaaaaatttaacgcgaattttaacaaaatattaacgtttacaattttatggtgcactctcagtacaatctgctctgatgccgcatagttaagccagccccgacacccgccaacacccgctgacgcgccctgacgggcttgtctgctcccggcatccgcttacagacaagctgtgaccgtctccgggagctgcatgtgtcagaggttttcaccgtcatcaccgaaacgcgcgagacgaaagggcctcgtgatacgcctatttttataggttaatgtcatgataataatggtttcttagacgtcaggtggcacttttcggggaaatgtgcgcggaacccctatttgtttatttttctaaatacattcaaatatgtatccgctcatgagacaataaccctgataaatgcttcaataatattgaaaaaggaagagtatgagtattcaacatttccgtgtcgcccttattcccttttttgcggcattttgccttcctgtttttgctcacccagaaacgctggtgaaagtaaaagatgctgaagatcagttgggtgcacgagtgggttacatcgaactggatctcaacagcggtaagatccttgagagttttcgccccgaagaacgttttccaatgatgagcacttttaaagttctgctatgtggcgcggtattatcccgtattgacgccgggcaagagcaactcggtcgccgcatacactattctcagaatgacttggttgagtactcaccagtcacagaaaagcatcttacggatggcatgacagtaagagaattatgcagtgctgccataaccatgagtgataacactgcggccaacttacttctgacaacgatcggaggaccgaaggagctaaccgcttttttgcacaacatgggggatcatgtaactcgccttgatcgttgggaaccggagctgaatgaagccataccaaacgacgagcgtgacaccacgatgcctgtagcaatggcaacaacgttgcgcaaactattaactggcgaactacttactctagcttcccggcaacaattaatagactggatggaggcggataaagttgcaggaccacttctgcgctcggcccttccggctggctggtttattgctgataaatctggagccggtgagcgtggaagccgcggtatcattgcagcactggggccagatggtaagccctcccgtatcgtagttatctacacgacggggagtcaggcaactatggatgaacgaaatagacagatcgctgagataggtgcctcactgattaagcattggtaactgtcagaccaagtttactcatatatactttagattgatttaaaacttcatttttaatttaaaaggatctaggtgaagatcctttttgataatctcatgaccaaaatcccttaacgtgagttttcgttccactgagcgtcagaccccgtagaaaagatcaaaggatcttcttgagatcctttttttctgcgcgtaatctgctgcttgcaaacaaaaaaaccaccgctaccagcggtggtttgtttgccggatcaagagctaccaactctttttccgaaggtaactggcttcagcagagcgcagataccaaatactgttcttctagtgtagccgtagttaggccaccacttcaagaactctgtagcaccgcctacatacctcgctctgctaatcctgttaccagtggctgctgccagtggcgataagtcgtgtcttaccgggttggactcaagacgatagttaccggataaggcgcagcggtcgggctgaacggggggttcgtgcacacagcccagcttggagcgaacgacctacaccgaactgagatacctacagcgtgagctatgagaaagcgccacgcttcccgaagggagaaaggcggacaggtatccggtaagcggcagggtcggaacaggagagcgcacgagggagcttccagggggaaacgcctggtatctttatagtcctgtcgggtttcgccacctctgacttgagcgtcgatttttgtgatgctcgtcaggggggcggagcctatggaaaaacgccagcaacgcggcctttttacggttcctggccttttgctggccttttgctcacatgt

SEQ ID NO: 93 - DNA, 6447 bp, synthetic construct
  source 1..6447: mol_type = other DNA
cctgcaggcagctgcgcgctcgctcgctcactgaggccgcccgggcgtcgggcgacctttggtcgcccggcctcagtgagcgagcgagcgcgcagagagggagtggccaactccatcactaggggttcctgcggcctctagactcgaggcgttgacattgattattgactagttattaatagtaatcaattacggggtcattagttcatagcccatatatggagttccgcgttacataacttacggtaaatggcccgcctggctgaccgcccaacgacccccgcccattgacgtcaataatgacgtatgttcccatagtaacgccaatagggactttccattgacgtcaatgggtggagtatttacggtaaactgcccacttggcagtacatcaagtgtatcatatgccaagtacgccccctattgacgtcaatgacggtaaatggcccgcctggcattatgcccagtacatgaccttatgggactttcctacttggcagtacatctacgtattagtcatcgctattaccatggtgatgcggttttggcagtacatcaatgggcgtggatagcggtttgactcacggggatttccaagtctccaccccattgacgtcaatgggagtttgttttggcaccaaaatcaacgggactttccaaaatgtcgtaacaactccgccccattgacgcaaatgggcggtaggcgtgtacggtgggaggtctatataagcagagctctctggctaactaccggtgccaccatgccggcagctaagaaaaagaaactggatggcagcgtcgacgcccaggtgtccaaacagaccagcaagaaaagggaactgagcatcgatgagtaccagggtgctagaaagtggtgcttcacaatcgcctttaacaaagctctggtcaatagggataaaaacgatggcctcttcgtggagtccctgctgagacacgagaagtacagcaaacacgactggtacgacgaggataccagagccctgatcaagtgctccactcaggccgccaatgcaaaggccgaggctctgagaaattatttcagccactaccggcactcccccgggtgtctgaccttcactgcagaggatgagcttaggacaattatggagcgcgcctacgagagggccatttttgagtgtcggcgaagagaaactgaggtgatcatcgagtttccatctctgtttgaaggggaccgcatcacaaccgccggagtggtattttttgtgagtttcttcgtggaacggagagtgctggaccggctgtacggggcagttagtggcctgaagaagaacgaggggcagtacaagctgacaaggaaagctctgagcatgtactgtctgaaagattccagatttacaaaggcatgggataagagagtgctcctctttcgcgatatcctggcccagctgggcagaatcccagctgaggcttacgagtactaccacggcgaacagggcgacaaaaagagggccaacgacaatgagggcaccaaccccaaaaggcacaaggataagtttattgagtttgcactgcactacctggaggcccagcactctgagatctgctttggcagaaggcacatcgtgagagaggaagctggcgccggcgatgagcacaagaagcacagaaccaaagggaaggtggtggtggacttctccaagaaggatgaggatcagtcttactacatcagtaagaacaacgtgattgtgaggatcgataagaatgccggccctcgctcctaccgcatggggctcaatgaactgaagtacctggtcctgctctctctgcaggggaagggcgatgacgctatcgccaagctgtataggtatcggcagcatgtggagaacattctggacgtggtgaaggtgactgataaagataaccacgtgttcctgccaaggtttgtgctcgaacagcacggaatcggccggaaggccttcaagcagagaattgacgggcgcgtgaaacatgtgcgcggggtgtgggaaaagaagaaggccgccacaaacgagatgacgctgcacgagaaggcccgcgacatcctccagtacgtgaatgagaattgcactcgcagcttcaatcctggcgagtataacaggctgctggtgtgcctggtgggtaaagacgtggagaacttccaggccggcctgaagcggcttcagctggctgagagaattgacggccgggtgtattctatcttcgcccagacttctaccatcaatgaaatgcaccaggtggtgtgtgaccagatcctcaatcggctgtgtcgaattggggatcagaagctgtacgactatgtgggcctgggcaagaaagatgagatcgactataaacagaaagtggcttggttcaaagagcacatcagtatcagacgcggctttctgaggaagaaattctggtacgactctaaaaagggcttcgctaagctggtggaggagcacctggaatccggaggcggacagcgggatgtggggctggataagaaatactaccacatcgatgccatcgggagattcgagggcgccaatcctgctctgtacgaaaccctggccagggacaggctgtgcctgatgatggcccagtactttctgggctccgttcgcaaagagctgggaaacaaaattgtgtggagcaacgactccatagagctgccggtggagggatctgtcgggaatgaaaaatcgatcgtgttctctgtgagcgattatggaaaactgtacgtcctggacgatgccgagtttctgggtagaatctgtgagtattttatgccacatgaaaagggcaagatcagataccacaccgtgtatgaaaaggggttcagagcctacaacgacctgcagaaaaaatgcgtggaggccgtgctggcattcgaagagaaggtggtgaaggccaagaaaatgtctgagaaagagggagcccactacatcgactttcgcgagatcctggcccagaccatgtgcaaggaagctgaaaagacagccgtcaataaggtgaggagggccttctttcaccaccaccttaaattcgtgatcgacgaatttggcctgttcagcgatgtgatgaaaaaatacggcatcgagaaggagtggaagtttccagtgaaaacaggcggcggccccggcggcggcgccgccgccggcagcggcagccctaagaaaaaacgaaaagttggcagcggaagcaaaaggccggcggccacgaaaaaggccggccaggcaaaaaagaaaaagctcgagtacccatacgatgttccagattacgcttgagaattccccttgagcatctgacttctggctaataaaggaaatttattttcattgcaatagtgtgttggaattttttgtgtctctcaggtaccgagggcctatttcccatgattccttcatatttgcatatacgatacaaggctgttagagagataattggaattaatttgactgtaaacacaaagatattagtacaaaatacgtgacgtagaaagtaataatttcttgggtagtttgcagttttaaaattatgttttaaaatggactatcatatgcttaccgtaacttgaaagtatttcgatttcttggctttatatatcttgtggaaaggacgaaacaccggtggttggagaactggatgtagatgggctggctggagcagcccccgatttgtggggtgattacagcttttttgcggccgcaggaacccctagtgatggagttggccactccctctctgcgcgctcgctcgctcactgaggccgggcgaccaaaggtcgcccgacgcccgggctttgcccgggcggcctcagtgagcgagcgagcgcgcagctgcctgcaggggcgcctgatgcggtattttctccttacgcatctgtgcggtatttcacaccgcatacgtcaaagcaaccatagtacgcgccctgtagcggcgcattaagcgcggcgggtgtggtggttacgcgcagcgtgaccgctacacttgccagcgccttagcgcccgctcctttcgctttcttcccttcctttctcgccacgttcgccggctttccccgtcaagctctaaatcgggggctccctttagggttccgatttagtgctttacggcacctcgaccccaaaaaacttgatttgggtgatggttcacgtagtgggccatcgccctgatagacggtttttcgccctttgacgttggagtccacgttctttaatagtggactcttgttccaaactggaacaacactcaactctatctcgggctattcttttgatttataagggattttgccgatttcggtctattggttaaaaaatgagctgatttaacaaaaatttaacgcgaattttaacaaaatattaacgtttacaattttatggtgcactctcagtacaatctgctctgatgccgcatagttaagccagccccgacacccgccaacacccgctgacgcgccctgacgggcttgtctgctcccggcatccgcttacagacaagctgtgaccgtctccgggagctgcatgtgtcagaggttttcaccgtcatcaccgaaacgcgcgagacgaaagggcctcgtgatacgcctatttttataggttaatgtcatgataataatggtttcttagacgtcaggtggcacttttcggggaaatgtgcgcggaacccctatttgtttatttttctaaatacattcaaatatgtatccgctcatgagacaataaccctgataaatgcttcaataatattgaaaaaggaagagtatgagtattcaacatttccgtgtcgcccttattcccttttttgcggcattttgccttcctgtttttgctcacccagaaacgctggtgaaagtaaaagatgctgaagatcagttgggtgcacgagtgggttacatcgaactggatctcaacagcggtaagatccttgagagttttcgccccgaagaacgttttccaatgatgagcacttttaaagttctgctatgtggcgcggtattatcccgtattgacgccgggcaagagcaactcggtcgccgcatacactattctcagaatgacttggttgagtactcaccagtcacagaaaagcatcttacggatggcatgacagtaagagaattatgcagtgctgccataaccatgagtgataacactgcggccaacttacttctgacaacgatcggaggaccgaaggagctaaccgcttttttgcacaacatgggggatcatgtaactcgccttgatcgttgggaaccggagctgaatgaagccataccaaacgacgagcgtgacaccacgatgcctgtagcaatggcaacaacgttgcgcaaactattaactggcgaactacttactctagcttcccggcaacaattaatagactggatggaggcggataaagttgcaggaccacttctgcgctcggcccttccggctggctggtttattgctgataaatctggagccggtgagcgtggaagccgcggtatcattgcagcactggggccagatggtaagccctcccgtatcgtagttatctacacgacggggagtcaggcaactatggatgaacgaaatagacagatcgctgagataggtgcctcactgattaagcattggtaactgtcagaccaagtttactcatatatactttagattgatttaaaacttcatttttaatttaaaaggatctaggtgaagatcctttttgataatctcatgaccaaaatcccttaacgtgagttttcgttccactgagcgtcagaccccgtagaaaagatcaaaggatcttcttgagatcctttttttctgcgcgtaatctgctgcttgcaaacaaaaaaaccaccgctaccagcggtggtttgtttgccggatcaagagctaccaactctttttccgaaggtaactggcttcagcagagcgcagataccaaatactgttcttctagtgtagccgtagttaggccaccacttcaagaactctgtagcaccgcctacatacctcgctctgctaatcctgttaccagtggctgctgccagtggcgataagtcgtgtcttaccgggttggactcaagacgatagttaccggataaggcgcagcggtcgggctgaacggggggttcgtgcacacagcccagcttggagcgaacgacctacaccgaactgagatacctacagcgtgagctatgagaaagcgccacgcttcccgaagggagaaaggcggacaggtatccggtaagcggcagggtcggaacaggagagcgcacgagggagcttccagggggaaacgcctggtatctttatagtcctgtcgggtttcgccacctctgacttgagcgtcgatttttgtgatgctcgtcaggggggcggagcctatggaaaaacgccagcaacgcggcctttttacggttcctggccttttgctggccttttgctcacatgt

SEQ ID NO: 94 - DNA, 6492 bp, synthetic construct
  source 1..6492: mol_type = other DNA
cctgcaggcagctgcgcgctcgctcgctcactgaggccgcccgggcgtcgggcgacctttggtcgcccggcctcagtgagcgagcgagcgcgcagagagggagtggccaactccatcactaggggttcctgcggcctctagactcgaggcgttgacattgattattgactagttattaatagtaatcaattacggggtcattagttcatagcccatatatggagttccgcgttacataacttacggtaaatggcccgcctggctgaccgcccaacgacccccgcccattgacgtcaataatgacgtatgttcccatagtaacgccaatagggactttccattgacgtcaatgggtggagtatttacggtaaactgcccacttggcagtacatcaagtgtatcatatgccaagtacgccccctattgacgtcaatgacggtaaatggcccgcctggcattatgcccagtacatgaccttatgggactttcctacttggcagtacatctacgtattagtcatcgctattaccatggtgatgcggttttggcagtacatcaatgggcgtggatagcggtttgactcacggggatttccaagtctccaccccattgacgtcaatgggagtttgttttggcaccaaaatcaacgggactttccaaaatgtcgtaacaactccgccccattgacgcaaatgggcggtaggcgtgtacggtgggaggtctatataagcagagctctctggctaactaccggtgccaccatgccggcagctaagaaaaagaaactggatggcagcgtcgacaatggcatcgagctcaaaaaggaggaagccgcattttatttcaaccaggcagaactcaatctgaaggctattgaggataatatcttcgacaaggagagaagaaagaccctgctgaataaccctcagattctggccaagatggaaaattttatttttaactttagagacgtgaccaagaacgccaagggcgaaatcgactgcctgctcctgaagctgcgggagctgagaaatttctactcacattatgtgcacaaaagagatgtgagggaactgagcaagggggagaagccaattctggagaagtattatcagtttgccatcgagtctactggctctgagaacgtgaaactggagatcattgaaaacgacgcctggctggcagacgccggggtgctgttttttctgtgcatcttcctgaaaaagtcccaggcgaacaagttgatcagcggcatctctggttttaagagaaacgacgataccggccaacctcgcagaaacctgttcacttatttcagcatcagggaggggtacaaagtggtgccagagatgcagaaacacttcctgctgttctccctcgtgaatcacctgagcaaccaggacgattacattgagaaggcccaccagccatacgatatcggcgagggcctgttctttcatcgcatcgccagtaccttcctgaacatcagcggaatcctgaggaatatgaagttttacacctatcagagcaaacggctggtggagcagagaggcgagctgaagagagagaaggatattttcgcctgggaggagccatttcagggcaactcctacttcgagatcaatgggcacaaaggagtgattggcgaggacgagctgaaagagctctgctatgccttcctgatcggcaatcaggacgccaacaaggtggagggcaggattacacagtttctggagaagttcagaaacgccaatagcgtgcagcaggtgaaggacgatgagatgctgaaacccgaatacttccccgccaattacttcgcagagagcggggtgggacggatcaaggatcgagtgctgaataggctgaacaaggctatcaagtccaacaaggccaaaaaaggggagattatcgcctatgacaagatgagggaggtgatggccttcatcaacaactcactgcctgtggacgagaagctgaagcccaaagattacaagaggtatctgggcatggtccggttctgggacagggagaaagataatatcaagagggagtttgagactaaggagtggagcaagtatctgccctccaacttctggaccgccaagaacctggagcgcgtgtatggcctggcacgcgagaaaaacgccgaactgttcaataagctgaaagccgatgtggagaagatggacgagcgggagctggagaagtaccagaagatcaatgatgcaaaggacctggccaatttgagacggctcgcctccgactttggagtgaagtgggaggagaaagactgggatgaatacagcggacagatcaagaagcagattacagactcccagaaactgactatcatgaaacagaggatcaccgctggcctgaaaaaaaaacacggaatcgagaatctgaatctgaggatcaccatcgacattaacaaatcccggaaggcggtgctgaacagaattgccatcccccgggggttcgtgaagaggcacatcctgggttggcaggagagcgagaaagtgagcaagaagattagggaggctgaatgtgaaattctgctgtccaaggagtacgaggagctgagcaaacagtttttccagtctaaagactacgacaagatgaccaggataaacggactgtacgagaagaacaagctgatcgccctgatggccgtgtacctcatggggcagctgagaatcctgttcaaagagcacactaagctggacgacatcaccaagactaccgtggacttcaagatcagtgataaggtcaccgtgaaaatccccttcagcaattaccctagcctggtgtacacaatgtcctccaaatacgtggacaatatcgggaactacggattctccaacaaggataaggataagcccattctgggcaaaatcgatgtgatcgaaaaacagagaatggagttcatcaaggaagtgctggggtttgagaagtatcttttcgacgacaagattatcgataaaagtaagttcgcagacaccgccactcacatctcttttgccgagatcgtggaggagctggtggagaagggctgggacaaggaccgcctgactaagctcaaagacgctagaaacaaagccctgcacggcgagatcctgacgggcaccagctttgacgaaaccaagtctctgatcaatgagttgaagaagacaggcggcggccccggcggcggcgccgccgccggcagcggcagccctaagaaaaaacgaaaagttggcagcggaagcaaaaggccggcggccacgaaaaaggccggccaggcaaaaaagaaaaagctcgagtacccatacgatgttccagattacgcttgagaattccccttgagcatctgacttctggctaataaaggaaatttattttcattgcaatagtgtgttggaattttttgtgtctctcaggtaccgagggcctatttcccatgattccttcatatttgcatatacgatacaaggctgttagagagataattggaattaatttgactgtaaacacaaagatattagtacaaaatacgtgacgtagaaagtaataatttcttgggtagtttgcagttttaaaattatgttttaaaatggactatcatatgcttaccgtaacttgaaagtatttcgatttcttggctttatatatcttgtggaaaggacgaaacaccggtggttggagaactggatgtagatgggctggctgtgatagacctcgatttgtggggtagtaacagcttttttgcggccgcaggaacccctagtgatggagttggccactccctctctgcgcgctcgctcgctcactgaggccgggcgaccaaaggtcgcccgacgcccgggctttgcccgggcggcctcagtgagcgagcgagcgcgcagctgcctgcaggggcgcctgatgcggtattttctccttacgcatctgtgcggtatttcacaccgcatacgtcaaagcaaccatagtacgcgccctgtagcggcgcattaagcgcggcgggtgtggtggttacgcgcagcgtgaccgctacacttgccagcgccttagcgcccgctcctttcgctttcttcccttcctttctcgccacgttcgccggctttccccgtcaagctctaaatcgggggctccctttagggttccgatttagtgctttacggcacctcgaccccaaaaaacttgatttgggtgatggttcacgtagtgggccatcgccctgatagacggtttttcgccctttgacgttggagtccacgttctttaatagtggactcttgttccaaactggaacaacactcaactctatctcgggctattcttttgatttataagggattttgccgatttcggtctattggttaaaaaatgagctgatttaacaaaaatttaacgcgaattttaacaaaatattaacgtttacaattttatggtgcactctcagtacaatctgctctgatgccgcatagttaagccagccccgacacccgccaacacccgctgacgcgccctgacgggcttgtctgctcccggcatccgcttacagacaagctgtgaccgtctccgggagctgcatgtgtcagaggttttcaccgtcatcaccgaaacgcgcgagacgaaagggcctcgtgatacgcctatttttataggttaatgtcatgataataatggtttcttagacgtcaggtggcacttttcggggaaatgtgcgcggaacccctatttgtttatttttctaaatacattcaaatatgtatccgctcatgagacaataaccctgataaatgcttcaataatattgaaaaaggaagagtatgagtattcaacatttccgtgtcgcccttattcccttttttgcggcattttgccttcctgtttttgctcacccagaaacgctggtgaaagtaaaagatgctgaagatcagttgggtgcacgagtgggttacatcgaactggatctcaacagcggtaagatccttgagagttttcgccccgaagaacgttttccaatgatgagcacttttaaagttctgctatgtggcgcggtattatcccgtattgacgccgggcaagagcaactcggtcgccgcatacactattctcagaatgacttggttgagtactcaccagtcacagaaaagcatcttacggatggcatgacagtaagagaattatgcagtgctgccataaccatgagtgataacactgcggccaacttacttctgacaacgatcggaggaccgaaggagctaaccgcttttttgcacaacatgggggatcatgtaactcgccttgatcgttgggaaccggagctgaatgaagccataccaaacgacgagcgtgacaccacgatgcctgtagcaatggcaacaacgttgcgcaaactattaactggcgaactacttactctagcttcccggcaacaattaatagactggatggaggcggataaagttgcaggaccacttctgcgctcggcccttccggctggctggtttattgctgataaatctggagccggtgagcgtggaagccgcggtatcattgcagcactggggccagatggtaagccctcccgtatcgtagttatctacacgacggggagtcaggcaactatggatgaacgaaatagacagatcgctgagataggtgcctcactgattaagcattggtaactgtcagaccaagtttactcatatatactttagattgatttaaaacttcatttttaatttaaaaggatctaggtgaagatcctttttgataatctcatgaccaaaatcccttaacgtgagttttcgttccactgagcgtcagaccccgtagaaaagatcaaaggatcttcttgagatcctttttttctgcgcgtaatctgctgcttgcaaacaaaaaaaccaccgctaccagcggtggtttgtttgccggatcaagagctaccaactctttttccgaaggtaactggcttcagcagagcgcagataccaaatactgttcttctagtgtagccgtagttaggccaccacttcaagaactctgtagcaccgcctacatacctcgctctgctaatcctgttaccagtggctgctgccagtggcgataagtcgtgtcttaccgggttggactcaagacgatagttaccggataaggcgcagcggtcgggctgaacggggggttcgtgcacacagcccagcttggagcgaacgacctacaccgaactgagatacctacagcgtgagctatgagaaagcgccacgcttcccgaagggagaaaggcggacaggtatccggtaagcggcagggtcggaacaggagagcgcacgagggagcttccagggggaaacgcctggtatctttatagtcctgtcgggtttcgccacctctgacttgagcgtcgatttttgtgatgctcgtcaggggggcggagcctatggaaaaacgccagcaacgcggcctttttacggttcctggccttttgctggccttttgctcacatgt

SEQ ID NO: 95 - DNA, 70 bp, synthetic construct
  source 1..70: mol_type = other DNA
tgccgttcttctgcttgtcggccatgatatagacgttgtggctgttgtagttgtactccagcttgtgccc

SEQ ID NO: 96 - DNA, 6793 bp, synthetic construct
  source 1..6793: mol_type = other DNA
cctgcaggcagctgcgcgctcgctcgctcactgaggccgcccgggcgtcgggcgacctttggtcgcccggcctcagtgagcgagcgagcgcgcagagagggagtggccaactccatcactaggggttcctgcggcctctagactcgaggcgttgacattgattattgactagttattaatagtaatcaattacggggtcattagttcatagcccatatatggagttccgcgttacataacttacggtaaatggcccgcctggctgaccgcccaacgacccccgcccattgacgtcaataatgacgtatgttcccatagtaacgccaatagggactttccattgacgtcaatgggtggagtatttacggtaaactgcccacttggcagtacatcaagtgtatcatatgccaagtacgccccctattgacgtcaatgacggtaaatggcccgcctggcattatgcccagtacatgaccttatgggactttcctacttggcagtacatctacgtattagtcatcgctattaccatggtgatgcggttttggcagtacatcaatgggcgtggatagcggtttgactcacggggatttccaagtctccaccccattgacgtcaatgggagtttgttttggcaccaaaatcaacgggactttccaaaatgtcgtaacaactccgccccattgacgcaaatgggcggtaggcgtgtacggtgggaggtctatataagcagagctctctggctaactaccggtgccaccatgccggcagctaagaaaaagaaactggatggcagcgtcgacatgagcaaggacaagaaaaccaaggccaagagaatgggcgtgaaggccctgctggcccacggcgaggacaagctgaccatgaccaccttcggcaagggcaacagaagcaagatcgagttcaccgagggctaccacggcagagccctggagacacccaagcacttcggcatcagaggcttcgaggtgagaagaatcgacgagaacgtggacctgtgcggcgacctggaggagggcaagaccatcgaggccctgctggtgaaccccagcgagaaggtgggcgaggactacctgaagctgaagggcaccctggagaagagattcttcggcagagagttcccccacgacaacatcagaatccagctgatctacaacatcctggacatctacaagatcctgggcatgaacgtggccgacatcctgtacgccctgggcaacatgcaggacaccgagctggacatcgacatgttcggccagagcctgaacaacgaggacaacctgaaggagtgcctgaagagaatgaggccctacatgggctacttcggcgacatcttcaagatcagccccaagggcgagaacatcgccgacagagagcacaacaagaaggtgctgagatgcatcagcgtgctggcaaacgccaccgccgccgacaagcaggacgagtacccctggttcaagagcagcgacatctacgagacaaagatcttcaaggccgacatgtggaagatcatcaaggaccagtacagagagaagatcaagaaggtgaacaaggacttcctgagcaagaacgccgtgaacatggccatcctgttcgacctgctgaacgccagagacgtggagcagaagaagcagatcaccgacgagttctacagattcaccatcagaaaggacggcaagaacctgggcatgaacctggtgaagatcagagagatcatcatcgacagatacgccagcggcctgagagacaagaagcacgacccccacagacagaagatcaacgtgatcgccgacttcctgatcttcagagccctgagccagaaccagggcatcatcgacaagaccgtgagcagcctgagactgaccaaggacgaggaggagaaggaccacgtgtaccagaacgccgccgagctggtgtggggcatggtgagcaactgcctgaccccctacttcaacgaccccaagaacaagtacatcctgaagtacaaggacgccaagacccccggcgacttcgaggactggatcaccagcaagatcagcgaggacgacggcgagcccttcgtgaaggtgctgagcttcctgtgcaacttcctggagggcaaggagatcaacgagctgctgaccgcctacatccacaagttcgagtgcatccaggacttcctgaacgtgatcagcagcctgggcgagaacgtgcagttccagcccagattcgccctgttcaacaacgccagcttcgcccagaacgtggccgtgcagctgagaatcctggccagcatcggcaagatgaagcccgacctgaccgaggccaagaggcccctgtacaaggccgccatcagaatgctgtgcccccccgagaagtgggagaagtacaccagcgacgagtggctggagaagaacatgctgctgaacagcgaggacagaaagaacgacaagaagaagaagcaggtgaaccccttcagaaacttcatcgccggcaacgtgatcgagagcagaagattcatgtacctggtgagatacagcaagcccaaggccgtgagagccatcatgcagaacagaagcatcgtgaactacgtgctgcacagactgcccagcgagcaggtgcacagatacgccagcgtgttccccgagaacttcgccgacctggagcaggagatcgacttcctgaccaagaagctgttcgagttcagcttcgaggagctgctgcacgagaaggacgtgatcctgaacaacagcagaagccacaagcccagcctggagatcgagagactgaaggccatcaccggcctgtacctgagcgtggcctacatcgccatcaagaacatcgtgaaggccaacgccagatactacatcgccttcgccgtgttcgagagagacaaggagctggtgaaggccaaggacgccagaatccagaccaagatccccgagacagacttccccgactacttctgcctgacccagtactacctggacagagacgaggagaagaagttccccggcgaccccagagacaaggaggccttcttcgagcacctggcaaagaccaagagagccttcagcaagcagtggagagagtggctgaacgagaagatcgccgacgccaagagcagccaggccaccggcctgctgctgagagaggccgcaaacgacgtggaggccctgaacgtgctgagagccatccccgactacatccaggacttcagacacggcgagaagggcgagacagccatgaacagctacttcgagctgtaccactacctgatgcagagactgatgctgaagaacaccgagctggacctgagccactggagcggctggatcatgagaagcggcagacccgacagagacttgatccagatcgccttcgtgagcctggcctacaacctgcccagatacagaaacctgaccaaggagcaccacttcgacgacaccgtgctgcagaagatcagagagaaggagagcctggacacaggcggcggccccggcggcggcgccgccgccggcagcggcagccctaagaaaaaacgaaaagttggcagcggaagcaaaaggccggcggccacgaaaaaggccggccaggcaaaaaagaaaaagctcgagtacccatacgatgttccagattacgcttgagaattccccttgagcatctgacttctggctaataaaggaaatttattttcattgcaatagtgtgttggaattttttgtgtctctcaggtaccgagggcctatttcccatgattccttcatatttgcatatacgatacaaggctgttagagagataattggaattaatttgactgtaaacacaaagatattagtacaaaatacgtgacgtagaaagtaataatttcttgggtagtttgcagttttaaaattatgttttaaaatggactatcatatgcttaccgtaacttgaaagtatttcgatttcttggctttatatatcttgtggaaaggacgaaacaccggaagataactctacaaacctgtagggttctgagacggagaccacggcaggtctcattttttgcggccgcaggaacccctagtgatggagttggccactccctctctgcgcgctcgctcgctcactgaggccgggcgaccaaaggtcgcccgacgcccgggctttgcccgggcggcctcagtgagcgagcgagcgcgcagctgcctgcaggggcgcctgatgcggtattttctccttacgcatctgtgcggtatttcacaccgcatacgtcaaagcaaccatagtacgcgccctgtagcggcgcattaagcgcggcgggtgtggtggttacgcgcagcgtgaccgctacacttgccagcgccttagcgcccgctcctttcgctttcttcccttcctttctcgccacgttcgccggctttccccgtcaagctctaaatcgggggctccctttagggttccgatttagtgctttacggcacctcgaccccaaaaaacttgatttgggtgatggttcacgtagtgggccatcgccctgatagacggtttttcgccctttgacgttggagtccacgttctttaatagtggactcttgttccaaactggaacaacactcaactctatctcgggctattcttttgatttataagggattttgccgatttcggtctattggttaaaaaatgagctgatttaacaaaaatttaacgcgaattttaacaaaatattaacgtttacaattttatggtgcactctcagtacaatctgctctgatgccgcatagttaagccagccccgacacccgccaacacccgctgacgcgccctgacgggcttgtctgctcccggcatccgcttacagacaagctgtgaccgtctccgggagctgcatgtgtcagaggttttcaccgtcatcaccgaaacgcgcgagacgaaagggcctcgtgatacgcctatttttataggttaatgtcatgataataatggtttcttagacgtcaggtggcacttttcggggaaatgtgcgcggaacccctatttgtttatttttctaaatacattcaaatatgtatccgctcatgagacaataaccctgataaatgcttcaataatattgaaaaaggaagagtatgagtattcaacatttccgtgtcgcccttattcccttttttgcggcattttgccttcctgtttttgctcacccagaaacgctggtgaaagtaaaagatgctgaagatcagttgggtgcacgagtgggttacatcgaactggatctcaacagcggtaagatccttgagagttttcgccccgaagaacgttttccaatgatgagcacttttaaagttctgctatgtggcgcggtattatcccgtattgacgccgggcaagagcaactcggtcgccgcatacactattctcagaatgacttggttgagtactcaccagtcacagaaaagcatcttacggatggcatgacagtaagagaattatgcagtgctgccataaccatgagtgataacactgcggccaacttacttctgacaacgatcggaggaccgaaggagctaaccgcttttttgcacaacatgggggatcatgtaactcgccttgatcgttgggaaccggagctgaatgaagccataccaaacgacgagcgtgacaccacgatgcctgtagcaatggcaacaacgttgcgcaaactattaactggcgaactacttactctagcttcccggcaacaattaatagactggatggaggcggataaagttgcaggaccacttctgcgctcggcccttccggctggctggtttattgctgataaatctggagccggtgagcgtggaagccgcggtatcattgcagcactggggccagatggtaagccctcccgtatcgtagttatctacacgacggggagtcaggcaactatggatgaacgaaatagacagatcgctgagataggtgcctcactgattaagcattggtaactgtcagaccaagtttactcatatatactttagattgatttaaaacttcatttttaatttaaaaggatctaggtgaagatcctttttgataatctcatgaccaaaatcccttaacgtgagttttcgttccactgagcgtcagaccccgtagaaaagatcaaaggatcttcttgagatcctttttttctgcgcgtaatctgctgcttgcaaacaaaaaaaccaccgctaccagcggtggtttgtttgccggatcaagagctaccaactctttttccgaaggtaactggcttcagcagagcgcagataccaaatactgttcttctagtgtagccgtagttaggccaccacttcaagaactctgtagcaccgcctacatacctcgctctgctaatcctgttaccagtggctgctgccagtggcgataagtcgtgtcttaccgggttggactcaagacgatagttaccggataaggcgcagcggtcgggctgaacggggggttcgtgcacacagcccagcttggagcgaacgacctacaccgaactgagatacctacagcgtgagctatgagaaagcgccacgcttcccgaagggagaaaggcggacaggtatccggtaagcggcagggtcggaacaggagagcgcacgagggagcttccagggggaaacgcctggtatctttatagtcctgtcgggtttcgccacctctgacttgagcgtcgatttttgtgatgctcgtcaggggggcggagcctatggaaaaacgccagcaacgcggcctttttacggttcctggccttttgctggccttttgctcacatgt

SEQ ID NO: 97 - DNA, 7830 bp, synthetic construct
  source 1..7830: mol_type = other DNA
cctgcaggcagctgcgcgctcgctcgctcactgaggccgcccgggcgtcgggcgacctttggtcgcccggcctcagtgagcgagcgagcgcgcagagagggagtggccaactccatcactaggggttcctgcggcctctagactcgaggcgttgacattgattattgactagttattaatagtaatcaattacggggtcattagttcatagcccatatatggagttccgcgttacataacttacggtaaatggcccgcctggctgaccgcccaacgacccccgcccattgacgtcaataatgacgtatgttcccatagtaacgccaatagggactttccattgacgtcaatgggtggagtatttacggtaaactgcccacttggcagtacatcaagtgtatcatatgccaagtacgccccctattgacgtcaatgacggtaaatggcccgcctggcattatgcccagtacatgaccttatgggactttcctacttggcagtacatctacgtattagtcatcgctattaccatggtgatgcggttttggcagtacatcaatgggcgtggatagcggtttgactcacggggatttccaagtctccaccccattgacgtcaatgggagtttgttttggcaccaaaatcaacgggactttccaaaatgtcgtaacaactccgccccattgacgcaaatgggcggtaggcgtgtacggtgggaggtctatataagcagagctctctggctaactaccggtgccaccatgagcaaggacaagaaaaccaaggccaagagaatgggcgtgaaggccctgctggcccacggcgaggacaagctgaccatgaccaccttcggcaagggcaacagaagcaagatcgagttcaccgagggctaccacggcagagccctggagacacccaagcacttcggcatcagaggcttcgaggtgagaagaatcgacgagaacgtggacctgtgcggcgacctggaggagggcaagaccatcgaggccctgctggtgaaccccagcgagaaggtgggcgaggactacctgaagctgaagggcaccctggagaagagattcttcggcagagagttcccccacgacaacatcagaatccagctgatctacaacatcctggacatctacaagatcctgggcatgaacgtggccgacatcctgtacgccctgggcaacatgcaggacaccgagctggacatcgacatgttcggccagagcctgaacaacgaggacaacctgaaggagtgcctgaagagaatgaggccctacatgggctacttcggcgacatcttcaagatcagccccaagggcgagaacatcgccgacagagagcacaacaagaaggtgctgagatgcatcagcgtgctggcaaacgccaccgccgccgacaagcaggacgagtacccctggttcaagagcagcgacatctacgagacaaagatcttcaaggccgacatgtggaagatcatcaaggaccagtacagagagaagatcaagaaggtgaacaaggacttcctgagcaagaacgccgtgaacatggccatcctgttcgacctgctgaacgccagagacgtggagcagaagaagcagatcaccgacgagttctacagattcaccatcagaaaggacggcaagaacctgggcatgaacctggtgaagatcagagagatcatcatcgacagatacgccagcggcctgagagacaagaagcacgacccccacagacagaagatcaacgtgatcgccgacttcctgatcttcagagccctgagccagaaccagggcatcatcgacaagaccgtgagcagcctgagactgaccaaggacgaggaggagaaggaccacgtgtaccagaacgccgccgagctggtgtggggcatggtgagcaactgcctgaccccctacttcaacgaccccaagaacaagtacatcctgaagtacaaggacgccaagacccccggcgacttcgaggactggatcaccagcaagatcagcgaggacgacggcgagcccttcgtgaaggtgctgagcttcctgtgcaacttcctggagggcaaggagatcaacgagctgctgaccgcctacatccacaagttcgagtgcatccaggacttcctgaacgtgatcagcagcctgggcgagaacgtgcagttccagcccagattcgccctgttcaacaacgccagcttcgcccagaacgtggccgtgcagctgagaatcctggccagcatcggcaagatgaagcccgacctgaccgaggccaagaggcccctgtacaaggccgccatcagaatgctgtgcccccccgagaagtgggagaagtacaccagcgacgagtggctggagaagaacatgctgctgaacagcgaggacagaaagaacgacaagaagaagaagcaggtgaaccccttcagaaacttcatcgccggcaacgtgatcgagagcagaagattcatgtacctggtgagatacagcaagcccaaggccgtgagagccatcatgcagaacagaagcatcgtgaactacgtgctgcacagactgcccagcgagcaggtgcacagatacgccagcgtgttccccgagaacttcgccgacctggagcaggagatcgacttcctgaccaagaagctgttcgagttcagcttcgaggagctgctgcacgagaaggacgtgatcctgaacaacagcagaagccacaagcccagcctggagatcgagagactgaaggccatcaccggcctgtacctgagcgtggcctacatcgccatcaagaacatcgtgaaggccaacgccagatactacatcgccttcgccgtgttcgagagagacaaggagctggtgaaggccaaggacgccagaatccagaccaagatccccgagacagacttccccgactacttctgcctgacccagtactacctggacagagacgaggagaagaagttccccggcgaccccagagacaaggaggccttcttcgagcacctggcaaagaccaagagagccttcagcaagcagtggagagagtggctgaacgagaagatcgccgacgccaagagcagccaggccaccggcctgctgctgagagaggccgcaaacgacgtggaggccctgaacgtgctgagagccatccccgactacatccaggacttcagacacggcgagaagggcgagacagccatgaacagctacttcgagctgtaccactacctgatgcagagactgatgctgaagaacaccgagctggacctgagccactggagcggctggatcatgagaagcggcagacccgacagagacttgatccagatcgccttcgtgagcctggcctacaacctgcccagatacagaaacctgaccaaggagcaccacttcgacgacaccgtgctgcagaagatcagagagaaggagagcctggacctgcctccacttgaaagactgacactgggatcccagctgcatttaccgcaggttttagctgacgctgtctcacgcctggtcctgggtaagtttggtgacctgaccgacaacttctcctcccctcacgctcgcagaaaagtgctggctggagtcgtcatgacaacaggcacagatgttaaagatgccaaggtgataagtgtttctacaggaggcaaatgtattaatggtgaatacatgagtgatcgtggccttgcattaaatgactgccatgcagaaataatatctcggagatccttgctcagatttctttatacacaacttgagctttacttaaataacaaagatgatcaaaaaagatccatctttcagaaatcagagcgaggggggtttaggctgaaggagaatgtccagtttcatctgtacatcagcacctctccctgtggagatgccagaatcttctcaccacatgagccaatcctggaagaaccagcagatagacacccaaatcgtaaagcaagaggacagctacggaccaaaatagagtctggtcaggggacgattccagtgcgctccaatgcgagcatccaaacgtgggacggggtgctgcaaggggagcggctgctcaccatgtcctgcagtgacaagattgcacgctggaacgtggtgggcatccagggatcactgctcagcattttcgtggagcccatttacttctcgagcatcatcctgggcagcctttaccacggggaccacctttccagggccatgtaccagcggatctccaacatagaggacctgccacctctctacaccctcaacaagcctttgctcagtggcatcagcaatgcagaagcacggcagccagggaaggcccccaacttcagtgtcaactggacggtaggcgactccgctattgaggtcatcaacgccacgactgggaaggatgagctgggccgcgcgtcccgcctgtgtaagcacgcgttgtactgtcgctggatgcgtgtgcacggcaaggttccctcccacttactacgctccaagattaccaagcccaacgtgtaccatgagtccaagctggcggcaaaggagtaccaggccgccaaggcgcgtctgttcacagccttcatcaaggcggggctgggggcctgggtggagaagcccaccgagcaggaccagttctcactcacgtaagaattccccttgagcatctgacttctggctaataaaggaaatttattttcattgcaatagtgtgttggaattttttgtgtctctcaggtaccgagggcctatttcccatgattccttcatatttgcatatacgatacaaggctgttagagagataattggaattaatttgactgtaaacacaaagatattagtacaaaatacgtgacgtagaaagtaataatttcttgggtagtttgcagttttaaaattatgttttaaaatggactatcatatgcttaccgtaacttgaaagtatttcgatttcttggctttatatatcttgtggaaaggacgaaacaccggaagataactctacaaacctgtagggttctgagactgccgttcttctgcttgtcggccatgatatagacgttgtggctgttgtagttgtactccagcttgtgcccttttttgcggccgcaggaacccctagtgatggagttggccactccctctctgcgcgctcgctcgctcactgaggccgggcgaccaaaggtcgcccgacgcccgggctttgcccgggcggcctcagtgagcgagcgagcgcgcagctgcctgcaggggcgcctgatgcggtattttctccttacgcatctgtgcggtatttcacaccgcatacgtcaaagcaaccatagtacgcgccctgtagcggcgcattaagcgcggcgggtgtggtggttacgcgcagcgtgaccgctacacttgccagcgccttagcgcccgctcctttcgctttcttcccttcctttctcgccacgttcgccggctttccccgtcaagctctaaatcgggggctccctttagggttccgatttagtgctttacggcacctcgaccccaaaaaacttgatttgggtgatggttcacgtagtgggccatcgccctgatagacggtttttcgccctttgacgttggagtccacgttctttaatagtggactcttgttccaaactggaacaacactcaactctatctcgggctattcttttgatttataagggattttgccgatttcggtctattggttaaaaaatgagctgatttaacaaaaatttaacgcgaattttaacaaaatattaacgtttacaattttatggtgcactctcagtacaatctgctctgatgccgcatagttaagccagccccgacacccgccaacacccgctgacgcgccctgacgggcttgtctgctcccggcatccgcttacagacaagctgtgaccgtctccgggagctgcatgtgtcagaggttttcaccgtcatcaccgaaacgcgcgagacgaaagggcctcgtgatacgcctatttttataggttaatgtcatgataataatggtttcttagacgtcaggtggcacttttcggggaaatgtgcgcggaacccctatttgtttatttttctaaatacattcaaatatgtatccgctcatgagacaataaccctgataaatgcttcaataatattgaaaaaggaagagtatgagtattcaacatttccgtgtcgcccttattcccttttttgcggcattttgccttcctgtttttgctcacccagaaacgctggtgaaagtaaaagatgctgaagatcagttgggtgcacgagtgggttacatcgaactggatctcaacagcggtaagatccttgagagttttcgccccgaagaacgttttccaatgatgagcacttttaaagttctgctatgtggcgcggtattatcccgtattgacgccgggcaagagcaactcggtcgccgcatacactattctcagaatgacttggttgagtactcaccagtcacagaaaagcatcttacggatggcatgacagtaagagaattatgcagtgctgccataaccatgagtgataacactgcggccaacttacttctgacaacgatcggaggaccgaaggagctaaccgcttttttgcacaacatgggggatcatgtaactcgccttgatcgttgggaaccggagctgaatgaagccataccaaacgacgagcgtgacaccacgatgcctgtagcaatggcaacaacgttgcgcaaactattaactggcgaactacttactctagcttcccggcaacaattaatagactggatggaggcggataaagttgcaggaccacttctgcgctcggcccttccggctggctggtttattgctgataaatctggagccggtgagcgtggaagccgcggtatcattgcagcactggggccagatggtaagccctcccgtatcgtagttatctacacgacggggagtcaggcaactatggatgaacgaaatagacagatcgctgagataggtgcctcactgattaagcattggtaactgtcagaccaagtttactcatatatactttagattgatttaaaacttcatttttaatttaaaaggatctaggtgaagatcctttttgataatctcatgaccaaaatcccttaacgtgagttttcgttccactgagcgtcagaccccgtagaaaagatcaaaggatcttcttgagatcctttttttctgcgcgtaatctgctgcttgcaaacaaaaaaaccaccgctaccagcggtggtttgtttgccggatcaagagctaccaactctttttccgaaggtaactggcttcagcagagcgcagataccaaatactgttcttctagtgtagccgtagttaggccaccacttcaagaactctgtagcaccgcctacatacctcgctctgctaatcctgttaccagtggctgctgccagtggcgataagtcgtgtcttaccgggttggactcaagacgatagttaccggataaggcgcagcggtcgggctgaacggggggttcgtgcacacagcccagcttggagcgaacgacctacaccgaactgagatacctacagcgtgagctatgagaaagcgccacgcttcccgaagggagaaaggcggacaggtatccggtaagcggcagggtcggaacaggagagcgcacgagggagcttccagggggaaacgcctggtatctttatagtcctgtcgggtttcgccacctctgacttgagcgtcgatttttgtgatgctcgtcaggggggcggagcctatggaaaaacgccagcaacgcggcctttttacggttcctggccttttgctggccttttgctcacatgt

SEQ ID NO: 98 - DNA, 7892 bp, synthetic construct
  source 1..7892: mol_type = other DNA
cctgcaggcagctgcgcgctcgctcgctcactgaggccgcccgggcgtcgggcgacctttggtcgcccggcctcagtgagcgagcgagcgcgcagagagggagtggccaactccatcactaggggttcctgcggcctctagactcgaggcgttgacattgattattgactagttattaatagtaatcaattacggggtcattagttcatagcccatatatggagttccgcgttacataacttacggtaaatggcccgcctggctgaccgcccaacgacccccgcccattgacgtcaataatgacgtatgttcccatagtaacgccaatagggactttccattgacgtcaatgggtggagtatttacggtaaactgcccacttggcagtacatcaagtgtatcatatgccaagtacgccccctattgacgtcaatgacggtaaatggcccgcctggcattatgcccagtacatgaccttatgggactttcctacttggcagtacatctacgtattagtcatcgctattaccatggtgatgcggttttggcagtacatcaatgggcgtggatagcggtttgactcacggggatttccaagtctccaccccattgacgtcaatgggagtttgttttggcaccaaaatcaacgggactttccaaaatgtcgtaacaactccgccccattgacgcaaatgggcggtaggcgtgtacggtgggaggtctatataagcagagctctctggctaactaccggtgccaccatgagcaaggacaagaaaaccaaggccaagagaatgggcgtgaaggccctgctggcccacggcgaggacaagctgaccatgaccaccttcggcaagggcaacagaagcaagatcgagttcaccgagggctaccacggcagagccctggagacacccaagcacttcggcatcagaggcttcgaggtgagaagaatcgacgagaacgtggacctgtgcggcgacctggaggagggcaagaccatcgaggccctgctggtgaaccccagcgagaaggtgggcgaggactacctgaagctgaagggcaccctggagaagagattcttcggcagagagttcccccacgacaacatcagaatccagctgatctacaacatcctggacatctacaagatcctgggcatgaacgtggccgacatcctgtacgccctgggcaacatgcaggacaccgagctggacatcgacatgttcggccagagcctgaacaacgaggacaacctgaaggagtgcctgaagagaatgaggccctacatgggctacttcggcgacatcttcaagatcagccccaagggcgagaacatcgccgacagagagcacaacaagaaggtgctgagatgcatcagcgtgctggcaaacgccaccgccgccgacaagcaggacgagtacccctggttcaagagcagcgacatctacgagacaaagatcttcaaggccgacatgtggaagatcatcaaggaccagtacagagagaagatcaagaaggtgaacaaggacttcctgagcaagaacgccgtgaacatggccatcctgttcgacctgctgaacgccagagacgtggagcagaagaagcagatcaccgacgagttctacagattcaccatcagaaaggacggcaagaacctgggcatgaacctggtgaagatcagagagatcatcatcgacagatacgccagcggcctgagagacaagaagcacgacccccacagacagaagatcaacgtgatcgccgacttcctgatcttcagagccctgagccagaaccagggcatcatcgacaagaccgtgagcagcctgagactgaccaaggacgaggaggagaaggaccacgtgtaccagaacgccgccgagctggtgtggggcatggtgagcaactgcctgaccccctacttcaacgaccccaagaacaagtacatcctgaagtacaaggacgccaagacccccggcgacttcgaggactggatcaccagcaagatcagcgaggacgacggcgagcccttcgtgaaggtgctgagcttcctgtgcaacttcctggagggcaaggagatcaacgagctgctgaccgcctacatccacaagttcgagtgcatccaggacttcctgaacgtgatcagcagcctgggcgagaacgtgcagttccagcccagattcgccctgttcaacaacgccagcttcgcccagaacgtggccgtgcagctgagaatcctggccagcatcggcaagatgaagcccgacctgaccgaggccaagaggcccctgtacaaggccgccatcagaatgctgtgcccccccgagaagtgggagaagtacaccagcgacgagtggctggagaagaacatgctgctgaacagcgaggacagaaagaacgacaagaagaagaagcaggtgaaccccttcagaaacttcatcgccggcaacgtgatcgagagcagaagattcatgtacctggtgagatacagcaagcccaaggccgtgagagccatcatgcagaacagaagcatcgtgaactacgtgctgcacagactgcccagcgagcaggtgcacagatacgccagcgtgttccccgagaacttcgccgacctggagcaggagatcgacttcctgaccaagaagctgttcgagttcagcttcgaggagctgctgcacgagaaggacgtgatcctgaacaacagcagaagccacaagcccagcctggagatcgagagactgaaggccatcaccggcctgtacctgagcgtggcctacatcgccatcaagaacatcgtgaaggccaacgccagatactacatcgccttcgccgtgttcgagagagacaaggagctggtgaaggccaaggacgccagaatccagaccaagatccccgagacagacttccccgactacttctgcctgacccagtactacctggacagagacgaggagaagaagttccccggcgaccccagagacaaggaggccttcttcgagcacctggcaaagaccaagagagccttcagcaagcagtggagagagtggctgaacgagaagatcgccgacgccaagagcagccaggccaccggcctgctgctgagagaggccgcaaacgacgtggaggccctgaacgtgctgagagccatccccgactacatccaggacttcagacacggcgagaagggcgagacagccatgaacagctacttcgagctgtaccactacctgatgcagagactgatgctgaagaacaccgagctggacctgagccactggagcggctggatcatgagaagcggcagacccgacagagacttgatccagatcgccttcgtgagcctggcctacaacctgcccagatacagaaacctgaccaaggagcaccacttcgacgacaccgtgctgcagaagatcagagagaaggagagcctggacggatcccttcaactgcctccacttgaaagactgacactgggatcccagctgcatttaccgcaggttttagctgacgctgtctcacgcctggtcctgggtaagtttggtgacctgaccgacaacttctcctcccctcacgctcgcagaaaagtgctggctggagtcgtcatgacaacaggcacagatgttaaagatgccaaggtgataagtgtttctacaggaggcaaatgtattaatggtgaatacatgagtgatcgtggccttgcattaaatgactgccatgcagaaataatatctcggagatccttgctcagatttctttatacacaacttgagctttacttaaataacaaagatgatcaaaaaagatccatctttcagaaatcagagcgaggggggtttaggctgaaggagaatgtccagtttcatctgtacatcagcacctctccctgtggagatgccagaatcttctcaccacatgagccaatcctggaagaaccagcagatagacacccaaatcgtaaagcaagaggacagctacggaccaaaatagagtctggtcaggggacgattccagtgcgctccaatgcgagcatccaaacgtgggacggggtgctgcaaggggagcggctgctcaccatgtcctgcagtgacaagattgcacgctggaacgtggtgggcatccagggatcactgctcagcattttcgtggagcccatttacttctcgagcatcatcctgggcagcctttaccacggggaccacctttccagggccatgtaccagcggatctccaacatagaggacctgccacctctctacaccctcaacaagcctttgctcagtggcatcagcaatgcagaagcacggcagccagggaaggcccccaacttcagtgtcaactggacggtaggcgactccgctattgaggtcatcaacgccacgactgggaaggatgagctgggccgcgcgtcccgcctgtgtaagcacgcgttgtactgtcgctggatgcgtgtgcacggcaaggttccctcccacttactacgctccaagattaccaagcccaacgtgtaccatgagtccaagctggcggcaaaggagtaccaggccgccaaggcgcgtctgttcacagccttcatcaaggcggggctgggggcctgggtggagaagcccaccgagcaggaccagttctcactcacgtaagcggccgctcgagtctagagggcccgtttaaacccgctgatcagcctcgagaattccccttgagcatctgacttctggctaataaaggaaatttattttcattgcaatagtgtgttggaattttttgtgtctctcaggtaccgagggcctatttcccatgattccttcatatttgcatatacgatacaaggctgttagagagataattggaattaatttgactgtaaacacaaagatattagtacaaaatacgtgacgtagaaagtaataatttcttgggtagtttgcagttttaaaattatgttttaaaatggactatcatatgcttaccgtaacttgaaagtatttcgatttcttggctttatatatcttgtggaaaggacgaaacaccggaagataactctacaaacctgtagggttctgagactgccgttcttctgcttgtcggccatgatatagacgttgtggctgttgtagttgtactccagcttgtgcccttttttgcggccgcaggaacccctagtgatggagttggccactccctctctgcgcgctcgctcgctcactgaggccgggcgaccaaaggtcgcccgacgcccgggctttgcccgggcggcctcagtgagcgagcgagcgcgcagctgcctgcaggggcgcctgatgcggtattttctccttacgcatctgtgcggtatttcacaccgcatacgtcaaagcaaccatagtacgcgccctgtagcggcgcattaagcgcggcgggtgtggtggttacgcgcagcgtgaccgctacacttgccagcgccttagcgcccgctcctttcgctttcttcccttcctttctcgccacgttcgccggctttccccgtcaagctctaaatcgggggctccctttagggttccgatttagtgctttacggcacctcgaccccaaaaaacttgatttgggtgatggttcacgtagtgggccatcgccctgatagacggtttttcgccctttgacgttggagtccacgttctttaatagtggactcttgttccaaactggaacaacactcaactctatctcgggctattcttttgatttataagggattttgccgatttcggtctattggttaaaaaatgagctgatttaacaaaaatttaacgcgaattttaacaaaatattaacgtttacaattttatggtgcactctcagtacaatctgctctgatgccgcatagttaagccagccccgacacccgccaacacccgctgacgcgccctgacgggcttgtctgctcccggcatccgcttacagacaagctgtgaccgtctccgggagctgcatgtgtcagaggttttcaccgtcatcaccgaaacgcgcgagacgaaagggcctcgtgatacgcctatttttataggttaatgtcatgataataatggtttcttagacgtcaggtggcacttttcggggaaatgtgcgcggaacccctatttgtttatttttctaaatacattcaaatatgtatccgctcatgagacaataaccctgataaatgcttcaataatattgaaaaaggaagagtatgagtattcaacatttccgtgtcgcccttattcccttttttgcggcattttgccttcctgtttttgctcacccagaaacgctggtgaaagtaaaagatgctgaagatcagttgggtgcacgagtgggttacatcgaactggatctcaacagcggtaagatccttgagagttttcgccccgaagaacgttttccaatgatgagcacttttaaagttctgctatgtggcgcggtattatcccgtattgacgccgggcaagagcaactcggtcgccgcatacactattctcagaatgacttggttgagtactcaccagtcacagaaaagcatcttacggatggcatgacagtaagagaattatgcagtgctgccataaccatgagtgataacactgcggccaacttacttctgacaacgatcggaggaccgaaggagctaaccgcttttttgcacaacatgggggatcatgtaactcgccttgatcgttgggaaccggagctgaatgaagccataccaaacgacgagcgtgacaccacgatgcctgtagcaatggcaacaacgttgcgcaaactattaactggcgaactacttactctagcttcccggcaacaattaatagactggatggaggcggataaagttgcaggaccacttctgcgctcggcccttccggctggctggtttattgctgataaatctggagccggtgagcgtggaagccgcggtatcattgcagcactggggccagatggtaagccctcccgtatcgtagttatctacacgacggggagtcaggcaactatggatgaacgaaatagacagatcgctgagataggtgcctcactgattaagcattggtaactgtcagaccaagtttactcatatatactttagattgatttaaaacttcatttttaatttaaaaggatctaggtgaagatcctttttgataatctcatgaccaaaatcccttaacgtgagttttcgttccactgagcgtcagaccccgtagaaaagatcaaaggatcttcttgagatcctttttttctgcgcgtaatctgctgcttgcaaacaaaaaaaccaccgctaccagcggtggtttgtttgccggatcaagagctaccaactctttttccgaaggtaactggcttcagcagagcgcagataccaaatactgttcttctagtgtagccgtagttaggccaccacttcaagaactctgtagcaccgcctacatacctcgctctgctaatcctgttaccagtggctgctgccagtggcgataagtcgtgtcttaccgggttggactcaagacgatagttaccggataaggcgcagcggtcgggctgaacggggggttcgtgcacacagcccagcttggagcgaacgacctacaccgaactgagatacctacagcgtgagctatgagaaagcgccacgcttcccgaagggagaaaggcggacaggtatccggtaagcggcagggtcggaacaggagagcgcacgagggagcttccagggggaaacgcctggtatctttatagtcctgtcgggtttcgccacctctgacttgagcgtcgatttttgtgatgctcgtcaggggggcggagcctatggaaaaacgccagcaacgcggcctttttacggttcctggccttttgctggccttttgctcacatgt

SEQ ID NO: 99 - DNA, 7943 bp, synthetic construct
  source 1..7943: mol_type = other DNA
cctgcaggcagctgcgcgctcgctcgctcactgaggccgcccgggcgtcgggcgacctttggtcgcccggcctcagtgagcgagcgagcgcgcagagagggagtggccaactccatcactaggggttcctgcggcctctagactcgaggcgttgacattgattattgactagttattaatagtaatcaattacggggtcattagttcatagcccatatatggagttccgcgttacataacttacggtaaatggcccgcctggctgaccgcccaacgacccccgcccattgacgtcaataatgacgtatgttcccatagtaacgccaatagggactttccattgacgtcaatgggtggagtatttacggtaaactgcccacttggcagtacatcaagtgtatcatatgccaagtacgccccctattgacgtcaatgacggtaaatggcccgcctggcattatgcccagtacatgaccttatgggactttcctacttggcagtacatctacgtattagtcatcgctattaccatggtgatgcggttttggcagtacatcaatgggcgtggatagcggtttgactcacggggatttccaagtctccaccccattgacgtcaatgggagtttgttttggcaccaaaatcaacgggactttccaaaatgtcgtaacaactccgccccattgacgcaaatgggcggtaggcgtgtacggtgggaggtctatataagcagagctctctggctaactaccggtgccaccatgagcaaggacaagaaaaccaaggccaagagaatgggcgtgaaggccctgctggcccacggcgaggacaagctgaccatgaccaccttcggcaagggcaacagaagcaagatcgagttcaccgagggctaccacggcagagccctggagacacccaagcacttcggcatcagaggcttcgaggtgagaagaatcgacgagaacgtggacctgtgcggcgacctggaggagggcaagaccatcgaggccctgctggtgaaccccagcgagaaggtgggcgaggactacctgaagctgaagggcaccctggagaagagattcttcggcagagagttcccccacgacaacatcagaatccagctgatctacaacatcctggacatctacaagatcctgggcatgaacgtggccgacatcctgtacgccctgggcaacatgcaggacaccgagctggacatcgacatgttcggccagagcctgaacaacgaggacaacctgaaggagtgcctgaagagaatgaggccctacatgggctacttcggcgacatcttcaagatcagccccaagggcgagaacatcgccgacagagagcacaacaagaaggtgctgagatgcatcagcgtgctggcaaacgccaccgccgccgacaagcaggacgagtacccctggttcaagagcagcgacatctacgagacaaagatcttcaaggccgacatgtggaagatcatcaaggaccagtacagagagaagatcaagaaggtgaacaaggacttcctgagcaagaacgccgtgaacatggccatcctgttcgacctgctgaacgccagagacgtggagcagaagaagcagatcaccgacgagttctacagattcaccatcagaaaggacggcaagaacctgggcatgaacctggtgaagatcagagagatcatcatcgacagatacgccagcggcctgagagacaagaagcacgacccccacagacagaagatcaacgtgatcgccgacttcctgatcttcagagccctgagccagaaccagggcatcatcgacaagaccgtgagcagcctgagactgaccaaggacgaggaggagaaggaccacgtgtaccagaacgccgccgagctggtgtggggcatggtgagcaactgcctgaccccctacttcaacgaccccaagaacaagtacatcctgaagtacaaggacgccaagacccccggcgacttcgaggactggatcaccagcaagatcagcgaggacgacggcgagcccttcgtgaaggtgctgagcttcctgtgcaacttcctggagggcaaggagatcaacgagctgctgaccgcctacatccacaagttcgagtgcatccaggacttcctgaacgtgatcagcagcctgggcgagaacgtgcagttccagcccagattcgccctgttcaacaacgccagcttcgcccagaacgtggccgtgcagctgagaatcctggccagcatcggcaagatgaagcccgacctgaccgaggccaagaggcccctgtacaaggccgccatcagaatgctgtgcccccccgagaagtgggagaagtacaccagcgacgagtggctggagaagaacatgctgctgaacagcgaggacagaaagaacgacaagaagaagaagcaggtgaaccccttcagaaacttcatcgccggcaacgtgatcgagagcagaagattcatgtacctggtgagatacagcaagcccaaggccgtgagagccatcatgcagaacagaagcatcgtgaactacgtgctgcacagactgcccagcgagcaggtgcacagatacgccagcgtgttccccgagaacttcgccgacctggagcaggagatcgacttcctgaccaagaagctgttcgagttcagcttcgaggagctgctgcacgagaaggacgtgatcctgaacaacagcagaagccacaagcccagcctggagatcgagagactgaaggccatcaccggcctgtacctgagcgtggcctacatcgccatcaagaacatcgtgaaggccaacgccagatactacatcgccttcgccgtgttcgagagagacaaggagctggtgaaggccaaggacgccagaatccagaccaagatccccgagacagacttccccgactacttctgcctgacccagtactacctggacagagacgaggagaagaagttccccggcgaccccagagacaaggaggccttcttcgagcacctggcaaagaccaagagagccttcagcaagcagtggagagagtggctgaacgagaagatcgccgacgccaagagcagccaggccaccggcctgctgctgagagaggccgcaaacgacgtggaggccctgaacgtgctgagagccatccccgactacatccaggacttcagacacggcgagaagggcgagacagccatgaacagctacttcgagctgtaccactacctgatgcagagactgatgctgaagaacaccgagctggacctgagccactggagcggctggatcatgagaagcggcagacccgacagagacttgatccagatcgccttcgtgagcctggcctacaacctgcccagatacagaaacctgaccaaggagcaccacttcgacgacaccgtgctgcagaagatcagagagaaggagagcctggacgccgaggccgccgccaaggaggccgccgccaaggaggccgccgccaaggccggatcccttcaactgcctccacttgaaagactgacactgggatcccagctgcatttaccgcaggttttagctgacgctgtctcacgcctggtcctgggtaagtttggtgacctgaccgacaacttctcctcccctcacgctcgcagaaaagtgctggctggagtcgtcatgacaacaggcacagatgttaaagatgccaaggtgataagtgtttctacaggaggcaaatgtattaatggtgaatacatgagtgatcgtggccttgcattaaatgactgccatgcagaaataatatctcggagatccttgctcagatttctttatacacaacttgagctttacttaaataacaaagatgatcaaaaaagatccatctttcagaaatcagagcgaggggggtttaggctgaaggagaatgtccagtttcatctgtacatcagcacctctccctgtggagatgccagaatcttctcaccacatgagccaatcctggaagaaccagcagatagacacccaaatcgtaaagcaagaggacagctacggaccaaaatagagtctggtcaggggacgattccagtgcgctccaatgcgagcatccaaacgtgggacggggtgctgcaaggggagcggctgctcaccatgtcctgcagtgacaagattgcacgctggaacgtggtgggcatccagggatcactgctcagcattttcgtggagcccatttacttctcgagcatcatcctgggcagcctttaccacggggaccacctttccagggccatgtaccagcggatctccaacatagaggacctgccacctctctacaccctcaacaagcctttgctcagtggcatcagcaatgcagaagcacggcagccagggaaggcccccaacttcagtgtcaactggacggtaggcgactccgctattgaggtcatcaacgccacgactgggaaggatgagctgggccgcgcgtcccgcctgtgtaagcacgcgttgtactgtcgctggatgcgtgtgcacggcaaggttccctcccacttactacgctccaagattaccaagcccaacgtgtaccatgagtccaagctggcggcaaaggagtaccaggccgccaaggcgcgtctgttcacagccttcatcaaggcggggctgggggcctgggtggagaagcccaccgagcaggaccagttctcactcacgtaagcggccgctcgagtctagagggcccgtttaaacccgctgatcagcctcgagaattccccttgagcatctgacttctggctaataaaggaaatttattttcattgcaatagtgtgttggaattttttgtgtctctcaggtaccgagggcctatttcccatgattccttcatatttgcatatacgatacaaggctgttagagagataattggaattaatttgactgtaaacacaaagatattagtacaaaatacgtgacgtagaaagtaataatttcttgggtagtttgcagttttaaaattatgttttaaaatggactatcatatgcttaccgtaacttgaaagtatttcgatttcttggctttatatatcttgtggaaaggacgaaacaccggaagataactctacaaacctgtagggttctgagactgccgttcttctgcttgtcggccatgatatagacgttgtggctgttgtagttgtactccagcttgtgcccttttttgcggccgcaggaacccctagtgatggagttggccactccctctctgcgcgctcgctcgctcactgaggccgggcgaccaaaggtcgcccgacgcccgggctttgcccgggcggcctcagtgagcgagcgagcgcgcagctgcctgcaggggcgcctgatgcggtattttctccttacgcatctgtgcggtatttcacaccgcatacgtcaaagcaaccatagtacgcgccctgtagcggcgcattaagcgcggcgggtgtggtggttacgcgcagcgtgaccgctacacttgccagcgccttagcgcccgctcctttcgctttcttcccttcctttctcgccacgttcgccggctttccccgtcaagctctaaatcgggggctccctttagggttccgatttagtgctttacggcacctcgaccccaaaaaacttgatttgggtgatggttcacgtagtgggccatcgccctgatagacggtttttcgccctttgacgttggagtccacgttctttaatagtggactcttgttccaaactggaacaacactcaactctatctcgggctattcttttgatttataagggattttgccgatttcggtctattggttaaaaaatgagctgatttaacaaaaatttaacgcgaattttaacaaaatattaacgtttacaattttatggtgcactctcagtacaatctgctctgatgccgcatagttaagccagccccgacacccgccaacacccgctgacgcgccctgacgggcttgtctgctcccggcatccgcttacagacaagctgtgaccgtctccgggagctgcatgtgtcagaggttttcaccgtcatcaccgaaacgcgcgagacgaaagggcctcgtgatacgcctatttttataggttaatgtcatgataataatggtttcttagacgtcaggtggcacttttcggggaaatgtgcgcggaacccctatttgtttatttttctaaatacattcaaatatgtatccgctcatgagacaataaccctgataaatgcttcaataatattgaaaaaggaagagtatgagtattcaacatttccgtgtcgcccttattcccttttttgcggcattttgccttcctgtttttgctcacccagaaacgctggtgaaagtaaaagatgctgaagatcagttgggtgcacgagtgggttacatcgaactggatctcaacagcggtaagatccttgagagttttcgccccgaagaacgttttccaatgatgagcacttttaaagttctgctatgtggcgcggtattatcccgtattgacgccgggcaagagcaactcggtcgccgcatacactattctcagaatgacttggttgagtactcaccagtcacagaaaagcatcttacggatggcatgacagtaagagaattatgcagtgctgccataaccatgagtgataacactgcggccaacttacttctgacaacgatcggaggaccgaaggagctaaccgcttttttgcacaacatgggggatcatgtaactcgccttgatcgttgggaaccggagctgaatgaagccataccaaacgacgagcgtgacaccacgatgcctgtagcaatggcaacaacgttgcgcaaactattaactggcgaactacttactctagcttcccggcaacaattaatagactggatggaggcggataaagttgcaggaccacttctgcgctcggcccttccggctggctggtttattgctgataaatctggagccggtgagcgtggaagccgcggtatcattgcagcactggggccagatggtaagccctcccgtatcgtagttatctacacgacggggagtcaggcaactatggatgaacgaaatagacagatcgctgagataggtgcctcactgattaagcattggtaactgtcagaccaagtttactcatatatactttagattgatttaaaacttcatttttaatttaaaaggatctaggtgaagatcctttttgataatctcatgaccaaaatcccttaacgtgagttttcgttccactgagcgtcagaccccgtagaaaagatcaaaggatcttcttgagatcctttttttctgcgcgtaatctgctgcttgcaaacaaaaaaaccaccgctaccagcggtggtttgtttgccggatcaagagctaccaactctttttccgaaggtaactggcttcagcagagcgcagataccaaatactgttcttctagtgtagccgtagttaggccaccacttcaagaactctgtagcaccgcctacatacctcgctctgctaatcctgttaccagtggctgctgccagtggcgataagtcgtgtcttaccgggttggactcaagacgatagttaccggataaggcgcagcggtcgggctgaacggggggttcgtgcacacagcccagcttggagcgaacgacctacaccgaactgagatacctacagcgtgagctatgagaaagcgccacgcttcccgaagggagaaaggcggacaggtatccggtaagcggcagggtcggaacaggagagcgcacgagggagcttccagggggaaacgcctggtatctttatagtcctgtcgggtttcgccacctctgacttgagcgtcgatttttgtgatgctcgtcaggggggcggagcctatggaaaaacgccagcaacgcggcctttttacggttcctggccttttgctggccttttgctcacatgt

SEQ ID NO: 100 - DNA, 7937 bp, synthetic construct
  source 1..7937: mol_type = other DNA
cctgcaggcagctgcgcgctcgctcgctcactgaggccgcccgggcgtcgggcgacctttggtcgcccggcctcagtgagcgagcgagcgcgcagagagggagtggccaactccatcactaggggttcctgcggcctctagactcgaggcgttgacattgattattgactagttattaatagtaatcaattacggggtcattagttcatagcccatatatggagttccgcgttacataacttacggtaaatggcccgcctggctgaccgcccaacgacccccgcccattgacgtcaataatgacgtatgttcccatagtaacgccaatagggactttccattgacgtcaatgggtggagtatttacggtaaactgcccacttggcagtacatcaagtgtatcatatgccaagtacgccccctattgacgtcaatgacggtaaatggcccgcctggcattatgcccagtacatgaccttatgggactttcctacttggcagtacatctacgtattagtcatcgctattaccatggtgatgcggttttggcagtacatcaatgggcgtggatagcggtttgactcacggggatttccaagtctccaccccattgacgtcaatgggagtttgttttggcaccaaaatcaacgggactttccaaaatgtcgtaacaactccgccccattgacgcaaatgggcggtaggcgtgtacggtgggaggtctatataagcagagctctctggctaactaccggtgccaccatgagcaaggacaagaaaaccaaggccaagagaatgggcgtgaaggccctgctggcccacggcgaggacaagctgaccatgaccaccttcggcaagggcaacagaagcaagatcgagttcaccgagggctaccacggcagagccctggagacacccaagcacttcggcatcagaggcttcgaggtgagaagaatcgacgagaacgtggacctgtgcggcgacctggaggagggcaagaccatcgaggccctgctggtgaaccccagcgagaaggtgggcgaggactacctgaagctgaagggcaccctggagaagagattcttcggcagagagttcccccacgacaacatcagaatccagctgatctacaacatcctggacatctacaagatcctgggcatgaacgtggccgacatcctgtacgccctgggcaacatgcaggacaccgagctggacatcgacatgttcggccagagcctgaacaacgaggacaacctgaaggagtgcctgaagagaatgaggccctacatgggctacttcggcgacatcttcaagatcagccccaagggcgagaacatcgccgacagagagcacaacaagaaggtgctgagatgcatcagcgtgctggcaaacgccaccgccgccgacaagcaggacgagtacccctggttcaagagcagcgacatctacgagacaaagatcttcaaggccgacatgtggaagatcatcaaggaccagtacagagagaagatcaagaaggtgaacaaggacttcctgagcaagaacgccgtgaacatggccatcctgttcgacctgctgaacgccagagacgtggagcagaagaagcagatcaccgacgagttctacagattcaccatcagaaaggacggcaagaacctgggcatgaacctggtgaagatcagagagatcatcatcgacagatacgccagcggcctgagagacaagaagcacgacccccacagacagaagatcaacgtgatcgccgacttcctgatcttcagagccctgagccagaaccagggcatcatcgacaagaccgtgagcagcctgagactgaccaaggacgaggaggagaaggaccacgtgtaccagaacgccgccgagctggtgtggggcatggtgagcaactgcctgaccccctacttcaacgaccccaagaacaagtacatcctgaagtacaaggacgccaagacccccggcgacttcgaggactggatcaccagcaagatcagcgaggacgacggcgagcccttcgtgaaggtgctgagcttcctgtgcaacttcctggagggcaaggagatcaacgagctgctgaccgcctacatccacaagttcgagtgcatccaggacttcctgaacgtgatcagcagcctgggcgagaacgtgcagttccagcccagattcgccctgttcaacaacgccagcttcgcccagaacgtggccgtgcagctgagaatcctggccagcatcggcaagatgaagcccgacctgaccgaggccaagaggcccctgtacaaggccgccatcagaatgctgtgcccccccgagaagtgggagaagtacaccagcgacgagtggctggagaagaacatgctgctgaacagcgaggacagaaagaacgacaagaagaagaagcaggtgaaccccttcagaaacttcatcgccggcaacgtgatcgagagcagaagattcatgtacctggtgagatacagcaagcccaaggccgtgagagccatcatgcagaacagaagcatcgtgaactacgtgctgcacagactgcccagcgagcaggtgcacagatacgccagcgtgttccccgagaacttcgccgacctggagcaggagatcgacttcctgaccaagaagctgttcgagttcagcttcgaggagctgctgcacgagaaggacgtgatcctgaacaacagcagaagccacaagcccagcctggagatcgagagactgaaggccatcaccggcctgtacctgagcgtggcctacatcgccatcaagaacatcgtgaaggccaacgccagatactacatcgccttcgccgtgttcgagagagacaaggagctggtgaaggccaaggacgccagaatccagaccaagatccccgagacagacttccccgactacttctgcctgacccagtactacctggacagagacgaggagaagaagttccccggcgaccccagagacaaggaggccttcttcgagcacctggcaaagaccaagagagccttcagcaagcagtggagagagtggctgaacgagaagatcgccgacgccaagagcagccaggccaccggcctgctgctgagagaggccgcaaacgacgtggaggccctgaacgtgctgagagccatccccgactacatccaggacttcagacacggcgagaagggcgagacagccatgaacagctacttcgagctgtaccactacctgatgcagagactgatgctgaagaacaccgagctggacctgagccactggagcggctggatcatgagaagcggcagacccgacagagacttgatccagatcgccttcgtgagcctggcctacaacctgcccagatacagaaacctgaccaaggagcaccacttcgacgacaccgtgctgcagaagatcagagagaaggagagcctggacggtggcggaggttctggtggcggaggttctggtggcggaggttctggatcccttcaactgcctccacttgaaagactgacactgggatcccagctgcatttaccgcaggttttagctgacgctgtctcacgcctggtcctgggtaagtttggtgacctgaccgacaacttctcctcccctcacgctcgcagaaaagtgctggctggagtcgtcatgacaacaggcacagatgttaaagatgccaaggtgataagtgtttctacaggaggcaaatgtattaatggtgaatacatgagtgatcgtggccttgcattaaatgactgccatgcagaaataatatctcggagatccttgctcagatttctttatacacaacttgagctttacttaaataacaaagatgatcaaaaaagatccatctttcagaaatcagagcgaggggggtttaggctgaaggagaatgtccagtttcatctgtacatcagcacctctccctgtggagatgccagaatcttctcaccacatgagccaatcctggaagaaccagcagatagacacccaaatcgtaaagcaagaggacagctacggaccaaaatagagtctggtcaggggacgattccagtgcgctccaatgcgagcatccaaacgtgggacggggtgctgcaaggggagcggctgctcaccatgtcctgcagtgacaagattgcacgctggaacgtggtgggcatccagggatcactgctcagcattttcgtggagcccatttacttctcgagcatcatcctgggcagcctttaccacggggaccacctttccagggccatgtaccagcggatctccaacatagaggacctgccacctctctacaccctcaacaagcctttgctcagtggcatcagcaatgcagaagcacggcagccagggaaggcccccaacttcagtgtcaactggacggtaggcgactccgctattgaggtcatcaacgccacgactgggaaggatgagctgggccgcgcgtcccgcctgtgtaagcacgcgttgtactgtcgctggatgcgtgtgcacggcaaggttccctcccacttactacgctccaagattaccaagcccaacgtgtaccatgagtccaagctggcggcaaaggagtaccaggccgccaaggcgcgtctgttcacagccttcatcaaggcggggctgggggcctgggtggagaagcccaccgagcaggaccagttctcactcacgtaagcggccgctcgagtctagagggcccgtttaaacccgctgatcagcctcgagaattccccttgagcatctgacttctggctaataaaggaaatttattttcattgcaatagtgtgttggaattttttgtgtctctcaggtaccgagggcctatttcccatgattccttcatatttgcatatacgatacaaggctgttagagagataattggaattaatttgactgtaaacacaaagatattagtacaaaatacgtgacgtagaaagtaataatttcttgggtagtttgcagttttaaaattatgttttaaaatggactatcatatgcttaccgtaacttgaaagtatttcgatttcttggctttatatatcttgtggaaaggacgaaacaccggaagataactctacaaacctgtagggttctgagactgccgttcttctgcttgtcggccatgatatagacgttgtggctgttgtagttgtactccagcttgtgcccttttttgcggccgcaggaacccctagtgatggagttggccactccctctctgcgcgctcgctcgctcactgaggccgggcgaccaaaggtcgcccgacgcccgggctttgcccgggcggcctcagtgagcgagcgagcgcgcagctgcctgcaggggcgcctgatgcggtattttctccttacgcatctgtgcggtatttcacaccgcatacgtcaaagcaaccatagtacgcgccctgtagcggcgcattaagcgcggcgggtgtggtggttacgcgcagcgtgaccgctacacttgccagcgccttagcgcccgctcctttcgctttcttcccttcctttctcgccacgttcgccggctttccccgtcaagctctaaatcgggggctccctttagggttccgatttagtgctttacggcacctcgaccccaaaaaacttgatttgggtgatggttcacgtagtgggccatcgccctgatagacggtttttcgccctttgacgttggagtccacgttctttaatagtggactcttgttccaaactggaacaacactcaactctatctcgggctattcttttgatttataagggattttgccgatttcggtctattggttaaaaaatgagctgatttaacaaaaatttaacgcgaattttaacaaaatattaacgtttacaattttatggtgcactctcagtacaatctgctctgatgccgcatagttaagccagccccgacacccgccaacacccgctgacgcgccctgacgggcttgtctgctcccggcatccgcttacagacaagctgtgaccgtctccgggagctgcatgtgtcagaggttttcaccgtcatcaccgaaacgcgcgagacgaaagggcctcgtgatacgcctatttttataggttaatgtcatgataataatggtttcttagacgtcaggtggcacttttcggggaaatgtgcgcggaacccctatttgtttatttttctaaatacattcaaatatgtatccgctcatgagacaataaccctgataaatgcttcaataatattgaaaaaggaagagtatgagtattcaacatttccgtgtcgcccttattcccttttttgcggcattttgccttcctgtttttgctcacccagaaacgctggtgaaagtaaaagatgctgaagatcagttgggtgcacgagtgggttacatcgaactggatctcaacagcggtaagatccttgagagttttcgccccgaagaacgttttccaatgatgagcacttttaaagttctgctatgtggcgcggtattatcccgtattgacgccgggcaagagcaactcggtcgccgcatacactattctcagaatgacttggttgagtactcaccagtcacagaaaagcatcttacggatggcatgacagtaagagaattatgcagtgctgccataaccatgagtgataacactgcggccaacttacttctgacaacgatcggaggaccgaaggagctaaccgcttttttgcacaacatgggggatcatgtaactcgccttgatcgttgggaaccggagctgaatgaagccataccaaacgacgagcgtgacaccacgatgcctgtagcaatggcaacaacgttgcgcaaactattaactggcgaactacttactctagcttcccggcaacaattaatagactggatggaggcggataaagttgcaggaccacttctgcgctcggcccttccggctggctggtttattgctgataaatctggagccggtgagcgtggaagccgcggtatcattgcagcactggggccagatggtaagccctcccgtatcgtagttatctacacgacggggagtcaggcaactatggatgaacgaaatagacagatcgctgagataggtgcctcactgattaagcattggtaactgtcagaccaagtttactcatatatactttagattgatttaaaacttcatttttaatttaaaaggatctaggtgaagatcctttttgataatctcatgaccaaaatcccttaacgtgagttttcgttccactgagcgtcagaccccgtagaaaagatcaaaggatcttcttgagatcctttttttctgcgcgtaatctgctgcttgcaaacaaaaaaaccaccgctaccagcggtggtttgtttgccggatcaagagctaccaactctttttccgaaggtaactggcttcagcagagcgcagataccaaatactgttcttctagtgtagccgtagttaggccaccacttcaagaactctgtagcaccgcctacatacctcgctctgctaatcctgttaccagtggctgctgccagtggcgataagtcgtgtcttaccgggttggactcaagacgatagttaccggataaggcgcagcggtcgggctgaacggggggttcgtgcacacagcccagcttggagcgaacgacctacaccgaactgagatacctacagcgtgagctatgagaaagcgccacgcttcccgaagggagaaaggcggacaggtatccggtaagcggcagggtcggaacaggagagcgcacgagggagcttccagggggaaacgcctggtatctttatagtcctgtcgggtttcgccacctctgacttgagcgtcgatttttgtgatgctcgtcaggggggcggagcctatggaaaaacgccagcaacgcggcctttttacggttcctggccttttgctggccttttgctcacatgt

SEQ ID NO: 101 - DNA, 4828 bp, synthetic construct; identical to SEQ ID NO: 13
  source 1..4828: mol_type = other DNA

SEQ ID NO: 102 - DNA, 7141 bp, synthetic construct
  source 1..7141: mol_type = other DNA
ttggggttgcgccttttccaaggcagccctgggtttgcgcagggacgcggctgctctgggcgtggttccgggaaacgcagcggcgccgaccctgggtctcgcacattcttcacgtccgttcgcagcgtcacccggatcttcgccgctacccttgtgggccccccggcgacgcttcctgctccgcccctaagtcgggaaggttccttgcggttcgcggcgtgccggacgtgacaaacggaagccgcacgtctcactagtaccctcgcagacggacagcgccagggagcaatggcagcgcgccgaccgcgatgggctgtggccaatagcggctgctcagcagggcgcgccgagagcagcggccgggaaggggcggtgcgggaggcggggtgtggggcggtagtgtgggccctgttcctgcccgcgcggtgttccgcattctgcaagcctccggagcgcacgtcggcagtcggctccctcgttgaccgaatcaccgacctctctccccagggggatccaccggagcttaccatgaccgagtacaagcccacggtgcgcctcgccacccgcgacgacgtccccagggccgtacgcaccctcgccgccgcgttcgccgactaccccgccacgcgccacaccgtcgatccggaccgccacatcgagcgggtcaccgagctgcaagaactcttcctcacgcgcgtcgggctcgacatcggcaaggtgtgggtcgcggacgacggcgccgcggtggcggtctggaccacgccggagagcgtcgaagcgggggcggtgttcgccgagatcggcccgcgcatggccgagttgagcggttcccggctggccgcgcagcaacagatggaaggcctcctggcgccgcaccggcccaaggagcccgcgtggttcctggccaccgtcggcgtctcgcccgaccaccagggcaagggtctgggcagcgccgtcgtgctccccggagtggaggcggccgagcgcgccggggtgcccgccttcctggagacctccgcgccccgcaacctccccttctacgagcggctcggcttcaccgtcaccgccgacgtcgaggtgcccgaaggaccgcgcacctggtgcatgacccgcaagcccggtgcctgacgcccgccccacgacccgcagcgcccgaccgaaaggagcgcacgaccccatgcatcggtacctttaagaccaatgacttacaaggcagctgtagatcttagccactttttaaaagaaaaggggggactggaagggctaattcactcccaacgaagacaagatctgctttttgcttgtactgggtctctctggttagaccagatctgagcctgggagctctctggctaactagggaacccactgcttaagcctcaataaagcttgccttgagtgcttcaagtagtgtgtgcccgtctgttgtgtgactctggtaactagagatccctcagacccttttagtcagtgtggaaaatctctagcagtagtagttcatgtcatcttattattcagtatttataacttgcaaagaaatgaatatcagagagtgagaggaacttgtttattgcagcttataatggttacaaataaagcaatagcatcacaaatttcacaaataaagcatttttttcactgcattctagttgtggtttgtccaaactcatcaatgtatcttatcatgtctggctctagctatcccgcccctaactccgcccatcccgcccctaactccgcccagttccgcccattctccgccccatggctgactaattttttttatttatgcagaggccgaggccgcctcggcctctgagctattccagaagtagtgaggaggcttttttggaggcctagggacgtacccaattcgccctatagtgagtcgtattacgcgcgctcactggccgtcgttttacaacgtcgtgactgggaaaaccctggcgttacccaacttaatcgccttgcagcacatccccctttcgccagctggcgtaatagcgaagaggcccgcaccgatcgcccttcccaacagttgcgcagcctgaatggcgaatgggacgcgccctgtagcggcgcattaagcgcggcgggtgtggtggttacgcgcagcgtgaccgctacacttgccagcgccctagcgcccgctcctttcgctttcttcccttcctttctcgccacgttcgccggctttccccgtcaagctctaaatcgggggctccctttagggttccgatttagtgctttacggcacctcgaccccaaaaaacttgattagggtgatggttcacgtagtgggccatcgccctgatagacggtttttcgccctttgacgttggagtccacgttctttaatagtggactcttgttccaaactggaacaacactcaaccctatctcggtctattcttttgatttataagggattttgccgatttcggcctattggttaaaaaatgagctgatttaacaaaaatttaacgcgaattttaacaaaatattaacgcttacaatttaggtggcacttttcggggaaatgtgcgcggaacccctatttgtttatttttctaaatacattcaaatatgtatccgctcatgagacaataaccctgataaatgcttcaataatattgaaaaaggaagagtatgagtattcaacatttccgtgtcgcccttattcccttttttgcggcattttgccttcctgtttttgctcacccagaaacgctggtgaaagtaaaagatgctgaagatcagttgggtgcacgagtgggttacatcgaactggatctcaacagcggtaagatccttgagagttttcgccccgaagaacgttttccaatgatgagcacttttaaagttctgctatgtggcgcggtattatcccgtattgacgccgggcaagagcaactcggtcgccgcatacactattctcagaatgacttggttgagtactcaccagtcacagaaaagcatcttacggatggcatgacagtaagagaattatgcagtgctgccataaccatgagtgataacactgcggccaacttacttctgacaacgatcggaggaccgaaggagctaaccgcttttttgcacaacatgggggatcatgtaactcgccttgatcgttgggaaccggagctgaatgaagccataccaaacgacgagcgtgacaccacgatgcctgtagcaatggcaacaacgttgcgcaaactattaactggcgaactacttactctagcttcccggcaacaattaatagactggatggaggcggataaagttgcaggaccacttctgcgctcggcccttccggctggctggtttattgctgataaatctggagccggtgagcgtgggtctcgcggtatcattgcagcactggggccagatggtaagccctcccgtatcgtagttatctacacgacggggagtcaggcaactatggatgaacgaaatagacagatcgctgagataggtgcctcactgattaagcattggtaactgtcagaccaagtttactcatatatactttagattgatttaaaacttcatttttaatttaaaaggatctaggtgaagatcctttttgataatctcatgaccaaaatcccttaacgtgagttttcgttccactgagcgtcagaccccgtagaaaagatcaaaggatcttcttgagatcctttttttctgcgcgtaatctgctgcttgcaaacaaaaaaaccaccgctaccagcggtggtttgtttgccggatcaagagctaccaactctttttccgaaggtaactggcttcagcagagcgcagataccaaatactgttcttctagtgtagccgtagttaggccaccacttcaagaactctgtagcaccgcctacatacctcgctctgctaatcctgttaccagtggctgctgccagtggcgataagtcgtgtcttaccgggttggactcaagacgatagttaccggataaggcgcagcggtcgggctgaacggggggttcgtgcacacagcccagcttggagcgaacgacctacaccgaactgagatacctacagcgtgagctatgagaaagcgccacgcttcccgaagggagaaaggcggacaggtatccggtaagcggcagggtcggaacaggagagcgcacgagggagcttccagggggaaacgcctggtatctttatagtcctgtcgggtttcgccacctctgacttgagcgtcgatttttgtgatgctcgtcaggggggcggagcctatggaaaaacgccagcaacgcggcctttttacggttcctggccttttgctggccttttgctcacatgttctttcctgcgttatcccctgattctgtggataaccgtattaccgcctttgagtgagctgataccgctcgccgcagccgaacgaccgagcgcagcgagtcagtgagcgaggaagcggaagagcgcccaatacgcaaaccgcctctccccgcgcgttggccgattcattaatgcagctggcacgacaggtttcccgactggaaagcgggcagtgagcgcaacgcaattaatgtgagttagctcactcattaggcaccccaggctttacactttatgcttccggctcgtatgttgtgtggaattgtgagcggataacaatttcacacaggaaacagctatgaccatgattacgccaagcgcgcaattaaccctcactaaagggaacaaaagctggagctgcaagcttaatgtagtcttatgcaatactcttgtagtcttgcaacatggtaacgatgagttagcaacatgccttacaaggagagaaaaagcaccgtgcatgccgattggtggaagtaaggtggtacgatcgtgccttattaggaaggcaacagacgggtctgacatggattggacgaaccactgaattgccgcattgcagagatattgtatttaagtgcctagctcgatacataaacgggtctctctggttagaccagatctgagcctgggagctctctggctaactagggaacccactgcttaagcctcaataaagcttgccttgagtgcttcaagtagtgtgtgcccgtctgttgtgtgactctggtaactagagatccctcagacccttttagtcagtgtggaaaatctctagcagtggcgcccgaacagggacttgaaagcgaaagggaaaccagaggagctctctcgacgcaggactcggcttgctgaagcgcgcacggcaagaggcgaggggcggcgactggtgagtacgccaaaaattttgactagcggaggctagaaggagagagatgggtgcgagagcgtcagtattaagcgggggagaattagatcgcgatgggaaaaaattcggttaaggccagggggaaagaaaaaatataaattaaaacatatagtatgggcaagcagggagctagaacgattcgcagttaatcctggcctgttagaaacatcagaaggctgtagacaaatactgggacagctacaaccatcccttcagacaggatcagaagaacttagatcattatataatacagtagcaaccctctattgtgtgcatcaaaggatagagataaaagacaccaaggaagctttagacaagatagaggaagagcaaaacaaaagtaagaccaccgcacagcaagcggccgctgatcttcagacctggaggaggagatatgagggacaattggagaagtgaattatataaatataaagtagtaaaaattgaaccattaggagtagcacccaccaaggcaaagagaagagtggtgcagagagaaaaaagagcagtgggaataggagctttgttccttgggttcttgggagcagcaggaagcactatgggcgcagcgtcaatgacgctgacggtacaggccagacaattattgtctggtatagtgcagcagcagaacaatttgctgagggctattgaggcgcaacagcatctgttgcaactcacagtctggggcatcaagcagctccaggcaagaatcctggctgtggaaagatacctaaaggatcaacagctcctggggatttggggttgctctggaaaactcatttgcaccactgctgtgccttggaatgctagttggagtaataaatctctggaacagatttggaatcacacgacctggatggagtgggacagagaaattaacaattacacaagcttaatacactccttaattgaagaatcgcaaaaccagcaagaaaagaatgaacaagaattattggaattagataaatgggcaagtttgtggaattggtttaacataacaaattggctgtggtatataaaattattcataatgatagtaggaggcttggtaggtttaagaatagtttttgctgtactttctatagtgaatagagttaggcagggatattcaccattatcgtttcagacccacctcccaaccccgaggggacccgacaggcccgaaggaatagaagaagaaggtggagagagagacagagacagatccattcgattagtgaacggatctcgacggtatcgatcacgagactagcctcgagcggccgcccccttcaccgagggcctatttcccatgattccttcatatttgcatatacgatacaaggctgttagagagataattggaattaatttgactgtaaacacaaagatattagtacaaaatacgtgacgtagaaagtaataatttcttgggtagtttgcagttttaaaattatgttttaaaatggactatcatatgcttaccgtaacttgaaagtatttcgatttcttggctttatatatcttgtggaaaggacgaaacacctgccgttcttctgcttgtcggccatgatatagacgttgtggctgttgtagttgtactccagcttgtgcccgttgtggaaggtccagttttgaggggctattacaacttttttgaattctcgacctcgagacaaatggcagtattcatccacaattttaaaagaaaaggggggattggggggtacagtgcaggggaaagaatagtagacataatagcaacagacatacaaactaaagaattacaaaaacaaattacaaaaattcaaaattttcgggtttattacagggacagcagagatccactttggccgcggctcgaggggg

SEQ ID NO: 103 - DNA, 16 bp, synthetic construct
  source 1..16: mol_type = other DNA
agggcgaggagctgtt

SEQ ID NO: 104 - DNA, 19 bp, synthetic construct
  source 1..19: mol_type = other DNA
gtacagctcgtccatgccg

SEQ ID NO: 105 - DNA, 33 bp, synthetic construct
  source 1..33: mol_type = other DNA
aaccaaggccaaggcaatgggcgtgaaggccct

SEQ ID NO: 106 - DNA, 33 bp, synthetic construct
  source 1..33: mol_type = other DNA
attgccttggccttggttttcttgtccttgctc

SEQ ID NO: 107 - DNA, 33 bp, synthetic construct
  source 1..33: mol_type = other DNA
cgccagaagcaagatcgagttcaccgagggcta

SEQ ID NO: 108 - DNA, 35 bp, synthetic construct
  source 1..35: mol_type = other DNA
tcgatcttgcttctggcgcccttgccgaaggtggt

SEQ ID NO: 109 - DNA, 33 bp, synthetic construct
  source 1..33: mol_type = other DNA
caacgcaagcaagatcgagttcaccgagggcta

SEQ ID NO: 110 - DNA, 33 bp, synthetic construct
  source 1..33: mol_type = other DNA
tcgatcttgcttgcgttgcccttgccgaaggtg

SEQ ID NO: 111 - DNA, 33 bp, synthetic construct
  source 1..33: mol_type = other DNA
taccacggcgcagccctggagacacccaagcac

SEQ ID NO: 112 - DNA, 33 bp, synthetic construct
  source 1..33: mol_type = other DNA
cagggctgcgccgtggtagccctcggtgaactc

SEQ ID NO: 113 - DNA, 40 bp, synthetic construct
  source 1..40: mol_type = other DNA
aagcacttcggcatcgcaggcttcgaggtgagaagaatcg

SEQ ID NO: 114 - DNA, 33 bp, synthetic construct
  source 1..33: mol_type = other DNA
tgcgatgccgaagtgcttgggtgtctccagggc

SEQ ID NO: 115 - DNA, 34 bp, synthetic construct
  source 1..34: mol_type = other DNA
ttcgaggtgagcagaatcgacgagaacgtggacc

SEQ ID NO: 116 - DNA, 33 bp, synthetic construct
  source 1..33: mol_type = other DNA
gattctgctcacctcgaagcctctgatgccgaa

SEQ ID NO: 117 - DNA, 33 bp, synthetic construct
  source 1..33: mol_type = other DNA
aggtgagaagcaatcgacgagaacgtggacctg

SEQ ID NO: 118 - DNA, 33 bp, synthetic construct
  source 1..33: mol_type = other DNA
gtcgattgcttctcacctcgaagcctctgatgc

SEQ ID NO: 119 - DNA, 33 bp, synthetic construct
  source 1..33: mol_type = other DNA
aagaatcgacgaggccgtggacctgtgcggcga

SEQ ID NO: 120 - DNA, 33 bp, synthetic construct
  source 1..33: mol_type = other DNA
acggcctcgtcgattcttctcacctcgaagcct

SEQ ID NO: 121 - DNA, 33 bp, synthetic construct
  source 1..33: mol_type = other DNA
tggtggcccccagcgagaaggtgggcgaggact

SEQ ID NO: 122 - DNA, 33 bp, synthetic construct
  source 1..33: mol_type = other DNA
tctcgctgggggccaccagcagggcctcgatgg

SEQ ID NO: 123 - DNA, 34 bp, synthetic construct
  source 1..34: mol_type = other DNA
aagaacgccgtggccatggccatcctgttcgacc

SEQ ID NO: 124 - DNA, 33 bp, synthetic construct
  source 1..33: mol_type = other DNA
catggccacggcgttcttgctcaggaagtcctt

SEQ ID NO: 125 - DNA, 34 bp, synthetic construct
  source 1..34: mol_type = other DNA
tgttcgacctgctggccgccagagacgtggagca

SEQ ID NO: 126 - DNA, 33 bp, synthetic construct
  source 1..33: mol_type = other DNA
cggccagcaggtcgaacaggatggccatgttca

SEQ ID NO: 127 - DNA, 33 bp, synthetic construct
  source 1..33: mol_type = other DNA
cgcagacgtggagcagaagaagcagatcaccga

SEQ ID NO: 128 - DNA, 36 bp, synthetic construct
  source 1..36: mol_type = other DNA
ttctgctccacgtctgcggcgttcagcaggtcgaac

SEQ ID NO: 129 - DNA, 33 bp, synthetic construct
  source 1..33: mol_type = other DNA
gagttctacgcattcaccatcagaaaggacggc

SEQ ID NO: 130 - DNA, 33 bp, synthetic construct
  source 1..33: mol_type = other DNA
ggtgaatgcgtagaactcgtcggtgatctgctt

SEQ ID NO: 131 - DNA, 33 bp, synthetic construct
  source 1..33: mol_type = other DNA
ttcaccatcgcaaaggacggcaagaacctgggc

SEQ ID NO: 132 - DNA, 34 bp, synthetic construct
  source 1..34: mol_type = other DNA
gtcctttgcgatggtgaatctgtagaactcgtcg

SEQ ID NO: 133 - DNA, 33 bp, synthetic construct
  source 1..33: mol_type = other DNA
caaggccctgggcatgaacctggtgaagatcag

SEQ ID NO: 134 - DNA, 34 bp, synthetic construct
  source 1..34: mol_type = other DNA
ttcatgcccagggccttgccgtcctttctgatgg

SEQ ID NO: 135 - DNA, 33 bp, synthetic construct
  source 1..33: mol_type = other DNA
catggccctggtgaagatcagagagatcatcat

SEQ ID NO: 136 - DNA, 33 bp, synthetic construct
  source 1..33: mol_type = other DNA
atcttcaccagggccatgcccaggttcttgccg

SEQ ID NO: 137 - DNA, 35 bp, synthetic construct
  source 1..35: mol_type = other DNA
gtgaagatcgcagagatcatcatcgacagatacgc

SEQ ID NO: 138 - DNA, 33 bp, synthetic construct
  source 1..33: mol_type = other DNA
gatctctgcgatcttcaccaggttcatgcccag

SEQ ID NO: 139 - DNA, 33 bp, synthetic construct
  source 1..33: mol_type = other DNA
tcatcatcgacgcatacgccagcggcctgagag

SEQ ID NO: 140 - DNA, 33 bp, synthetic construct
  source 1..33: mol_type = other DNA
cgtatgcgtcgatgatgatctctctgatcttca

SEQ ID NO: 141 - DNA, 33 bp, synthetic construct
  source 1..33: mol_type = other DNA
cctggcagacaagaagcacgacccccacagaca

SEQ ID NO: 142 - DNA, 33 bp, synthetic construct
  source 1..33: mol_type = other DNA
tgcttcttgtctgccaggccgctggcgtatctg

SEQ ID NO: 143 - DNA, 33 bp, synthetic construct
  source 1..33: mol_type = other DNA
ccacgcacagaagatcaacgtgatcgccgactt

SEQ ID NO: 144 - DNA, 33 bp, synthetic construct
  source 1..33: mol_type = other DNA
ttgatcttctgtgcgtgggggtcgtgcttcttg

SEQ ID NO: 145 - DNA, 33 bp, synthetic construct
  source 1..33: mol_type = other DNA
acagaagatcgccgtgatcgccgacttcctgat

SEQ ID NO: 146 - DNA, 33 bp, synthetic construct
  source 1..33: mol_type = other DNA
atcacggcgatcttctgtctgtgggggtcgtgc

SEQ ID NO: 147 - DNA, 36 bp, synthetic construct
  source 1..36: mol_type = other DNA
acttcctgatcttcgcagccctgagccagaaccagg

SEQ ID NO: 148 - DNA, 32 bp, synthetic construct
  source 1..32: mol_type = other DNA
ctgcgaagatcaggaagtcggcgatcacgttg

SEQ ID NO: 149 - DNA, 33 bp, synthetic construct
  source 1..33: mol_type = other DNA
ccaggcccagggcatcatcgacaagaccgtgag

SEQ ID NO: 150 - DNA, 34 bp, synthetic construct
  source 1..34: mol_type = other DNA
atgatgccctgggcctggctcagggctctgaaga

SEQ ID NO: 151 - DNA, 33 bp, synthetic construct
  source 1..33: mol_type = other DNA
cagcctggcactgaccaaggacgaggaggagaa

SEQ ID NO: 152 - DNA, 33 bp, synthetic construct
  source 1..33: mol_type = other DNA
ttggtcagtgccaggctgctcacggtcttgtcg

SEQ ID NO: 153 - DNA, 34 bp, synthetic construct
  source 1..34: mol_type = other DNA
accacgtgtaccaggccgccgccgagctggtgtg

SEQ ID NO: 154 - DNA, 33 bp, synthetic construct
  source 1..33: mol_type = other DNA
cggcctggtacacgtggtccttctcctcctcgt

SEQ ID NO: 155 - DNA, 33 bp, synthetic construct
  source 1..33: mol_type = other DNA
tggtgagcgcctgcctgaccccctacttcaacg

SEQ ID NO: 156 - DNA, 33 bp, synthetic construct
  source 1..33: mol_type = other DNA
tcaggcaggcgctcaccatgccccacaccagct

SEQ ID NO: 157 - DNA, 33 bp, synthetic construct
  source 1..33: mol_type = other DNA
ctacttcgccgaccccaagaacaagtacatcct

SEQ ID NO: 158 - DNA, 33 bp, synthetic construct
  source 1..33: mol_type = other DNA
ttggggtcggcgaagtagggggtcaggcagttg

SEQ ID NO: 159 - DNA, 33 bp, synthetic construct
  source 1..33: mol_type = other DNA
caaggccaagtacatcctgaagtacaaggacgc

SEQ ID NO: 160 - DNA, 35 bp, synthetic construct
  source 1..35: mol_type = other DNA
aggatgtacttggccttggggtcgttgaagtaggg

SEQ ID NO: 161 - DNA, 6798 bp, synthetic construct
  source 1..6798: mol_type = other DNA
cctgcaggcagctgcgcgctcgctcgctcactgaggccgcccgggcgtcgggcgacctttggtcgcccggcctcagtgagcgagcgagcgcgcagagagggagtggccaactccatcactaggggttcctgcggcctctagactcgaggcgttgacattgattattgactagttattaatagtaatcaattacggggtcattagttcatagcccatatatggagttccgcgttacataacttacggtaaatggcccgcctggctgaccgcccaacgacccccgcccattgacgtcaataatgacgtatgttcccatagtaacgccaatagggactttccattgacgtcaatgggtggagtatttacggtaaactgcccacttggcagtacatcaagtgtatcatatgccaagtacgccccctattgacgtcaatgacggtaaatggcccgcctggcattatgcccagtacatgaccttatgggactttcctacttggcagtacatctacgtattagtcatcgctattaccatggtgatgcggttttggcagtacatcaatgggcgtggatagcggtttgactcacggggatttccaagtctccaccccattgacgtcaatgggagtttgttttggcaccaaaatcaacgggactttccaaaatgtcgtaacaactccgccccattgacgcaaatgggcggtaggcgtgtacggtgggaggtctatataagcagagctctctggctaactaccggtgccaccatgccggcagctaagaaaaagaaactggatggcagcgtcgacatgagcaaggacaagaaaaccaaggccaagagaatgggcgtgaaggccctgctggcccacggcgaggacaagctgaccatgaccaccttcggcaagggcaacagaagcaagatcgagttcaccgagggctaccacggcagagccctggagacacccaagcacttcggcatcagaggcttcgaggtgagaagaatcgacgagaacgtggacctgtgcggcgacctggaggagggcaagaccatcgaggccctgctggtgaaccccagcgagaaggtgggcgaggactacctgaagctgaagggcaccctggagaagagattcttcggcagagagttcccccacgacaacatcagaatccagctgatctacaacatcctggacatctacaagatcctgggcatgaacgtggccgacatcctgtacgccctgggcaacatgcaggacaccgagctggacatcgacatgttcggccagagcctgaacaacgaggacaacctgaaggagtgcctgaagagaatgaggccctacatgggctacttcggcgacatcttcaagatcagccccaagggcgagaacatcgccgacagagagcacaacaagaaggtgctgagatgcatcagcgtgctgagaaacgccaccgcccacgacaagcaggacgagtacccctggttcaagagcagcgacatctacgagacaaagatcttcaaggccgacatgtggaagatcatcaaggaccagtacagagagaagatcaagaaggtgaacaaggacttcctgagcaagaacgccgtgaacatggccatcctgttcgacctgctgaacgccagagacgtggagcagaagaagcagatcaccgacgagttctacagattcaccatcagaaaggacggcaagaacctgggcatgaacctggtgaagatcagagagatcatcatcgacagatacgccagcggcctgagagacaagaagcacgacccccacagacagaagatcaacgtgatcgccgacttcctgatcttcagagccctgagccagaaccagggcatcatcgacaagaccgtgagcagcctgagactgaccaaggacgaggaggagaaggaccacgtgtaccagaacgccgccgagctggtgtggggcatggtgagcaactgcctgaccccctacttcaacgaccccaagaacaagtacatcctgaagtacaaggacgccaagacccccggcgacttcgaggactggatcaccagcaagatcagcgaggacgacggcgagcccttcgtgaaggtgctgagcttcctgtgcaacttcctggagggcaaggagatcaacgagctgctgaccgcctacatccacaagttcgagtgcatccaggacttcctgaacgtgatcagcagcctgggcgagaacgtgcagttccagcccagattcgccctgttcaacaacgccagcttcgcccagaacgtggccgtgcagctgagaatcctggccagcatcggcaagatgaagcccgacctgaccgaggccaagaggcccctgtacaaggccgccatcagaatgctgtgcccccccgagaagtgggagaagtacaccagcgacgagtggctggagaagaacatgctgctgaacagcgaggacagaaagaacgacaagaagaagaagcaggtgaaccccttcagaaacttcatcgccggcaacgtgatcgagagcagaagattcatgtacctggtgagatacagcaagcccaaggccgtgagagccatcatgcagaacagaagcatcgtgaactacgtgctgcacagactgcccagcgagcaggtgcacagatacgccagcgtgttccccgagaacttcgccgacctggagcaggagatcgacttcctgaccaagaagctgttcgagttcagcttcgaggagctgctgcacgagaaggacgtgatcctgaacaacagcagaagccacaagcccagcctggagatcgagagactgaaggccatcaccggcctgtacctgagcgtggcctacatcgccatcaagaacatcgtgaaggccaacgccagatactacatcgccttcgccgtgttcgagagagacaaggagctggtgaaggccaaggacgccagaatccagaccaagatccccgagacagacttccccgactacttctgcctgacccagtactacctggacagagacgaggagaagaagttccccggcgaccccagagacaaggaggccttcttcgagcacctgagaaagaccaagagacacttcagcaagcagtggagagagtggctgaacgagaagatcgccgacgccaagagcagccaggccaccggcctgctgctgagagaggccagaaacgacgtggagcacctgaacgtgctgagagccatccccgactacatccaggacttcagacacggcgagaagggcgagacagccatgaacagctacttcgagctgtaccactacctgatgcagagactgatgctgaagaacaccgagctggacctgagccactggagcggctggatcatgagaagcggcagacccgacagagacttgatccagatcgccttcgtgagcctggcctacaacctgcccagatacagaaacctgaccaaggagcaccacttcgacgacaccgtgctgcagaagatcagagagaaggagagcctggacacaggcggcggccccggcggcggcgccgccgccggcagcggcagccctaagaaaaaacgaaaagttggcagcggaagcaaaaggccggcggccacgaaaaaggccggccaggcaaaaaagaaaaagctcgagtacccatacgatgttccagattacgcttgagaattccccttgagcatctgacttctggctaataaaggaaatttattttcattgcaatagtgtgttggaattttttgtgtctctcaggtaccgagggcctatttcccatgattccttcatatttgcatatacgatacaaggctgttagagagataattggaattaatttgactgtaaacacaaagatattagtacaaaatacgtgacgtagaaagtaataatttcttgggtagtttgcagttttaaaattatgttttaaaatggactatcatatgcttaccgtaacttgaaagtatttcgatttcttggctttatatatcttgtggaaaggacgaaacaccggaagataactctacaaacctgtagggttctgagacataacatttccgaagacgacaagatttttttgcggccgcaggaacccctagtgatggagttggccactccctctctgcgcgctcgctcgctcactgaggccgggcgaccaaaggtcgcccgacgcccgggctttgcccgggcggcctcagtgagcgagcgagcgcgcagctgcctgcaggggcgcctgatgcggtattttctccttacgcatctgtgcggtatttcacaccgcatacgtcaaagcaaccatagtacgcgccctgtagcggcgcattaagcgcggcgggtgtggtggttacgcgcagcgtgaccgctacacttgccagcgccttagcgcccgctcctttcgctttcttcccttcctttctcgccacgttcgccggctttccccgtcaagctctaaatcgggggctccctttagggttccgatttagtgctttacggcacctcgaccccaaaaaacttgatttgggtgatggttcacgtagtgggccatcgccctgatagacggtttttcgccctttgacgttggagtccacgttctttaatagtggactcttgttccaaactggaacaacactcaactctatctcgggctattcttttgatttataagggattttgccgatttcggtctattggttaaaaaatgagctgatttaacaaaaatttaacgcgaattttaacaaaatattaacgtttacaattttatggtgcactctcagtacaatctgctctgatgccgcatagttaagccagccccgacacccgccaacacccgctgacgcgccctgacgggcttgtctgctcccggcatccgcttacagacaagctgtgaccgtctccgggagctgcatgtgtcagaggttttcaccgtcatcaccgaaacgcgcgagacgaaagggcctcgtgatacgcctatttttataggttaatgtcatgataataatggtttcttagacgtcaggtggcacttttcggggaaatgtgcgcggaacccctatttgtttatttttctaaatacattcaaatatgtatccgctcatgagacaataaccctgataaatgcttcaataatattgaaaaaggaagagtatgagtattcaacatttccgtgtcgcccttattcccttttttgcggcattttgccttcctgtttttgctcacccagaaacgctggtgaaagtaaaagatgctgaagatcagttgggtgcacgagtgggttacatcgaactggatctcaacagcggtaagatccttgagagttttcgccccgaagaacgttttccaatgatgagcacttttaaagttctgctatgtggcgcggtattatcccgtattgacgccgggcaagagcaactcggtcgccgcatacactattctcagaatgacttggttgagtactcaccagtcacagaaaagcatcttacggatggcatgacagtaagagaattatgcagtgctgccataaccatgagtgataacactgcggccaacttacttctgacaacgatcggaggaccgaaggagctaaccgcttttttgcacaacatgggggatcatgtaactcgccttgatcgttgggaaccggagctgaatgaagccataccaaacgacgagcgtgacaccacgatgcctgtagcaatggcaacaacgttgcgcaaactattaactggcgaactacttactctagcttcccggcaacaattaatagactggatggaggcggataaagttgcaggaccacttctgcgctcggcccttccggctggctggtttattgctgataaatctggagccggtgagcgtggaagccgcggtatcattgcagcactggggccagatggtaagccctcccgtatcgtagttatctacacgacggggagtcaggcaactatggatgaacgaaatagacagatcgctgagataggtgcctcactgattaagcattggtaactgtcagaccaagtttactcatatatactttagattgatttaaaacttcatttttaatttaaaaggatctaggtgaagatcctttttgataatctcatgaccaaaatcccttaacgtgagttttcgttccactgagcgtcagaccccgtagaaaagatcaaaggatcttcttgagatcctttttttctgcgcgtaatctgctgcttgcaaacaaaaaaaccaccgctaccagcggtggtttgtttgccggatcaagagctaccaactctttttccgaaggtaactggcttcagcagagcgcagataccaaatactgttcttctagtgtagccgtagttaggccaccacttcaagaactctgtagcaccgcctacatacctcgctctgctaatcctgttaccagtggctgctgccagtggcgataagtcgtgtcttaccgggttggactcaagacgatagttaccggataaggcgcagcggtcgggctgaacggggggttcgtgcacacagcccagcttggagcgaacgacctacaccgaactgagatacctacagcgtgagctatgagaaagcgccacgcttcccgaagggagaaaggcggacaggtatccggtaagcggcagggtcggaacaggagagcgcacgagggagcttccagggggaaacgcctggtatctttatagtcctgtcgggtttcgccacctctgacttgagcgtcgatttttgtgatgctcgtcaggggggcggagcctatggaaaaacgccagcaacgcggcctttttacggttcctggccttttgctggccttttgctcacatgt

SEQ ID NO: 162 - DNA, 25 bp, synthetic construct
  source 1..25: mol_type = other DNA
ataacatttccgaagacgacaagat

SEQ ID NO: 163 - DNA, 31 bp, synthetic construct
  source 1..31: mol_type = other DNA
taccacggcgcagccctggagacacccaagc

SEQ ID NO: 164 - DNA, 32 bp, synthetic construct
  source 1..32: mol_type = other DNA
ggtgaatgcgtagaactcgtcggtgatctgct

SEQ ID NO: 165 - DNA, 33 bp, synthetic construct; identical to SEQ ID NO: 129
  source 1..33: mol_type = other DNA

SEQ ID NO: 166 - DNA, 27 bp, synthetic construct
  source 1..27: mol_type = other DNA
cagggctgcgccgtggtagccctcggt

SEQ ID NO: 167 - DNA, 31 bp, synthetic construct; identical to SEQ ID NO: 163
  source 1..31: mol_type = other DNA

SEQ ID NO: 168 - DNA, 33 bp, synthetic construct; identical to SEQ ID NO: 140
  source 1..33: mol_type = other DNA

SEQ ID NO: 169 - DNA, 31 bp, synthetic construct
  source 1..31: mol_type = other DNA
tcatcatcgacgcatacgccagcggcctgag

SEQ ID NO: 170 - DNA, 27 bp, synthetic construct
  source 1..27: mol_type = other DNA
cagggctgcgccgtggtagccctcggt

SEQ ID NO: 171 - DNA, 33 bp, synthetic construct; identical to SEQ ID NO: 129
  source 1..33: mol_type = other DNA

SEQ ID NO: 172 - DNA, 33 bp, synthetic construct; identical to SEQ ID NO: 140
  source 1..33: mol_type = other DNA

SEQ ID NO: 173 - DNA, 31 bp, synthetic construct; identical to SEQ ID NO: 169
  source 1..31: mol_type = other DNA

SEQ ID NO: 174 - DNA, 32 bp, synthetic construct; identical to SEQ ID NO: 164
  source 1..32: mol_type = other DNA

SEQ ID NO: 175 - DNA, 31 bp, synthetic construct; identical to SEQ ID NO: 163
  source 1..31: mol_type = other DNA

SEQ ID NO: 176 - DNA, 32 bp, synthetic construct; identical to SEQ ID NO: 164
  source 1..32: mol_type = other DNA

SEQ ID NO: 177 - DNA, 33 bp, synthetic construct; identical to SEQ ID NO: 129
  source 1..33: mol_type = other DNA

SEQ ID NO: 178 - DNA, 33 bp, synthetic construct; identical to SEQ ID NO: 140
  source 1..33: mol_type = other DNA

SEQ ID NO: 179 - DNA, 31 bp, synthetic construct; identical to SEQ ID NO: 169
  source 1..31: mol_type = other DNA

SEQ ID NO: 180 - DNA, 27 bp, synthetic construct
  source 1..27: mol_type = other DNA
cagggctgcgccgtggtagccctcggt

SEQ ID NO: 181 - DNA, 33 bp, synthetic construct; identical to SEQ ID NO: 119
  source 1..33: mol_type = other DNA

SEQ ID NO: 182 - DNA, 31 bp, synthetic construct
  source 1..31: mol_type = other DNA
gatctctgcgatcttcaccaggttcatgccc

SEQ ID NO: 183 - DNA, 35 bp, synthetic construct; identical to SEQ ID NO: 137
  source 1..35: mol_type = other DNA

SEQ ID NO: 184 - DNA, 27 bp, synthetic construct
  source 1..27: mol_type = other DNA
acggcctcgtcgattcttctcacctcg

SEQ ID NO: 185 - DNA, 33 bp, synthetic construct; identical to SEQ ID NO: 119
  source 1..33: mol_type = other DNA

SEQ ID NO: 186 - DNA, 35 bp, synthetic construct; identical to SEQ ID NO: 160
  source 1..35: mol_type = other DNA

SEQ ID NO: 187 - DNA, 32 bp, synthetic construct
  source 1..32: mol_type = other DNA
caaggccaagtacatcctgaagtacaaggacg

SEQ ID NO: 188 - DNA, 27 bp, synthetic construct
  source 1..27: mol_type = other DNA
acggcctcgtcgattcttctcacctcg

SEQ ID NO: 189 - DNA, 33 bp, synthetic construct; identical to SEQ ID NO: 119
  source 1..33: mol_type = other DNA

SEQ ID NO: 190 - DNA, 31 bp, synthetic construct
  source 1..31: mol_type = other DNA
tctcgctgggggccaccagcagggcctcgat

SEQ ID NO: 191 - DNA, 25 bp, synthetic construct
  source 1..25: mol_type = other DNA
tggtggcccccagcgagaaggtggg

SEQ ID NO: 192 - DNA, 27 bp, synthetic construct
  source 1..27: mol_type = other DNA
acggcctcgtcgattcttctcacctcg

SEQ ID NO: 193 - DNA, 34 bp, synthetic construct; identical to SEQ ID NO: 123
  source 1..34: mol_type = other DNA

SEQ ID NO: 194 - DNA, 31 bp, synthetic construct; identical to SEQ ID NO: 182
  source 1..31: mol_type = other DNA

SEQ ID NO: 195 - DNA, 35 bp, synthetic construct; identical to SEQ ID NO: 137
  source 1..35: mol_type = other DNA

SEQ ID NO: 196 - DNA, 25 bp, synthetic construct
  source 1..25: mol_type = other DNA
catggccacggcgttcttgctcagg

SEQ ID NO: 197 - DNA, 34 bp, synthetic construct; identical to SEQ ID NO: 123
  source 1..34: mol_type = other DNA

SEQ ID NO: 198 - DNA, 35 bp, synthetic construct; identical to SEQ ID NO: 160
  source 1..35: mol_type = other DNA

SEQ ID NO: 199 - DNA, 32 bp, synthetic construct; identical to SEQ ID NO: 187
  source 1..32: mol_type = other DNA

SEQ ID NO: 200 - DNA, 25 bp, synthetic construct
  source 1..25: mol_type = other DNA
catggccacggcgttcttgctcagg

SEQ ID NO: 201 - DNA, 25 bp, synthetic construct
  source 1..25: mol_type = other DNA
tggtggcccccagcgagaaggtggg

SEQ ID NO: 202 - DNA, 25 bp, synthetic construct
  source 1..25: mol_type = other DNA
catggccacggcgttcttgctcagg

SEQ ID NO: 203 - DNA, 34 bp, synthetic construct; identical to SEQ ID NO: 123
  source 1..34: mol_type = other DNA

SEQ ID NO: 204 - DNA, 31 bp, synthetic construct; identical to SEQ ID NO: 190
  source 1..31: mol_type = other DNA

SEQ ID NO: 205 - DNA, 33 bp, synthetic construct; identical to SEQ ID NO: 119
  source 1..33: mol_type = other DNA

SEQ ID NO: 206 - DNA, 25 bp, synthetic construct
  source 1..25: mol_type = other DNA
catggccacggcgttcttgctcagg

SEQ ID NO: 207 - DNA, 34 bp, synthetic construct; identical to SEQ ID NO: 123
  source 1..34: mol_type = other DNA

SEQ ID NO: 208 - DNA, 31 bp, synthetic construct; identical to SEQ ID NO: 182
  source 1..31: mol_type = other DNA

SEQ ID NO: 209 - DNA, 35 bp, synthetic construct; identical to SEQ ID NO: 137
  source 1..35: mol_type = other DNA

SEQ ID NO: 210 - DNA, 27 bp, synthetic construct
  source 1..27: mol_type = other DNA
acggcctcgtcgattcttctcacctcg

SEQ ID NO: 211 - DNA, 33 bp, synthetic construct; identical to SEQ ID NO: 119
  source 1..33: mol_type = other DNA

SEQ ID NO: 212 - DNA, 31 bp, synthetic construct; identical to SEQ ID NO: 190
  source 1..31: mol_type = other DNA

SEQ ID NO: 213 - DNA, 25 bp, synthetic construct
  source 1..25: mol_type = other DNA
tggtggcccccagcgagaaggtggg

SEQ ID NO: 214 - DNA, 25 bp, synthetic construct
  source 1..25: mol_type = other DNA
catggccacggcgttcttgctcagg

SEQ ID NO: 215 - DNA, 34 bp, synthetic construct; identical to SEQ ID NO: 123
  source 1..34: mol_type = other DNA

SEQ ID NO: 216 - DNA, 27 bp, synthetic construct
  source 1..27: mol_type = other DNA
acggcctcgtcgattcttctcacctcg

SEQ ID NO: 217 - DNA, 32 bp, synthetic construct
  source 1..32: mol_type = other DNA
acaagaaatccaaggccaagagaatgggcgtg

SEQ ID NO: 218 - DNA, 32 bp, synthetic construct
  source 1..32: mol_type = other DNA
ggccttggatttcttgtccttgctcatgtcga

SEQ ID NO: 219 - DNA, 34 bp, synthetic construct
  source 1..34: mol_type = other DNA
agaatgggcgtgaagtccctgctggcccacggcg

SEQ ID NO: 220 - DNA, 32 bp, synthetic construct
  source 1..32: mol_type = other DNA
gacttcacgcccattctcttggccttggtttt

SEQ ID NO: 221 - DNA, 32 bp, synthetic construct
  source 1..32: mol_type = other DNA
cttcctggaaaagaacgccgtgaacatggcca

SEQ ID NO: 222 - DNA, 34 bp, synthetic construct
  source 1..34: mol_type = other DNA
cgttcttttccaggaagtccttgttcaccttctt

SEQ ID NO: 223 - DNA, 33 bp, synthetic construct
  source 1..33: mol_type = other DNA
gcaagaacaaggtgaacatggccatcctgttcg

SEQ ID NO: 224 - DNA, 33 bp, synthetic construct
  source 1..33: mol_type = other DNA
gttcaccttgttcttgctcaggaagtccttgtt

SEQ ID NO: 225 - DNA, 32 bp, synthetic construct
  source 1..32: mol_type = other DNA
gtgaacatagccatcctgttcgacctgctgaa

SEQ ID NO: 226 - DNA, 32 bp, synthetic construct
  source 1..32: mol_type = other DNA
aggatggctatgttcacggcgttcttgctcag

SEQ ID NO: 227 - DNA, 37 bp, synthetic construct
  source 1..37: mol_type = other DNA
tgttcgacctgctgaaggccagagacgtggagcagaa

SEQ ID NO: 228 - DNA, 32 bp, synthetic construct
  source 1..32: mol_type = other DNA
cttcagcaggtcgaacaggatggccatgttca

SEQ ID NO: 229 - DNA, 35 bp, synthetic construct
  source 1..35: mol_type = other DNA
cgacgagtactacagattcaccatcagaaaggacg

SEQ ID NO: 230 - DNA, 32 bp, synthetic construct
  source 1..32: mol_type = other DNA
atctgtagtactcgtcggtgatctgcttcttc

SEQ ID NO: 231 - DNA, 37 bp, synthetic construct
  source 1..37: mol_type = other DNA
aacctgggcttcaacctggtgaagatcagagagatca

SEQ ID NO: 232 - DNA, 32 bp, synthetic construct
  source 1..32: mol_type = other DNA
aggttgaagcccaggttcttgccgtcctttct

SEQ ID NO: 233 - DNA, 32 bp, synthetic construct
  source 1..32: mol_type = other DNA
catgagcctggtgaagatcagagagatcatca

SEQ ID NO: 234 - DNA, 32 bp, synthetic construct
  source 1..32: mol_type = other DNA
tcttcaccaggctcatgcccaggttcttgccg

SEQ ID NO: 235 - DNA, 37 bp, synthetic construct
  source 1..37: mol_type = other DNA
gcatgaacatcgtgaagatcagagagatcatcatcga

SEQ ID NO: 236 - DNA, 32 bp, synthetic construct
  source 1..32: mol_type = other DNA
cttcacgatgttcatgcccaggttcttgccgt

SEQ ID NO: 237 - DNA, 40 bp, synthetic construct
  source 1..40: mol_type = other DNA
ggcatgaacctgaagaagatcagagagatcatcatcgaca

SEQ ID NO: 238 - DNA, 33 bp, synthetic construct
  source 1..33: mol_type = other DNA
cttcttcaggttcatgcccaggttcttgccgtc

SEQ ID NO: 239 - DNA, 32 bp, synthetic construct
  source 1..32: mol_type = other DNA
gagatcatgatcgacagatacgccagcggcct

SEQ ID NO: 240 - DNA, 34 bp, synthetic construct
  source 1..34: mol_type = other DNA
ctgtcgatcatgatctctctgatcttcaccaggt

SEQ ID NO: 241 - DNA, 32 bp, synthetic construct
  source 1..32: mol_type = other DNA
atcatcgagagatacgccagcggcctgagaga

SEQ ID NO: 242 - DNA, 34 bp, synthetic construct
  source 1..34: mol_type = other DNA
gcgtatctctcgatgatgatctctctgatcttca

SEQ ID NO: 243 - DNA, 32 bp, synthetic construct
  source 1..32: mol_type = other DNA
acaagaagtacgacccccacagacagaagatc

SEQ ID NO: 244 - DNA, 32 bp, synthetic construct
  source 1..32: mol_type = other DNA
ggggtcgtacttcttgtctctcaggccgctgg

SEQ ID NO: 245 - DNA, 36 bp, synthetic construct
  source 1..36: mol_type = other DNA
aagaagcacgactcccacagacagaagatcaacgtg

SEQ ID NO: 246 - DNA, 32 bp, synthetic construct
  source 1..32: mol_type = other DNA
tgggagtcgtgcttcttgtctctcaggccgct

SEQ ID NO: 247 - DNA, 33 bp, synthetic construct
  source 1..33: mol_type = other DNA
ccgtcagacagaagatcaacgtgatcgccgact

SEQ ID NO: 248 - DNA, 37 bp, synthetic construct
  source 1..37: mol_type = other DNA
tgatcttctgtctgacggggtcgtgcttcttgtctct

SEQ ID NO: 249 - DNA, 32 bp, synthetic construct
  source 1..32: mol_type = other DNA
gaagatctacgtgatcgccgacttcctgatct

SEQ ID NO: 250 - DNA, 32 bp, synthetic construct
  source 1..32: mol_type = other DNA
cgatcacgtagatcttctgtctgtgggggtcg

SEQ ID NO: 251 - DNA, 32 bp, synthetic construct
  source 1..32: mol_type = other DNA
caggaccagggcatcatcgacaagaccgtgag

SEQ ID NO: 252 - DNA, 34 bp, synthetic construct
  source 1..34: mol_type = other DNA
atgatgccctggtcctggctcagggctctgaaga

SEQ ID NO: 253 - DNA, 34 bp, synthetic construct
  source 1..34: mol_type = other DNA
tcatcgacaagctcgtgagcagcctgagactgac

SEQ ID NO: 254 - DNA, 33 bp, synthetic construct
  source 1..33: mol_type = other DNA
tcacgagcttgtcgatgatgccctggttctggc

SEQ ID NO: 255 - DNA, 32 bp, synthetic construct
  source 1..32: mol_type = other DNA
tgagactgtccaaggacgaggaggagaaggac

SEQ ID NO: 256 - DNA, 32 bp, synthetic construct
  source 1..32: mol_type = other DNA
gtccttggacagtctcaggctgctcacggtct

SEQ ID NO: 257 - DNA, 37 bp, synthetic construct
  source 1..37: mol_type = other DNA
aaggacgaggaggacaaggaccacgtgtaccagaacg

SEQ ID NO: 258 - DNA, 32 bp, synthetic construct
  source 1..32: mol_type = other DNA
ttgtcctcctcgtccttggtcagtctcaggct

SEQ ID NO: 259 - DNA, 35 bp, synthetic construct
  source 1..35: mol_type = other DNA
acgtgtaccagaacgaggccgagctggtgtggggc

SEQ ID NO: 260 - DNA, 33 bp, synthetic construct
  source 1..33: mol_type = other DNA
cctcgttctggtacacgtggtccttctcctcct

SEQ ID NO: 261 - DNA, 32 bp, synthetic construct
  source 1..32: mol_type = other DNA
aaggtgagcaactgcctgaccccctacttcaa

SEQ ID NO: 262 - DNA, 34 bp, synthetic construct
  source 1..34: mol_type = other DNA
aggcagttgctcaccttgccccacaccagctcgg

SEQ ID NO: 263 - DNA, 32 bp, synthetic construct
  source 1..32: mol_type = other DNA
atggtgaggaactgcctgaccccctacttcaa

SEQ ID NO: 264 - DNA, 32 bp, synthetic construct
  source 1..32: mol_type = other DNA
aggcagttcctcaccatgccccacaccagctc

SEQ ID NO: 265 - DNA, 33 bp, synthetic construct
  source 1..33: mol_type = other DNA
caagaacgggtacatcctgaagtacaaggacgc

SEQ ID NO: 266 - DNA, 34 bp, synthetic construct
  source 1..34: mol_type = other DNA
aggatgtacccgttcttggggtcgttgaagtagg

SEQ ID NO: 267 - DNA, 32 bp, synthetic construct
  source 1..32: mol_type = other DNA
agaacaaggacatcctgaagtacaaggacgcc

SEQ ID NO: 268 - DNA, 32 bp, synthetic construct
  source 1..32: mol_type = other DNA
caggatgtccttgttcttggggtcgttgaagt

SEQ ID NO: 269 - DNA, 33 bp, synthetic construct
  source 1..33: mol_type = other DNA
agtacaagctcgccaagacccccggcgacttcg

SEQ ID NO: 270 - DNA, 38 bp, synthetic construct
  source 1..38: mol_type = other DNA
tcttggcgagcttgtacttcaggatgtacttgttcttg

SEQ ID NO: 271 - DNA, 32 bp, synthetic construct
  source 1..32: mol_type = other DNA
ttcgaggagtggatcaccagcaagatcagcga

SEQ ID NO: 272 - DNA, 32 bp, synthetic construct
  source 1..32: mol_type = other DNA
gtgatccactcctcgaagtcgccgggggtctt

SEQ ID NO: 273 - DNA, 33 bp, synthetic construct
  source 1..33: mol_type = other DNA
caagatcaaggaggacgacggcgagcccttcgt

SEQ ID NO: 274 - DNA, 33 bp, synthetic construct
  source 1..33: mol_type = other DNA
tcgtcctccttgatcttgctggtgatccagtcc

SEQ ID NO: 275 - DNA, 19 bp, synthetic construct
  source 1..19: mol_type = other DNA
ccagggaccatgttttgcc

SEQ ID NO: 276 - DNA, 21 bp, synthetic construct
  source 1..21: mol_type = other DNA
cgaagacgacaagatggacaa

SEQ ID NO: 277 - DNA, 36 bp, synthetic construct
  source 1..36: mol_type = other DNA
  modified_base 26: mod_base = OTHER; note = n is a or g
ggaagatnactctacaaacctgtagngnnnnnnnnn

SEQ ID NO: 278 - DNA, 36 bp, synthetic construct; identical to SEQ ID NO: 277
  source 1..36: mol_type = other DNA
  modified_base 8: mod_base = OTHER; note = n is a or g
  modified_base 26: mod_base = OTHER; note = n is a or g
  modified_base 28: mod_base = OTHER; note = n is a or t
  modified_base 29: mod_base = OTHER; note = n is c or t
  modified_base 30: mod_base = OTHER; note = n is c or t
  modified_base 31: mod_base = OTHER; note = n is g or t
  modified_base 32: mod_base = OTHER; note = n is g or t
  modified_base 33: mod_base = OTHER; note = n is a or g
  modified_base 34: mod_base = OTHER; note = n is c or g
  modified_base 35: mod_base = OTHER; note = n is a or g
  modified_base 36: mod_base = OTHER; note = n is c or g

SEQ ID NO: 279 - protein, 17 aa, synthetic construct
AEAAAKEAAAKEAAAKA

SEQ ID NO: 280 - protein, 15 aa, synthetic construct
GGGGSGGGGSGGGGS